European Patent Specification EP 3 431 099 B1, published January 3, 2024. Title: Attenuated Viruses Useful For Vaccines. Applicant: The Research Foundation of State University of New York. Application not assigned. The sequence listing filed with the application follows.

SEQUENCE LISTING (42 sequences)

SEQ ID NO: 1 - DNA, 2643 bp, Human poliovirus 1 Mahoney
atgggtgctcaggtttcatcacagaaagtgggcgcacatgaaaactcaaatagagcgtatggtggttctaccattaattacaccaccattaattattatagagattcagctagtaacgcggcttcgaaacaggacttctctcaagacccttccaagttcaccgagcccatcaaggatgtcctgataaaaacagccccaatgctaaactcgccaaacatagaggcttgcgggtatagcgatagagtactgcaattaacactgggaaactccactataaccacacaggaggcggctaattcagtagtcgcttatgggcgttggcctgaatatctgagggacagcgaagccaatccagtggaccagccgacagaaccagacgtcgctgcatgcaggttttatacgctagacaccgtgtcttggacgaaagagtcgcgagggtggtggtggaagttgcctgatgcactgagggacatgggactctttgggcaaaatatgtactaccactacctaggtaggtccgggtacaccgtgcatgtacagtgtaacgcctccaaattccaccagggggcactaggggtattcgccgtaccagagatgtgtctggccggggatagcaacaccactaccatgcacaccagctatcaaaatgccaatcctggcgagaaaggaggcactttcacgggtacgttcactcctgacaacaaccagacatcacctgcccgcaggttctgcccggtggattacctccttggaaatggcacgttgttggggaatgcctttgtgttcccgcaccagataataaacctacggaccaacaactgtgctacactggtactcccttacgtgaactccctctcgatagatagtatggtaaagcacaataattggggaattgcaatattaccattggccccattaaattttgctagtgagtcctccccagagattccaatcaccttgaccatagcccctatgtgctgtgagttcaatggattaagaaacatcaccctgccacgcttacagggcctgccggtcatgaacacccctggtagcaatcaatatcttactgcagacaacttccagtcaccgtgtgcgctgcctgaatttgatgtgaccccacctattgacatacccggtgaagtaaagaacatgatggaattggcagaaatcgacaccatgattccctttgacttaagtgccacaaaaaagaacaccatggaaatgtatagggttcggttaagtgacaaaccacatacagacgatcccatactctgcctgtcactctctccagcttcagatcctaggttgtcacatactatgcttggagaaatcctaaattactacacacactgggcaggatccctgaagttcacgtttctgttctgtggattcatgatggcaactggcaaactgttggtgtcatacgcgcctcctggagccgacccaccaaagaagcgtaaggaggcgatgttgggaacacatgtgatctgggacataggactgcagtcctcatgtactatggtagtgccatggattagcaacaccacgtatcggcaaaccatagatgatagtttcaccgaaggcggatacatcagcgtcttctaccaaactagaatagtcgtccctctttcgacacccagagagatggacatccttggttttgtgtcagcgtgtaatgacttcagcgtgcgcttgttgcgagataccacacatatagagcaaaaagcgctagcacaggggttaggtcagatgcttgaaagcatgattgacaacacagtccgtgaaacggtgggggcggcaacatctagagacgctctcccaaacactgaagccagtggaccaacacactccaaggaaattccggcactcaccgcagtggaaactggggccacaaatccactagtcccttctgatacagtgcaaaccagacatgttgtacaacataggtcaaggtcagagtctagcatagagtctttcttcgcgcggggtgcatgcgtgaccattatgaccgtggataacccagcttccaccacgaataaggataagctatttgcagtgtggaagatcacttataaagatactgtccagttacggaggaaattggagttcttcacctattctagatttgatatggaacttacctttgtggttactgcaaatttcactgagactaacaatgggcatgccttaaatcaagtgtaccaaattatgtacgtaccaccaggcgctccagtgcccgagaaatgggacgactacacatggcaaacctcatcaaatccatcaatcttttacacctacggaacagctccagcccggatctcggtaccgtatgttggtatttcgaacgcctattcacacttttacgacggtttttccaaagtaccactgaaggaccagtcggcagcactaggtgactccctttatggtgcagcatctctaaatgacttcggtattttggctgttagagtagtcaatgatcacaacccgaccaaggtcacctccaaaatcagagtgtatctaaaacccaaacacatcagagtctggtgcccgcgtccaccgagggcagtggcgtactacggccctggagtggattacaaggatggtacgcttacacccctctccaccaaggatctgaccacatat

SEQ ID NO: 2 - DNA, 7521 bp, Unknown
  synthetic
ttaaaacagctctggggttgtacccaccccagaggcccacgtggcggctagtactccggtattgcggtacccttgtacgcctgttttatactcccttcccgtaacttagacgcacaaaaccaagttcaatagaagggggtacaaaccagtaccaccacgaacaagcacttctgtttccccggtgatgtcgtatagactgcttgcgtggttgaaagcgacggatccgttatccgcttatgtacttcgagaagcccagtaccacctcggaatcttcgatgcgttgcgctcagcactcaaccccagagtgtagcttaggctgatgagtctggacatccctcaccggtgacggtggtccaggctgcgttggcggcctacctatggctaacgccatgggacgctagttgtgaacaaggtgtgaagagcctattgagctacataagaatcctccggcccctgaatgcggctaatcccaacctcggagcaggtggtcacaaaccagtgattggcctgtcgtaacgcgcaagtccgtggcggaaccgactactttgggtgtccgtgtttccttttattttattgtggctgcttatggtgacaatcacagattgttatcataaagcgaattggattggccatccggtgaaagtgagactcattatctatctgtttgctggatccgctccattgagtgtgtttactctaagtacaatttcaacagttatttcaatcagacaattgtatcataatgggtgctcaggtttcgtcgcaaaaagtaggtgcgcatgaaaactcgaatcgtgcgtatggttcgtcgacgataaattatacgacgataaattattatcgtgattcggcgtctaatgcggcttcgaaacaagatttttcgcaagatccgtcgaaatttacggaaccgataaaagatgtattaataaaaacggcgccgatgttaaattcgccgaatatagaagcgtgtggttattcggatcgtgtattacaattaacgttaggtaattcgacgataacgacgcaagaagcggctaattcggtagtagcgtatggtcgttggccggagtatttacgtgattcggaagcgaatccggtagatcaaccgacggaaccggacgtcgcggcgtgtcgtttttatacgttagatacggtatcgtggacgaaagaatcgcgaggttggtggtggaaattaccggatgcgttacgtgatatgggtttatttggtcaaaatatgtattatcattatttaggtcgttcgggttatacggtacatgtacaatgtaatgcgtcgaaatttcatcaaggtgcgttaggtgtatttgcggtaccggaaatgtgtttagcgggtgactcgaatacgacgacgatgcatacgtcgtatcaaaatgcgaatccgggtgaaaaaggtggtacgtttacgggtacgtttacgccggataataatcaaacgtcgccggcgcgtcgtttttgtccggtagattatttattaggtaatggtacgttattagggaatgcctttgtatttccgcatcaaataataaatttgcgtacgaataattgtgcgacgttagtattaccgtatgtaaattcgttatcgatagattcgatggtaaaacataataattggggtatagcaatattaccgttagcgccgttaaattttgcgtcggaatcgtcgccggaaataccgataacgttaacgatagcgccgatgtgttgtgaatttaatggtttgcgtaatataacgttaccgcgtttacaaggtttaccggtaatgaatacgccgggctcgaatcagtatttaacggcggataattttcaatcgccgtgtgcgttaccggaatttgatgtaacgccgccgatagatataccgggtgaagtaaaaaatatgatggaattagcggaaatagatacgatgataccgtttgatttatcggcgacgaaaaaaaatacgatggaaatgtatcgtgtacgtttatcggataaaccgcatacggatgatccgatattatgtttatcgttatcgccggcgtcggatcctaggttatcgcatacgatgttaggtgagatattaaattattatacgcattgggcgggttcgttaaaatttacgtttttattttgtggttcgatgatggcgacgggtaaattattagtatcgtatgcgccgccgggtgcggatccgccgaaaaaacgtaaagaagcgatgttaggtacgcatgtaatatgggatataggtttacaatcgtcgtgtacgatggtagtaccgtggatatcgaatacgacgtatcgtcaaacgatagatgattcgtttacggaaggtggttatatatcggtattttatcaaacgcgtatagtagtaccgttatcgacgccgcgtgaaatggatatattaggttttgtatcggcgtgtaatgatttttcggtacgtttattacgtgatacgacgcatatagaacaaaaagcgctagcacaaggtttaggtcaaatgttagaatcgatgatagataatacggtacgtgaaacggtaggtgcggctacgtcgcgtgatgcgttaccgaatacggaagcgtcgggtccgacgcactcgaaagaaataccggcgttaacggcggtagaaacgggtgcgacgaatccactagtcccgtcggatacggtacaaacgcgtcatgtagtacaacatcgttcgcgttcggaatcgtcgatagaatcgttttttgcgcgtggtgcgtgtgtaacgataatgacggtagataatccggcgtcgacgacgaataaagataaattatttgcggtatggaaaataacgtataaagatacggtacaattacgtcgtaaattagaatttttcacgtattcgcgttttgatatggaattaacgtttgtagtaacggcgaattttacggaaacgaataatggtcatgcgttaaatcaagtatatcaaataatgtacgtaccgccgggtgcgccggtacccgaaaaatgggatgattatacgtggcaaacgtcgtcgaatccgtcgatattttacacgtatggtacggcgccggcgcgtatatcggtaccgtatgtaggtatatctaatgcgtattcgcatttttatgatggtttctcgaaagtaccgttaaaagatcaatcggcggcgttaggtgattcgttatatggtgcggcgtcgttaaatgattttggtatattagcggtacgtgtagtaaatgatcataatccgacgaaggtcacctcgaaaatacgtgtatatttaaaaccgaaacatatacgtgtatggtgtccgcgtccgccgcgtgcggtagcgtattatggtccgggtgtagattataaagatggtacgttaacgccgttatcgacgaaagatttaacgacgtatggattcggacaccaaaacaaagcggtgtacactgcaggttacaaaatttgcaactaccacttggccactcaggatgatttgcaaaacgcagtgaacgtcatgtggagtagagacctcttagtcacagaatcaagagcccagggcaccgattcaatcgcaaggtgcaattgcaacgcaggggtgtactactgcgagtctagaaggaaatactacccagtatccttcgttggcccaacgttccagtacatggaggctaataactattacccagctaggtaccagtcccatatgctcattggccatggattcgcatctccaggggattgtggtggcatactcagatgtcaccacggggtgatagggatcattactgctggtggagaagggttggttgcattttcagacattagagacttgtatgcctacgaagaagaagccatggaacaaggcctcaccaattacatagagtcacttggggccgcatttggaagtggatttactcagcagattagcgacaaaataacagagttgaccaatatggtgaccagtaccatcactgaaaagctacttaagaacttgatcaagatcatatcctcactagttattataactaggaactatgaagacaccacaacagtgctcgctaccctggcccttcttgggtgtgatgcttcaccatggcagtggcttagaaagaaagcatgcgatgttctggagataccttatgtcatcaagcaaggtgacagttggttgaagaagtttactgaagcatgcaacgcagctaagggactggagtgggtgtcaaacaaaatctcaaaattcattgattggctcaaggagaaaattatcccacaagctagagataagttggaatttgtaacaaaacttagacaactagaaatgctggaaaaccaaatctcaactatacaccaatcatgccctagtcaggaacaccaggaaattctattcaataatgtcagatggttatccatccagtctaagaggtttgcccctctttacgcagtggaagccaaaagaatacagaaactcgagcatactattaacaactacatacagttcaagagcaaacaccgtattgaaccagtatgtttgctagtacatggcagccccggaacaggtaaatctgtagcaaccaacctgattgctagagccatagctgaaagagaaaacacgtccacgtactcgctacccccggatccatcacacttcgacggatacaaacaacagggagtggtgattatggacgacctgaatcaaaacccagatggtgcggacatgaagctgttctgtcagatggtatcaacagtggagtttataccacccatggcatccctggaggagaaaggaatcctgtttacttcaaattacgttctagcatccacaaactcaagcagaatttccccccccactgtggcacacagtgacgcgttagccaggcgctttgcgttcgacatggacattcaggtcatgaatgagtattctagagatgggaaattgaacatggccatggctactgaaatgtgtaagaactgtcaccaaccagcaaactttaagagatgctgtcctttagtgtgtggtaaggcaattcaattaatggacaaatcttccagagttagatacagtattgaccagatcactacaatgattatcaatgagagaaacagaagatccaacattggcaattgtatggaggctttgtttcaaggaccactccagtataaagacttgaaaattgacatcaagacgagtccccctcctgaatgtatcaatgacttgctccaagcagttgactcccaggaggtgagagattactgtgagaagaagggttggatagttaacatcaccagccaggttcaaacagaaaggaacatcaacagggcaatgacaattctacaagcggtgacaaccttcgccgcagtggctggagttgtctatgtcatgtataaactgtttgctggacaccagggagcatacactggtttaccaaacaaaaaacccaacgtgcccaccattcggacagcaaaggtacaaggaccagggttcgattacgcagtggctatggctaaaagaaacattgttacagcaactactagcaagggagagttcactatgttaggagtccacgacaacgtggctattttaccaacccacgcttcacctggtgaaagcattgtgatcgatggcaaagaagtggagatcttggatgccaaagcgctcgaagatcaagcaggaaccaatcttgaaatcactataatcactctaaagagaaatgaaaagttcagagacattagaccacatatacctactcaaatcactgagacaaatgatggagtcttgatcgtgaacactagcaagtaccccaatatgtatgttcctgtcggtgctgtgactgaacagggatatctaaatctcggtgggcgccaaactgctcgtactctaatgtacaactttccaaccagagcaggacagtgtggtggagtcatcacatgtactgggaaagtcatcgggatgcatgttggtgggaacggttcacacgggtttgcagcggccctgaagcgatcatacttcactcagagtcaaggtgaaatccagtggatgagaccttcgaaggaagtgggatatccaatcataaatgccccgtccaaaaccaagcttgaacccagtgctttccactatgtgtttgaaggggtgaaggaaccagcagtcctcactaaaaacgatcccaggcttaagacagactttgaggaggcaattttctccaagtacgtgggtaacaaaattactgaagtggatgagtacatgaaagaggcagtagaccactatgctggccagctcatgtcactagacatcaacatagaacaaatgtgcttggaggatgccatgtatggcactgatggtctagaagcacttgatttgtccaccagtgctggctacccttatgtagcaatgggaaagaagaagagagacatcttgaacaaacaaaccagagacactaaggaaatgcaaaaactgctcgacacatatggaatcaacctcccactggtgacttatgtaaaggatgaacttagatccaaaacaaaggttgagcaggggaaatccagattaattgaagcttctagtttgaatgactcagtggcaatgagaatggcttttgggaacctatatgctgcttttcacaaaaacccaggagtgataacaggttcagcagtggggtgcgatccagatttgttttggagcaaaattccggtattgatggaagagaagctgtttgcttttgactacacagggtatgatgcatctctcagccctgcttggttcgaggcactaaagatggtgcttgagaaaatcggattcggagacagagttgactacatcgactacctaaaccactcacaccacctgtacaagaataaaacatactgtgtcaagggcggtatgccatctggctgctcaggcacttcaatttttaactcaatgattaacaacttgattatcaggacactcttactgaaaacctacaagggcatagatttagaccacctaaaaatgattgcctatggtgatgatgtaattgcttcctacccccatgaagttgacgctagtctcctagcccaatcaggaaaagactatggactaactatgactccagctgacaaatcagctacatttgaaacagtcacatgggagaatgtaacattcttgaagagattcttcagggcagacgagaaatacccatttcttattcatccagtaatgccaatgaaggaaattcatgaatcaattagatggacaaaagatcctaggaacactcaggatcacgttcgctctctgtgccttttagcttggcacaatggcgaagaagaatataacaaattcctagctaaaatcaggagtgtgccaattggaagagctttattgctcccagagtactcaacattgtaccgccgttggcttgactcattttagtaaccctacctcagtcgaattggattgggtcatactggtgtaggggtaaatttttctttaattcggaggaaaaaaaaaaaaaaaaaaaaaaaaaaaaaaaaaaaaaaaaaaaaaaaaaaaaaaaaaaaaaaaaaaaaaaaaaaaaaaaa

SEQ ID NO: 3 - DNA, 7521 bp, Unknown
  synthetic
ttaaaacagctctggggttgtacccaccccagaggcccacgtggcggctagtactccggtattgcggtacccttgtacgcctgttttatactcccttcccgtaacttagacgcacaaaaccaagttcaatagaagggggtacaaaccagtaccaccacgaacaagcacttctgtttccccggtgatgtcgtatagactgcttgcgtggttgaaagcgacggatccgttatccgcttatgtacttcgagaagcccagtaccacctcggaatcttcgatgcgttgcgctcagcactcaaccccagagtgtagcttaggctgatgagtctggacatccctcaccggtgacggtggtccaggctgcgttggcggcctacctatggctaacgccatgggacgctagttgtgaacaaggtgtgaagagcctattgagctacataagaatcctccggcccctgaatgcggctaatcccaacctcggagcaggtggtcacaaaccagtgattggcctgtcgtaacgcgcaagtccgtggcggaaccgactactttgggtgtccgtgtttccttttattttattgtggctgcttatggtgacaatcacagattgttatcataaagcgaattggattggccatccggtgaaagtgagactcattatctatctgtttgctggatccgctccattgagtgtgtttactctaagtacaatttcaacagttatttcaatcagacaattgtatcataatgggtgctcaggtttcgtctcagaaggtaggtgctcacgaaaatagcaacagggcatacggatcatccacaatcaactatacaacaatcaactactaccgggactccgcctccaatgcagcttcgaaacaagattttagccaggatccatctaaatttactgaaccaattaaagacgtgctcatcaagactgcacctatgttgaatagccctaacattgaagcctgtggctactcagaccgggtgcttcagctgaccctcggtaattcaaccatcacaacgcaagaagctgcaaacagcgtggtggcatacggaaggtggccagagtacttaagagattctgaggcaaaccctgtcgatcaaccaaccgagccggacgtcgcggcgtgtcgattctacaccctcgatactgtaagctggaccaaggaatcgcgaggttggtggtggaaacttccagacgccctacgcgatatgggtttgttcggtcagaacatgtattatcattatttgggacgctctggatatacagtccacgtgcaatgcaatgcttcaaagtttcatcagggagctttgggtgtgttcgcggtgccggaaatgtgcttagcaggagactcaaatacgaccacaatgcatacttcttaccagaacgcaaaccccggagaaaagggcggtacgtttaccgggacctttaccccagataataatcaaacctccccagcaagacgtttttgtccagttgactatttgttgggcaacggtacactactagggaatgccttcgtatttcctcatcagattatcaatcttagaactaataattgcgcaactctcgtgttgccatatgtaaattctctgtccatcgactcgatggtgaaacataacaactgggggatagcaatattacctctcgcgcctctgaacttcgcgtcagaatcaagtccggaaatcccgataacacttactatcgctcccatgtgttgcgagttcaacgggctcaggaatataacactacccaggctgcaagggctaccagttatgaatacaccaggatctaaccagtacttaaccgccgataacttccaatccccatgcgccttaccagagttcgatgtcacgccgcccatcgatatccctggggaggtgaaaaatatgatggagcttgccgagattgatacaatgataccattcgatctgtccgcaactaagaaaaatacaatggagatgtaccgtgtgagactttccgataagcctcacaccgacgacccaattctgtgtctcagtctatctcctgcaagtgaccctaggcttagccacaccatgctgggcgagatattgaactattatacccactgggcgggcagtcttaaattcaccttcttattttgtgggtcaatgatggctacgggtaagttgctagtaagctacgctccaccaggcgcagatcctccgaagaaaaggaaagaagctatgcttgggacccacgtcatttgggatattggtttacaatcttcgtgcaccatggtggttccttggatatcaaatacgacctacagacagacaatcgacgactcctttacggagggtggttatatatcagtgttttatcagacccgtattgtggtgccactgtctaccccacgggaaatggatattctgggattcgtctccgcctgcaacgacttctcagtcaggctcctaagggacacgacccacattgaacagaaggcgctagcacaaggactgggtcaaatgttggagtcaatgatagataataccgtaagggagaccgtaggagctgccacttcacgggatgcactgccgaatacagaggcatcagggcccacccattcaaaagagatcccagctctgacagctgtagagaccggtgcaaccaacccactagtcccatcggacactgttcagacacggcacgtggtgcagcacagaagtagatccgaatcctcgattgaaagctttttcgccagaggcgcctgtgtaacaataatgacggtagacaatcccgcaagtactaccaacaaagacaaactgttcgctgtctggaaaataacatacaaggacaccgtacaactgagaagaaagcttgaattttttacttacagcaggttcgacatggagttaacattcgtagtgaccgctaacttcaccgaaaccaataacgggcacgccctgaaccaggtttatcagataatgtacgtaccgccgggtgcccccgtacccgaaaagtgggatgattatacttggcagactagctccaacccttccatattctatacttatggcaccgcgccggcgagaatttcagttccatacgtgggaatatcaaatgcatactctcatttctatgatggcttctcaaaggtgcctttaaaagaccaatcagcggccctgggagattcgttgtacggggccgcctccttgaacgattttgggatcctagcagtgagggtggtgaacgaccataatccaacgaaggtcaccagtaagatacgggtctacttgaagcctaagcatattcgtgtgtggtgtccaagacctccacgcgccgtcgcatattatggacccggtgtcgactataaagacgggaccttgaccccactgagtacaaaagacctcacaacttacggattcggacaccaaaacaaagcggtgtacactgcaggttacaaaatttgcaactaccacttggccactcaggatgatttgcaaaacgcagtgaacgtcatgtggagtagagacctcttagtcacagaatcaagagcccagggcaccgattcaatcgcaaggtgcaattgcaacgcaggggtgtactactgcgagtctagaaggaaatactacccagtatccttcgttggcccaacgttccagtacatggaggctaataactattacccagctaggtaccagtcccatatgctcattggccatggattcgcatctccaggggattgtggtggcatactcagatgtcaccacggggtgatagggatcattactgctggtggagaagggttggttgcattttcagacattagagacttgtatgcctacgaagaagaagccatggaacaaggcctcaccaattacatagagtcacttggggccgcatttggaagtggatttactcagcagattagcgacaaaataacagagttgaccaatatggtgaccagtaccatcactgaaaagctacttaagaacttgatcaagatcatatcctcactagttattataactaggaactatgaagacaccacaacagtgctcgctaccctggcccttcttgggtgtgatgcttcaccatggcagtggcttagaaagaaagcatgcgatgttctggagataccttatgtcatcaagcaaggtgacagttggttgaagaagtttactgaagcatgcaacgcagctaagggactggagtgggtgtcaaacaaaatctcaaaattcattgattggctcaaggagaaaattatcccacaagctagagataagttggaatttgtaacaaaacttagacaactagaaatgctggaaaaccaaatctcaactatacaccaatcatgccctagtcaggaacaccaggaaattctattcaataatgtcagatggttatccatccagtctaagaggtttgcccctctttacgcagtggaagccaaaagaatacagaaactcgagcatactattaacaactacatacagttcaagagcaaacaccgtattgaaccagtatgtttgctagtacatggcagccccggaacaggtaaatctgtagcaaccaacctgattgctagagccatagctgaaagagaaaacacgtccacgtactcgctacccccggatccatcacacttcgacggatacaaacaacagggagtggtgattatggacgacctgaatcaaaacccagatggtgcggacatgaagctgttctgtcagatggtatcaacagtggagtttataccacccatggcatccctggaggagaaaggaatcctgtttacttcaaattacgttctagcatccacaaactcaagcagaatttccccccccactgtggcacacagtgacgcgttagccaggcgctttgcgttcgacatggacattcaggtcatgaatgagtattctagagatgggaaattgaacatggccatggctactgaaatgtgtaagaactgtcaccaaccagcaaactttaagagatgctgtcctttagtgtgtggtaaggcaattcaattaatggacaaatcttccagagttagatacagtattgaccagatcactacaatgattatcaatgagagaaacagaagatccaacattggcaattgtatggaggctttgtttcaaggaccactccagtataaagacttgaaaattgacatcaagacgagtccccctcctgaatgtatcaatgacttgctccaagcagttgactcccaggaggtgagagattactgtgagaagaagggttggatagttaacatcaccagccaggttcaaacagaaaggaacatcaacagggcaatgacaattctacaagcggtgacaaccttcgccgcagtggctggagttgtctatgtcatgtataaactgtttgctggacaccagggagcatacactggtttaccaaacaaaaaacccaacgtgcccaccattcggacagcaaaggtacaaggaccagggttcgattacgcagtggctatggctaaaagaaacattgttacagcaactactagcaagggagagttcactatgttaggagtccacgacaacgtggctattttaccaacccacgcttcacctggtgaaagcattgtgatcgatggcaaagaagtggagatcttggatgccaaagcgctcgaagatcaagcaggaaccaatcttgaaatcactataatcactctaaagagaaatgaaaagttcagagacattagaccacatatacctactcaaatcactgagacaaatgatggagtcttgatcgtgaacactagcaagtaccccaatatgtatgttcctgtcggtgctgtgactgaacagggatatctaaatctcggtgggcgccaaactgctcgtactctaatgtacaactttccaaccagagcaggacagtgtggtggagtcatcacatgtactgggaaagtcatcgggatgcatgttggtgggaacggttcacacgggtttgcagcggccctgaagcgatcatacttcactcagagtcaaggtgaaatccagtggatgagaccttcgaaggaagtgggatatccaatcataaatgccccgtccaaaaccaagcttgaacccagtgctttccactatgtgtttgaaggggtgaaggaaccagcagtcctcactaaaaacgatcccaggcttaagacagactttgaggaggcaattttctccaagtacgtgggtaacaaaattactgaagtggatgagtacatgaaagaggcagtagaccactatgctggccagctcatgtcactagacatcaacatagaacaaatgtgcttggaggatgccatgtatggcactgatggtctagaagcacttgatttgtccaccagtgctggctacccttatgtagcaatgggaaagaagaagagagacatcttgaacaaacaaaccagagacactaaggaaatgcaaaaactgctcgacacatatggaatcaacctcccactggtgacttatgtaaaggatgaacttagatccaaaacaaaggttgagcaggggaaatccagattaattgaagcttctagtttgaatgactcagtggcaatgagaatggcttttgggaacctatatgctgcttttcacaaaaacccaggagtgataacaggttcagcagtggggtgcgatccagatttgttttggagcaaaattccggtattgatggaagagaagctgtttgcttttgactacacagggtatgatgcatctctcagccctgcttggttcgaggcactaaagatggtgcttgagaaaatcggattcggagacagagttgactacatcgactacctaaaccactcacaccacctgtacaagaataaaacatactgtgtcaagggcggtatgccatctggctgctcaggcacttcaatttttaactcaatgattaacaacttgattatcaggacactcttactgaaaacctacaagggcatagatttagaccacctaaaaatgattgcctatggtgatgatgtaattgcttcctacccccatgaagttgacgctagtctcctagcccaatcaggaaaagactatggactaactatgactccagctgacaaatcagctacatttgaaacagtcacatgggagaatgtaacattcttgaagagattcttcagggcagacgagaaatacccatttcttattcatccagtaatgccaatgaaggaaattcatgaatcaattagatggacaaaagatcctaggaacactcaggatcacgttcgctctctgtgccttttagcttggcacaatggcgaagaagaatataacaaattcctagctaaaatcaggagtgtgccaattggaagagctttattgctcccagagtactcaacattgtaccgccgttggcttgactcattttagtaaccctacctcagtcgaattggattgggtcatactggtgtaggggtaaatttttctttaattcggaggaaaaaaaaaaaaaaaaaaaaaaaaaaaaaaaaaaaaaaaaaaaaaaaaaaaaaaaaaaaaaaaaaaaaaaaaaaaaaaaa

SEQ ID NO: 4 - DNA, 2643 bp, Unknown
  synthetic
atgggagctcaggtgtcatcccaaaaagtaggcgcacacgaaaactcgaatcgggcatacggatctagtacgattaactatactacaatcaattactatagggactccgcctctaacgccgcttcgaaacaggacttttcgcaagaccctagcaagtttaccgaaccgattaaggacgtgttgatcaaaaccgcacctatgcttaactcacctaacatagaggcatgcggatactccgatagggtgttgcaactgacactcggcaatagtacgattacgacacaggaagccgctaatagcgtagtcgcatacggaaggtggcccgaataccttagagactccgaagcgaatccagtcgatcagcctaccgaacctgacgtcgccgcatgtcggttttacacactcgataccgtgtcatggactaaggaatcgcgagggtggtggtggaaactgccagacgcattgcgcgatatggggttgttcggacagaatatgtactatcactatctcggaagatccgggtataccgtacacgtgcaatgtaacgcctctaagtttcaccagggagcgttaggcgtattcgcagtgccagagatgtgtctagccggagactccaatacgactactatgcatacctcataccaaaacgctaacccaggcgaaaagggggggacatttaccggaacattcacacccgataacaatcagacatcccccgctagacggttttgcccagtcgactatctactcggaaacggtacactgttagggaatgccttcgtattcccacaccagataattaacttacggactaacaattgcgcaaccctagtgttgccatacgttaactcactgtcaatcgatagtatggtgaaacataacaattgggggatcgcaatattaccgttagcgccactgaatttcgccagcgaatcgtcacctgagataccgattacccttacaatcgcacctatgtgttgcgagttcaacggattgcgtaatataaccctaccacggttgcaggggttgcccgttatgaataccccagggtctaaccaataccttaccgccgataatttccaatccccttgcgcactgccagagttcgacgtaacccctccaatcgacatacccggcgaggttaagaatatgatggagttagccgaaatcgatactatgataccgttcgatctatccgctacgaaaaagaatactatggagatgtatcgcgtgagattgtccgataagccacataccgacgatccgatactgtgtctgtcactgtcacccgccagcgatcctaggttgtcccatacaatgttaggcgagatactgaattactatacccattgggccggtagtctgaaattcacatttctgttttgcggatctatgatggcgaccggaaagctgttagtgtcatacgctccacccggagccgatccacctaaaaaacgcaaggaagcgatgctcggtacacacgtgatatgggatatcggactgcaatcgtcatgtactatggtcgtgccatggatatcgaatacgacttatagacagacaatcgacgatagctttaccgagggggggtatattagcgtattctatcagacacgtatcgtagtgccactgtcaacccctagagagatggacatactcggattcgtatccgcatgtaacgactttagcgtgagactgttacgcgatactacccatatcgaacagaaagcgctagcacaggggttagggcaaatgctagagtcaatgatcgacaatactgtacgcgaaaccgtaggcgcagcgaccagtagggacgcactaccgaataccgaagcgagcggacctacccactctaaagagataccggcactaaccgccgtcgaaaccggagcgactaacccactagtcccatccgataccgtgcaaaccagacacgtagtgcaacatcggtctagatccgagtcatcaatcgaatcctttttcgctagaggcgcatgcgttacgattatgaccgtcgataacccagcgtcaacgactaacaaagacaaattgttcgccgtatggaaaattacctataaggataccgtgcaattgcgacgtaaactagagttctttacatactctagattcgatatggagcttacattcgtagtgaccgctaactttaccgagactaataacggtcacgcccttaatcaggtgtatcagattatgtacgtaccgccaggcgcaccagtgcccgaaaaatgggacgactatacatggcagactagctctaatccgtcaattttctatacatacggtaccgcaccagctaggattagcgtgccatacgtcggtatatcgaacgcttactcacacttttacgacggattctctaaagtgccacttaaggaccaatccgccgcactaggcgatagcctatacggagccgctagtcttaacgatttcggtatactcgccgttagggtcgtgaacgaccataaccctactaaggtcacctctaagattagggtgtatcttaagcctaagcatattagggtgtggtgtcctagaccgcctagagccgttgcgtattacggaccaggcgtcgactataaggacggtacattgaccccactgtcaacgaaagaccttacgacgtac

SEQ ID NO: 5 - DNA, 2643 bp, Unknown
  synthetic
atgggagctcaagtatcttcacaaaaagttggtgctcatgaaaattcaaacagagcatatggttcttcaacaataaactacaccacaataaattattacagggacagtgcttcaaatgcagcttcgaaacaagatttttctcaagatccttccaagttcacagagcccatcaaagatgttttaataaaaacagcacccatgctgaacagccccaacattgaagcatgtggttatagtgacagagttctacagctcacgctgggaaattcaacaataacaactcaagaagcagcaaattctgtggtggcctatggtcgttggccagagtatctgcgggactcggaggcaaatcctgtggaccagccaacagagccggacgtcgctgcctgccgcttctacacgttagacacggtctcctggaccaaggagtcgcgaggctggtggtggaaacttccagatgctctgcgggacatgggcctctttgggcagaacatgtactatcattatttgggaagaagtggctacacggtccatgtgcagtgtaatgcatccaagtttcatcaaggtgccctgggcgtgttcgcggttcctgagatgtgtttggctggggacagcaacaccaccaccatgcacacgtcctaccaaaatgcaaatccaggagaaaaaggtggcaccttcacgggcaccttcactccagacaacaaccagacctcgccggcgcgccgcttctgcccagtagattatcttcttggaaatggcacgctgctggggaatgcctttgtatttcctcatcaaataataaatttgaggaccaacaactgtgccaccttggttcttccttatgtcaacagcctctccattgactccatggtgaagcacaacaactggggaatagcaatattacctttggcacctttaaattttgcctcggagagttctccagagatccccatcaccctcaccatcgcgccgatgtgctgcgagttcaatgggctgaggaacatcaccctgcccaggctacaaggtcttcctgtcatgaacacaccaggttcaaatcagtatttaacagcagacaacttccagtctccatgtgctttgccagaatttgatgtcactccaccaatagatattccaggagaagtaaagaacatgatggaactagcagaaatagacaccatgattccatttgatctttcagccaccaagaagaacaccatggagatgtaccgtgtcaggctttcagataaaccacacacagatgatccaattctctgcctcagtctttctccagcctcggaccctaggctcagccacaccatgctaggagagatattaaattattacacgcactgggcaggctccctgaagttcaccttcctcttctgtggctccatgatggcaactggaaaattattagtatcatatgcgccgccgggggcagatcctccaaagaagaggaaggaggccatgctaggaactcatgtaatatgggacattgggttgcagagcagctgcaccatggttgttccctggatctccaacaccacctacaggcagaccattgatgacagcttcacagaaggtggttatatttctgtcttctaccagacaagaattgtggtgccgctgtccactccaagagaaatggatattcttggatttgtatcagcctgcaatgacttctctgtgaggctgctgcgggacaccactcatattgagcagaaggcgctagcacaaggacttggacaaatgctggagtccatgattgacaacactgtgcgggagactgtgggggcggccacctcaagagatgctttgccaaatacagaggcttcggggccaacacacagcaaagaaataccagctttgacagcagtagaaactggagcaacaaatccactagtcccttcagatactgtacaaacaagacatgtggtgcagcacagatcaagaagtgaaagttcaatagaatccttctttgctcgtggggcctgtgtcaccatcatgactgtggacaacccagcctccaccaccaacaaagataaattatttgctgtgtggaagatcacctacaaagatactgtgcagctaagaagaaaactagagttcttcacctactcaagatttgacatggaactaacttttgtggtcacagccaacttcacagagaccaacaatggacatgctttgaatcaagtctaccagattatgtacgtaccaccaggggctcctgtgcccgaaaaatgggatgactacacgtggcagacttcatcaaatccttccatcttctacacatatggaacagcgccggccaggatatcagttccttatgtgggcatctcaaatgcttacagccacttctatgatggcttctccaaagtacctttgaaggaccagtcggcggcgctgggggacagtttatatggtgcagcatctctaaatgattttggaattttggctgtccgtgtagtaaatgaccacaaccccaccaaggtcaccagcaagatccgagtatatttaaaaccaaagcacatccgagtgtggtgtccgagaccgccaagagctgtagcgtattacggtcctggtgtggactataaagatgggactttgactcctttgtccaccaaagacctcaccacgtac

SEQ ID NO: 6 - DNA, 7441 bp, Unknown
  synthetic
ttaaaacagctctggggttgtacccaccccagaggcccacgtggcggctagtactccggtattgcggtacccttgtacgcctgttttatactcccttcccgtaacttagacgcacaaaaccaagttcaatagaagggggtacaaaccagtaccaccacgaacaagcacttctgtttccccggtgatgtcgtatagactgcttgcgtggttgaaagcgacggatccgttatccgcttatgtacttcgagaagcccagtaccacctcggaatcttcgatgcgttgcgctcagcactcaaccccagagtgtagcttaggctgatgagtctggacatccctcaccggtgacggtggtccaggctgcgttggcggcctacctatggctaacgccatgggacgctagttgtgaacaaggtgtgaagagcctattgagctacataagaatcctccggcccctgaatgcggctaatcccaacctcggagcaggtggtcacaaaccagtgattggcctgtcgtaacgcgcaagtccgtggcggaaccgactactttgggtgtccgtgtttccttttattttattgtggctgcttatggtgacaatcacagattgttatcataaagcgaattggattggccatccggtgaaagtgagactcattatctatctgtttgctggatccgctccattgagtgtgtttactctaagtacaatttcaacagttatttcaatcagacaattgtatcataatgggcgcgcaagtgtcgtctcaaaaggttggagcccacgagaatagtaacagagcatacggatcaagcacaataaattatacgacgatcaattactaccgtgactcggcatccaacgccgctagcaaacaggacttttctcaggatccatctaaattcacggaacccataaaagacgtgcttattaagaccgcacctatgctgaattcaccgaatatcgaagcctgtggttactctgaccgggtgctacagctgacacttggcaactcaacgatcacaacccaagaggccgcaaattccgtagtagcgtacggtaggtggccagagtacctacgtgattcagaggctaaccctgtagatcaacctaccgaaccggacgtggcagcttgtcgtttctacactcttgataccgtgtcctggaccaaggaaagtaggggttggtggtggaaactccccgacgcccttagggatatggggctgttcggtcagaacatgtactatcactatctgggacgctcaggctatacggtacacgtgcaatgcaacgcaagtaagtttcatcagggcgcgctgggagtgttcgcagttccggaaatgtgcctagctggcgactcaaatacaacgactatgcatacaagttatcagaacgcgaacccaggagaaaaggggggaacatttacaggcacatttaccccagataataaccaaacctccccagcacggagattctgtcctgtagactacttgttggggaacggaaccctacttggtaacgcattcgtttttccacatcaaattatcaatcttagaactaataattgtgcaactctcgtgttgccatatgtcaattccttgtcgatagactccatggtcaaacataacaactggggcatagccattctaccgctcgcaccactgaacttcgcatccgaatcctcacccgaaatccccataacactcacaatcgcaccaatgtgttgcgaatttaacggactgcggaatataaccctaccgagactccagggtttacccgtaatgaatacgccaggatcaaatcagtacttaaccgccgataatttccaatccccatgcgccttaccagaattcgacgtaacgcctccaattgatattccaggagaggtgaaaaatatgatggagctcgcagagattgatactatgataccgttcgatctttccgctaccaagaaaaatacgatggagatgtaccgcgtgagactgtccgataagccacacaccgatgacccaatactgtgtttaagtttgtctccagcttccgacccacgtctctctcataccatgttaggggagatacttaactattatactcattgggccgggtcattaaagtttaccttcctgttttgcgggtctatgatggccaccgggaagctgctagttagctatgccccacctggtgcggatcctcctaaaaagagaaaagaagcaatgctcggtacccacgtaatttgggatattggactgcaatcgagctgcaccatggtggtgccttggatatctaatacaacctacagacagacaatcgacgactcattcacagagggtgggtatatatcggtgttttatcagacccgaatcgttgtgccattgtccacccctcgggaaatggatatccttggcttcgtgagtgcttgcaacgacttttcagtgagactactaagggacactacgcatattgaacagaaggcactggctcaaggcctgggccaaatgctcgagtcaatgatcgataataccgtgagagagaccgtaggtgcagcgacctcaagggacgcgttgcctaataccgaggcgtccgggccgactcacagtaaagagataccagcgttaacagcagtcgaaaccggtgcgactaatcccttggtgccaagcgatacagtgcaaacaaggcacgtagtccagcaccgatccaggtcggaaagctctatcgagtccttttttgctaggggggcttgtgtcactataatgacagtcgacaatccggcatcaacaaccaacaaagacaagttattcgctgtatggaaaattacctacaaggacaccgtccaactgagacggaagttagaattctttacatactcacggttcgacatggaattgactttcgtagtgaccgctaactttaccgaaaccaataacggtcacgccctgaatcaggtataccagatcatgtacgtccctcctggggcaccagttccggagaaatgggatgactatacttggcagacatctagcaaccctagcattttctacacttatggtaccgcccccgctagaattagtgtgccttacgtaggaatttcaaacgcatatagccatttctacgacggattctcaaaggtgccattaaaggatcagagcgcggccttgggggattcgttgtacggagccgcttcattgaacgatttcgggatactagcagtcagggtcgtgaacgaccataaccctactaaagtgacatcgaagatacgcgtctaccttaagccaaaacacatcagggtgtggtgtcctaggccgccaagagccgtcgcctattatggtcccggtgtcgattataaagacggaaccctgaccccattgtcaactaaagacctaaccacttatggattcggacaccaaaacaaagcggtgtacactgcaggttacaaaatttgcaactaccacttggccactcaggatgatttgcaaaacgcagtgaacgtcatgtggagtagagacctcttagtcacagaatcaagagcccagggcaccgattcaatcgcaaggtgcaattgcaacgcaggggtgtactactgcgagtctagaaggaaatactacccagtatccttcgttggcccaacgttccagtacatggaggctaataactattacccagctaggtaccagtcccatatgctcattggccatggattcgcatctccaggggattgtggtggcatactcagatgtcaccacggggtgatagggatcattactgctggtggagaagggttggttgcattttcagacattagagacttgtatgcctacgaagaagaagccatggaacaaggcctcaccaattacatagagtcacttggggccgcatttggaagtggatttactcagcagattagcgacaaaataacagagttgaccaatatggtgaccagtaccatcactgaaaagctacttaagaacttgatcaagatcatatcctcactagttattataactaggaactatgaagacaccacaacagtgctcgctaccctggcccttcttgggtgtgatgcttcaccatggcagtggcttagaaagaaagcatgcgatgttctggagataccttatgtcatcaagcaaggtgacagttggttgaagaagtttactgaagcatgcaacgcagctaagggactggagtgggtgtcaaacaaaatctcaaaattcattgattggctcaaggagaaaattatcccacaagctagagataagttggaatttgtaacaaaacttagacaactagaaatgctggaaaaccaaatctcaactatacaccaatcatgccctagtcaggaacaccaggaaattctattcaataatgtcagatggttatccatccagtctaagaggtttgcccctctttacgcagtggaagccaaaagaatacagaaactcgagcatactattaacaactacatacagttcaagagcaaacaccgtattgaaccagtatgtttgctagtacatggcagccccggaacaggtaaatctgtagcaaccaacctgattgctagagccatagctgaaagagaaaacacgtccacgtactcgctacccccggatccatcacacttcgacggatacaaacaacagggagtggtgattatggacgacctgaatcaaaacccagatggtgcggacatgaagctgttctgtcagatggtatcaacagtggagtttataccacccatggcatccctggaggagaaaggaatcctgtttacttcaaattacgttctagcatccacaaactcaagcagaatttccccccccactgtggcacacagtgacgcgttagccaggcgctttgcgttcgacatggacattcaggtcatgaatgagtattctagagatgggaaattgaacatggccatggctactgaaatgtgtaagaactgtcaccaaccagcaaactttaagagatgctgtcctttagtgtgtggtaaggcaattcaattaatggacaaatcttccagagttagatacagtattgaccagatcactacaatgattatcaatgagagaaacagaagatccaacattggcaattgtatggaggctttgtttcaaggaccactccagtataaagacttgaaaattgacatcaagacgagtccccctcctgaatgtatcaatgacttgctccaagcagttgactcccaggaggtgagagattactgtgagaagaagggttggatagttaacatcaccagccaggttcaaacagaaaggaacatcaacagggcaatgacaattctacaagcggtgacaaccttcgccgcagtggctggagttgtctatgtcatgtataaactgtttgctggacaccagggagcatacactggtttaccaaacaaaaaacccaacgtgcccaccattcggacagcaaaggtacaaggaccagggttcgattacgcagtggctatggctaaaagaaacattgttacagcaactactagcaagggagagttcactatgttaggagtccacgacaacgtggctattttaccaacccacgcttcacctggtgaaagcattgtgatcgatggcaaagaagtggagatcttggatgccaaagcgctcgaagatcaagcaggaaccaatcttgaaatcactataatcactctaaagagaaatgaaaagttcagagacattagaccacatatacctactcaaatcactgagacaaatgatggagtcttgatcgtgaacactagcaagtaccccaatatgtatgttcctgtcggtgctgtgactgaacagggatatctaaatctcggtgggcgccaaactgctcgtactctaatgtacaactttccaaccagagcaggacagtgtggtggagtcatcacatgtactgggaaagtcatcgggatgcatgttggtgggaacggttcacacgggtttgcagcggccctgaagcgatcatacttcactcagagtcaaggtgaaatccagtggatgagaccttcgaaggaagtgggatatccaatcataaatgccccgtccaaaaccaagcttgaacccagtgctttccactatgtgtttgaaggggtgaaggaaccagcagtcctcactaaaaacgatcccaggcttaagacagactttgaggaggcaattttctccaagtacgtgggtaacaaaattactgaagtggatgagtacatgaaagaggcagtagaccactatgctggccagctcatgtcactagacatcaacatagaacaaatgtgcttggaggatgccatgtatggcactgatggtctagaagcacttgatttgtccaccagtgctggctacccttatgtagcaatgggaaagaagaagagagacatcttgaacaaacaaaccagagacactaaggaaatgcaaaaactgctcgacacatatggaatcaacctcccactggtgacttatgtaaaggatgaacttagatccaaaacaaaggttgagcaggggaaatccagattaattgaagcttctagtttgaatgactcagtggcaatgagaatggcttttgggaacctatatgctgcttttcacaaaaacccaggagtgataacaggttcagcagtggggtgcgatccagatttgttttggagcaaaattccggtattgatggaagagaagctgtttgcttttgactacacagggtatgatgcatctctcagccctgcttggttcgaggcactaaagatggtgcttgagaaaatcggattcggagacagagttgactacatcgactacctaaaccactcacaccacctgtacaagaataaaacatactgtgtcaagggcggtatgccatctggctgctcaggcacttcaatttttaactcaatgattaacaacttgattatcaggacactcttactgaaaacctacaagggcatagatttagaccacctaaaaatgattgcctatggtgatgatgtaattgcttcctacccccatgaagttgacgctagtctcctagcccaatcaggaaaagactatggactaactatgactccagctgacaaatcagctacatttgaaacagtcacatgggagaatgtaacattcttgaagagattcttcagggcagacgagaaatacccatttcttattcatccagtaatgccaatgaaggaaattcatgaatcaattagatggacaaaagatcctaggaacactcaggatcacgttcgctctctgtgccttttagcttggcacaatggcgaagaagaatataacaaattcctagctaaaatcaggagtgtgccaattggaagagctttattgctcccagagtactcaacattgtaccgccgttggcttgactcattttagtaaccctacctcagtcgaattggattgggtcatactggtgtaggggtaaatttttctttaattcggagg

SEQ ID NO: 7 - DNA, 32 bp, Unknown
  synthetic
gcactgataatgaactcctctggatctactgg

SEQ ID NO: 8 - DNA, 32 bp, Unknown
  synthetic
ccagtagatccagaggagttcattatcagtgc

SEQ ID NO: 9 - DNA, 50 bp, Unknown
  synthetic
caagaattcctgaccacatacggtgctcaggtttcatcacagaaagtggg

SEQ ID NO: 10 - DNA, 50 bp, synthetic
caagaattcctgaccacatacggtgcgcaagtatcgtcgcaaaaagtagg

SEQ ID NO: 11 - DNA, 40 bp, Unknown
  synthetic
ttcgaattctccatatgtggtcagatccttggtggagagg

SEQ ID NO: 12 - DNA, 41 bp, Unknown
  synthetic
ttcgaattctccatacgtcgttaaatctttcgtcgataacg

SEQ ID NO: 13 - DNA, 2341 bp, Influenza virus
agcgaaagcaggcaaaccatttgaatggatgtcaatccgaccttacttttcttaaaagtgccagcacaaaatgctataagcacaactttcccttatactggagaccctccttacagccatgggacaggaacaggatacaccatggatactgtcaacaggacacatcagtactcagaaaagggaagatggacaacaaacaccgaaactggagcaccgcaactcaacccgattgatgggccactgccagaagacaatgaaccaagtggttatgcccaaacagattgtgtattggaagcaatggctttccttgaggaatcccatcctggtatttttgaaaactcgtgtattgaaacgatggaggttgttcagcaaacacgagtagacaagctgacacaaggccgacagacctatgactggactctaaatagaaaccaacctgctgcaacagcattggccaacacaatagaagtgttcagatcaaatggcctcacggccaatgagtctggaaggctcatagacttccttaaggatgtaatggagtcaatgaaaaaagaagaaatggggatcacaactcattttcagagaaagagacgggtgagagacaatatgactaagaaaatgataacacagagaacaataggtaaaaagaagcagagattgaacaaaaggagttatctaattagagcattgaccctgaacacaatgaccaaagatgctgagagagggaagctaaaacggagagcaattgcaaccccagggatgcaaataagggggtttgtatactttgttgagacactggcaaggagtatatgtgagaaacttgaacaatcagggttgccagttggaggcaatgagaagaaagcaaagttggcaaatgttgtaaggaagatgatgaccaattctcaggacaccgaactttctttcaccatcactggagataacaccaaatggaacgaaaatcagaatcctcggatgtttttggccatgatcacatatatgacaagaaatcagcccgaatggttcagaaatgttctaagtattgctccaataatgttctcaaacaaaatggcgagactgggaaaagggtatatgtttgagagcaagagtatgaaacttagaactcaaatacctgcagaaatgctagcaagcatcgatttgaaatatttcaatgattcaacaagaaagaagattgaaaaaatccgaccgctcttaatagaggggactgcatcattgagccctggaatgatgatgggcatgttcaatatgttaagcactgtattaggcgtctccatcctgaatcttggacaaaagagatacaccaagactacttactggtgggatggtcttcaatcctctgacgattttgctctgattgtgaatgcacccaatcatgaagggattcaagccggagtcgacaggttttatcgaacctgtaagctacttggaatcaatatgagcaagaaaaagtcttacataaacagaacaggtacatttgaattcacaagttttttctatcgttatgggtttgttgccaatttcagcatggagctccccagttttggggtgtctgggatcaacgagtcagcggacatgagtattggagttactgtcatcaaaaacaatatgataaacaatgatcttggtccagcaacagctcaaatggcccttcagttgttcatcaaagattacaggtacacgtaccgatgccatagaggtgacacacaaatacaaacccgaagatcatttgaaataaagaaactgtgggagcaaacccgttccaaagctggactgctggtctccgacggaggcccaaatttatacaacattagaaatctccacattcctgaagtctgcctaaaatgggaattgatggatgaggattaccaggggcgtttatgcaacccactgaacccatttgtcagccataaagaaattgaatcaatgaacaatgcagtgatgatgccagcacatggtccagccaaaaacatggagtatgatgctgttgcaacaacacactcctggatccccaaaagaaatcgatccatcttgaatacaagtcaaagaggagtacttgaagatgaacaaatgtaccaaaggtgctgcaatttatttgaaaaattcttccccagcagttcatacagaagaccagtcgggatatccagtatggtggaggctatggtttccagagcccgaattgatgcacggattgatttcgaatctggaaggataaagaaagaagagttcactgagatcatgaagatctgttccaccattgaagagctcagacggcaaaaatagtgaatttagcttgtccttcatgaaaaaatgccttgtttctact

SEQ ID NO: 14 - DNA, 2341 bp, unknown
  synthetic
agcgaaagcaggcaaaccatttgaatggatgtcaatccgaccttacttttcttaaaagtgccagcacaaaatgctataagcacaactttcccttatactggagaccctccttacagccatgggacaggaacaggatacaccatggatactgtcaacaggacacatcagtactcagaaaagggaagatggacaacaaacaccgaaactggagcaccgcaactcaacccgattgatgggccactgccagaagacaatgaaccaagtggttatgcccaaacagattgtgtattggaagcaatggctttccttgaggaatcccatcctggtatttttgaaaactcgtgtattgaaacgatggaggttgttcagcaaacacgagtagacaagctgacacaaggccgacagacctatgactggactctaaatagaaaccaacctgctgcaacagcattggccaacacaatagaagtgttcagatcaaatggcctcacggccaatgagtctggaaggctcatagacttccttaaggacgttatggagtctatgaaaaaagaggaaatggggattacgacacattttcaacgaaaaagacgggttagggataatatgacaaaaaaaatgattacgcaacgaacaatcggaaagaaaaaacagagactgaataagcgatcatacttgattagggcacttacacttaacactatgactaaggacgccgaaaggggaaagctaaagcgtagagcaattgcaacacccggaatgcaaattagggggttcgtatacttcgtcgagacactcgctagatccatatgcgaaaagttagagcaatccggactgccagtcggggggaacgaaaaaaaagcgaaactcgctaacgtcgttagaaaaatgatgactaatagtcaggataccgaactgtcatttacgattaccggcgataatactaagtggaacgagaatcagaatcctagaatgtttctcgcaatgatcacatatatgacacgtaaccaacccgaatggtttagaaacgtactgtcaatcgcaccaattatgtttagcaataagatggctagattgggcaaggggtatatgtttgaatctaagagtatgaaattgcgaacacagatacctgccgaaatgctagcatcaatcgatctaaagtactttaacgatagtacacgaaaaaaaatcgaaaagattagaccgttactgatagagggaaccgccagcctatcccccggaatgatgatggggatgtttaatatgcttagtaccgtgttaggcgttagcatacttaacttagggcaaaaacgttatactaagactacatattggtgggacggactgcaatctagcgacgatttcgcactaatcgttaacgcacctaaccatgaggggatacaagccggagtcgatagattctatagaacatgcaaactgttagggattaatatgtctaaaaaaaagtcatacataaatagaaccggaacatttgaattcactagctttttttacagatacggattcgttgctaattttagtatggagttacctagtttcggagttagcggaattaacgaatccgccgatatgtcaatcggcgtaaccgttattaagaataatatgattaataacgatctagggccagcaaccgcacaaatggcattgcagttgttcataaaggattatcgttatacatatagatgtcatagaggcgatacacagatacagactagacgatcatttgaaatcaaaaaattgtgggagcaaactaggtctaaagccggactgttagtgtccgacggagggcctaatctatacaatattaggaatctgcatatacccgaagtgtgtctaaagtgggagcttatggacgaagactatcaggggagattgtgcaatccgcttaacccattcgttagccataaagagatagagtcaatgaataacgccgttatgatgccagcacacggacccgctaagaatatggaatacgacgcagtcgcaactacacatagttggataccgaaacggaatcgatccatactgaatacatcccaaagaggcgtactcgaagacgaacaaatgtaccaacggtgttgcaatctatttgaaaaattttttcctagtagtagctatagacgaccagtcgggatatccagtatggtggaggctatggtttccagagcccgaattgatgcacggattgatttcgaatctggaaggataaagaaagaagagttcactgagatcatgaagatctgttccaccattgaagagctcagacggcaaaaatagtgaatttagcttgtccttcatgaaaaaatgccttgtttctact

SEQ ID NO: 15 - DNA, 2341 bp, unknown
  synthetic
agcgaaagcaggcaaaccatttgaatggatgtcaatccgaccttacttttcttaaaagtgccagcacaaaatgctataagcacaactttcccttatactggagaccctccttacagccatgggacaggaacaggatacaccatggatactgtcaacaggacacatcagtactcagaaaagggaagatggacaacaaacaccgaaactggagcaccgcaactcaacccgattgatgggccactgccagaagacaatgaaccaagtggttatgcccaaacagattgtgtattggaagcaatggctttccttgaggaatcccatcctggtatttttgaaaactcgtgtattgaaacgatggaggttgttcagcaaacacgagtagacaagctgacacaaggccgacagacctatgactggactctaaatagaaaccaacctgctgcaacagcattggccaacacaatagaagtgttcagatcaaatggcctcacggccaatgagtctggaaggctcatagacttccttaaggacgttatggagtctatgaaaaaagaggaaatggggattacgacacattttcaacgaaaaagacgggttagggataatatgacaaaaaaaatgattacgcaacgaacaatcggaaagaaaaaacagagactgaataagcgatcatacttgattagggcacttacacttaacactatgactaaggacgccgaaaggggaaagctaaagcgtagagcaattgcaacacccggaatgcaaattagggggttcgtatacttcgtcgagacactcgctagatccatatgcgaaaagttagagcaatccggactgccagtcggggggaacgaaaaaaaagcgaaactcgctaacgtcgttagaaaaatgatgactaatagtcaggataccgaactgtcatttacgattaccggcgataatactaagtggaacgagaatcagaatcctagaatgtttctcgcaatgatcacatatatgacacgtaaccaacccgaatggtttagaaacgtactgtcaatcgcaccaattatgtttagcaataagatggctagattgggcaaggggtatatgtttgaatctaagagtatgaaattgcgaacacagatacctgccgaaatgctagcatcaatcgatctaaagtactttaacgatagtacacgaaaaaaaatcgaaaagattagaccgttactgatagagggaaccgccagcctatcccccggaatgatgatggggatgtttaatatgcttagtaccgtgttaggcgttagcatacttaacttagggcaaaaacgttatactaagactacatattggtgggacggactgcaatctagcgacgatttcgcactaatcgttaacgcacctaaccatgaggggatacaagccggagtcgatagattctatagaacatgcaaactgttagggattaatatgtctaaaaaaaagtcatacataaatagaaccggaacatttgaattcacaagttttttctatcgttatgggtttgttgccaatttcagcatggagctccccagttttggggtgtctgggatcaacgagtcagcggacatgagtattggagttactgtcatcaaaaacaatatgataaacaatgatcttggtccagcaacagctcaaatggcccttcagttgttcatcaaagattacaggtacacgtaccgatgccatagaggtgacacacaaatacaaacccgaagatcatttgaaataaagaaactgtgggagcaaacccgttccaaagctggactgctggtctccgacggaggcccaaatttatacaacattagaaatctccacattcctgaagtctgcctaaaatgggaattgatggatgaggattaccaggggcgtttatgcaacccactgaacccatttgtcagccataaagaaattgaatcaatgaacaatgcagtgatgatgccagcacatggtccagccaaaaacatggagtatgatgctgttgcaacaacacactcctggatccccaaaagaaatcgatccatcttgaatacaagtcaaagaggagtacttgaagatgaacaaatgtaccaaaggtgctgcaatttatttgaaaaattcttccccagcagttcatacagaagaccagtcgggatatccagtatggtggaggctatggtttccagagcccgaattgatgcacggattgatttcgaatctggaaggataaagaaagaagagttcactgagatcatgaagatctgttccaccattgaagagctcagacggcaaaaatagtgaatttagcttgtccttcatgaaaaaatgccttgtttctact

SEQ ID NO: 16 - DNA, 2341 bp, Influenza virus
agcgaaagcaggtcaattatattcaatatggaaagaataaaagaactaagaaatctaatgtcgcagtctcgcacccgcgagatactcacaaaaaccaccgtggaccatatggccataatcaagaagtacacatcaggaagacaggagaagaacccagcacttaggatgaaatggatgatggcaatgaaatatccaattacagcagacaagaggataacggaaatgattcctgagagaaatgagcaaggacaaactttatggagtaaaatgaatgatgcaggatcagaccgagtgatggtatcacctctggctgtgacatggtggaataggaatggaccaataacaaatacagttcattatccaaaaatctacaaaacttattttgaaagagtcgaaaggctaaagcatggaacctttggccctgtccattttagaaaccaagtcaaaatacgtcggagagttgacataaatcctggtcatgcagatctcagtgccaaggaggcacaggatgtaatcatggaagttgttttccctaacgaagtgggagccaggatactaacatcggaatcgcaactaacgataaccaaagagaagaaagaagaactccaggattgcaaaatttctcctttgatggttgcatacatgttggagagagaactggtccgcaaaacgagattcctcccagtggctggtggaacaagcagtgtgtacattgaagtgttgcatttgactcaaggaacatgctgggaacagatgtatactccaggaggggaagtgaggaatgatgatgttgatcaaagcttgattattgctgctaggaacatagtgagaagagctgcagtatcagcagatccactagcatctttattggagatgtgccacagcacacagattggtggaattaggatggtagacatccttaggcagaacccaacagaagagcaagccgtggatatatgcaaggctgcaatgggactgagaattagctcatccttcagttttggtggattcacatttaagagaacaagcggatcatcagtcaagagagaggaagaggtgcttacgggcaatcttcaaacattgaagataagagtgcatgagggatatgaagagttcacaatggttgggagaagagcaacagccatactcagaaaagcaaccaggagattgattcagctgatagtgagtgggagagacgaacagtcgattgccgaagcaataattgtggccatggtattttcacaagaggattgtatgataaaagcagtcagaggtgatctgaatttcgtcaatagggcgaatcagcgattgaatcctatgcatcaacttttaagacattttcagaaggatgcgaaagtgctttttcaaaattggggagttgaacctatcgacaatgtgatgggaatgattgggatattgccagacatgactccaagcatcgagatgtcaatgagaggagtgagaatcagcaaaatgggtgtagatgagtactccagcacggagagggtagtggtgagcattgaccgttttttgagaatccgggaccaacgaggaaatgtactactgtctcccgaggaggtcagtgaaacacagggaacagagaaactgacaataacttactcatcgtcaatgatgtgggagattaatggtcctgaatcagtgttggtcaatacctatcaatggatcatcagaaactgggaaactgttaaaattcagtggtcccagaaccctacaatgctatacaataaaatggaatttgaaccatttcagtctttagtacctaaggccattagaggccaatacagtgggtttgtaagaactctgttccaacaaatgagggatgtgcttgggacatttgataccgcacagataataaaacttcttcccttcgcagccgctccaccaaagcaaagtagaatgcagttctcctcatttactgtgaatgtgaggggatcaggaatgagaatacttgtaaggggcaattctcctgtattcaactataacaaggccacgaagagactcacagttctcggaaaggatgctggcactttaactgaagacccagatgaaggcacagctggagtggagtccgctgttctgaggggattcctcattctgggcaaagaagacaagagatatgggccagcactaagcatcaatgaactgagcaaccttgcgaaaggagagaaggctaatgtgctaattgggcaaggagacgtggtgttggtaatgaaacggaaacgggactctagcatacttactgacagccagacagcgaccaaaagaattcggatggccatcaattagtgtcgaatagtttaaaaacgaccttgtttctact

SEQ ID NO: 17 - DNA, 2341 bp, unknown
  synthetic
agcgaaagcaggtcaattatattcaatatggagagaatcaaagagcttaggaatcttatgtcacaatctagaactagagagatactgactaagactacagtcgatcatatggctataatcaaaaaatatactagcggaagacaggaaaaaaatcccgcacttagaatgaaatggatgatggctatgaaataccctattacagccgataagcgaattaccgaaatgataccagagagaaacgaacagggacagacattgtggtctaaaatgaacgacgccggatccgatagagtgatggtttcgccactagccgtaacatggtggaatagaaacggacctattacgaatacagtgcattaccctaagatatacaaaacatatttcgaaagagtcgagagactgaaacacggaacattcggaccagtgcattttcggaatcaggttaagattagacgtagagtcgatattaatccagggcatgcagatctctccgctaaagaggcacaagacgttattatggaggtcgtgtttcctaacgaggtcggcgctaggatactgactagcgaatcgcaattgacaattacgaaagagaaaaaagaggaactccaggattgcaaaattagcccacttatggtcgcatatatgctcgaacgcgaattggttagaaagactagattcctaccagtcgcaggcggaacgtctagcgtgtatatcgaagtgttgcatctaacacagggaacatgttgggagcaaatgtatactccaggaggcgaagtgagaaacgacgacgttgatcaatcgctaatcatagccgctaggaatatagtgagaagggcagccgttagcgcagacccacttgcgtcactactcgaaatgtgccatagtacgcaaatcggagggattagaatggtcgatatccttaggcagaatcctacagaggaacaggccgtagacatatgcaaagccgcaatgggattgcgaattagctcatcattctcattcggagggtttacgtttaaacggactagcggatctagcgtaaaacgcgaagaggaagtgcttactggcaatctgcaaacactaaagattagggtgcatgagggatacgaagagtttacaatggtcggacgtagagcaaccgctatacttagaaaagcgactaggagactgatacaattgatcgttagcggaagggacgaacagtcaatcgccgaagcgataatagtcgcaatggtgttttcgcaagaggattgcatgattaaggccgttaggggggatctgaatttcgttaatagggctaatcagagactgaatcctatgcatcaattgcttagacattttcagaaagacgctaaagtgttgtttcagaattggggagtcgaacctatcgataacgttatgggtatgatagggatactgccagatatgacaccatcaatcgaaatgtcaatgagaggcgttaggattagtaagatgggcgtagacgaatactccagcactgagagagtggtagtgtcaatcgatagatttcttaggattagggatcagagaggcaacgtactgctatcacccgaagaagttagcgaaacacagggaaccgaaaaattgacaattacgtatagtagtagtatgatgtgggagattaacggaccagagtcagtgttagtgaatacatatcaatggataatacggaattgggagacagtgaaaatacaatggtcacagaatcctacaatgctatacaataagatggagttcgaaccttttcaatcgttagtgcctaaggccataagaggccaatatagtgggttcgttagaacattgtttcagcaaatgagagacgtactcggaacattcgataccgcacagataattaagctattgccattcgcagccgcaccacctaagcaatctagaatgcaattttctagctttaccgttaacgttaggggatccggaatgcgaatactcgttagggggaatagtccagtgtttaattacaataaggcaactaagagattgacagtgttaggcaaggacgcaggaacattgaccgaagacccagacgagggaaccgctggagtggaatccgcagtgcttagggggtttctgatactcggaaaggaggataagagatacggacctgcactatcgattaacgaactatctaatctcgctaaaggcgaaaaagcgaatgtgttaatcggacagggagacgtagtgttagtgatgaaacggaaacgcgatagctcaatactgacagactcacaaaccgctactaagagaattcggatggcaattaattagtgtcgaatagtttaaaaacgaccttgtttctact

SEQ ID NO: 18 - DNA, 2233 bp, Influenza virus
agcgaaagcaggtactgatccaaaatggaagattttgtgcgacaatgcttcaatccgatgattgtcgagcttgcggaaaaaacaatgaaagagtatggggaggacctgaaaatcgaaacaaacaaatttgcagcaatatgcactcacttggaagtatgcttcatgtattcagattttcacttcatcaatgagcaaggcgagtcaataatcgtagaacttggtgatccaaatgcacttttgaagcacagatttgaaataatcgagggaagagatcgcacaatggcctggacagtagtaaacagtatttgcaacactacaggggctgagaaaccaaagtttctaccagatttgtatgattacaaggagaatagattcatcgaaattggagtaacaaggagagaagttcacatatactatctggaaaaggccaataaaattaaatctgagaaaacacacatccacattttctcgttcactggggaagaaatggccacaaaggcagactacactctcgatgaagaaagcagggctaggatcaaaaccagactattcaccataagacaagaaatggccagcagaggcctctgggattcctttcgtcagtccgagagaggagaagagacaattgaagaaaggtttgaaatcacaggaacaatgcgcaagcttgccgaccaaagtctcccgccgaacttctccagccttgaaaattttagagcctatgtggatggattcgaaccgaacggctacattgagggcaagctgtctcaaatgtccaaagaagtaaatgctagaattgaaccttttttgaaaacaacaccacgaccacttagacttccgaatgggcctccctgttctcagcggtccaaattcctgctgatggatgccttaaaattaagcattgaggacccaagtcatgaaggagagggaataccgctatatgatgcaatcaaatgcatgagaacattctttggatggaaggaacccaatgttgttaaaccacacgaaaagggaataaatccaaattatcttctgtcatggaagcaagtactggcagaactgcaggacattgagaatgaggagaaaattccaaagactaaaaatatgaagaaaacaagtcagctaaagtgggcacttggtgagaacatggcaccagaaaaggtagactttgacgactgtaaagatgtaggtgatttgaagcaatatgatagtgatgaaccagaattgaggtcgctagcaagttggattcagaatgagtttaacaaggcatgcgaactgacagattcaagctggatagagctcgatgagattggagaagatgtggctccaattgaacacattgcaagcatgagaaggaattatttcacatcagaggtgtctcactgcagagccacagaatacataatgaagggggtgtacatcaatactgccttgcttaatgcatcttgtgcagcaatggatgatttccaattaattccaatgataagcaagtgtagaactaaggagggaaggcgaaagaccaacttgtatggtttcatcataaaaggaagatcccacttaaggaatgacaccgacgtggtaaactttgtgagcatggagttttctctcactgacccaagacttgaaccacataaatgggagaagtactgtgttcttgagataggagatatgcttataagaagtgccataggccaggtttcaaggcccatgttcttgtatgtgagaacaaatggaacctcaaaaattaaaatgaaatggggaatggagatgaggcgttgcctcctccagtcacttcaacaaattgagagtatgattgaagctgagtcctctgtcaaagagaaagacatgaccaaagagttctttgagaacaaatcagaaacatggcccattggagagtcccccaaaggagtggaggaaagttccattgggaaggtctgcaggactttattagcaaagtcggtattcaacagcttgtatgcatctccacaactagaaggattttcagctgaatcaagaaaactgcttcttatcgttcaggctcttagggacaaccttgaacctgggacctttgatcttggggggctatatgaagcaattgaggagtgcctgattaatgatccctgggttttgcttaatgcttcttggttcaactccttccttacacatgcattgagttagttgtggcagtgctactatttgctatccatactgtccaaaaaagtaccttgtttctact

SEQ ID NO: 19 - DNA, 2233 bp, unknown
  synthetic
agcgaaagcaggtactgatccaaaatggaggatttcgttaggcaatgctttaatccaatgatagtcgagttagccgaaaagactatgaaagagtatggcgaagacctaaagattgagactaataaattcgccgcaatttgcacacaccttgaggtttgctttatgtattccgattttcactttattaacgaacagggagagtcaattatagtcgagttaggcgatccgaacgcattgctaaagcatagatttgaaattatagagggacgcgataggacaatggcatggaccgtagttaattcgatttgcaatacaaccggagccgaaaaaccgaaattcttacccgatctatacgattataaagagaataggtttatcgaaatcggagtgactagacgcgaagtgcatatttattatctcgaaaaagcgaataagattaagtccgaaaagacacacatacacatttttagctttaccggagaggaaatggcaacaaaagccgattatacacttgacgaagagtctagggctaggattaagactagactgtttacaattagacaggaaatggctagtagggggttgtgggatagctttagacaatccgaaagaggcgaagagacaatcgaagagagatttgaaattaccggaacaatgcgaaagcttgccgatcaatccctaccccccaatttctctagccttgagaattttagggcatacgttgacggattcgaacctaacggatatatagagggaaagctatcgcaaatgtctaaagaggttaacgctagaatcgaaccattcctaaagacaacacctagaccacttagactgccaaacggaccaccatgctcacagcgatctaagtttctgcttatggacgcactaaagttgtcaatcgaagacccatcacacgagggagaggggataccattgtacgacgcaattaagtgtatgcgaacatttttcggatggaaagagcctaacgtagtgaaaccacacgaaaaagggattaatccgaattatctgcttagttggaaacaggtgttagccgaattgcaggatatcgaaaacgaagagaaaattccgaaaactaagaatatgaaaaaaactagccaactgaaatgggcacttggcgagaatatggcacccgaaaaagtcgatttcgacgattgcaaagacgtcggcgatctaaagcaatacgatagcgacgaacccgaacttagatcactcgctagttggatacagaacgagttcaataaggcatgcgaattgaccgatagctcatggatagagcttgacgagataggcgaagacgtagcaccaatcgaacacatagcctctatgagacggaattattttacatccgaagtgtcacattgtagggcaacagagtatattatgaaaggggtgtatattaataccgcattgcttaacgctagttgcgccgcaatggacgatttccaactgataccgatgatctcgaagtgtagaacaaaagagggacgtagaaagactaatctgtatgggttcattattaagggaaggtctcatttaaggaacgatacagacgtagtgaatttcgttagtatggagtttagccttaccgatccgagactcgaaccacacaaatgggaaaagtattgcgtactagagataggggatatgttgattagatccgcaatcggacaggtttcgagaccaatgtttttgtacgttaggactaacggaacctcgaagattaaaatgaaatggggaatggagatgcgtagatgcctattgcaatcccttcagcaaatcgaatctatgatagaggccgaatctagcgttaaagagaaagatatgacaaaagagttttttgaaaataagtccgaaacatggccaatcggagagtcaccaaaaggggttgaggaatcctcaatcggaaaagtttgtagaacattgctcgcaaaatccgtattcaatagtctatacgccagcccacaactagagggattctctgctgagtcacgaaaactgttactgatagtgcaagcccttagggataatctcgaacccggaacattcgatctaggggggttgtacgaagcaatcgaagagtgtctgattaacgatccatgggtactgcttaacgctagttggtttaattcgttccttacacacgcactatcttagttgtggcagtgctactatttgctatccatactgtccaaaaaagtaccttgtttctact

SEQ ID NO: 20 - DNA, 1775 bp, Influenza virus
agcaaaagcaggggaaaataaaaacaaccaaaatgaaggcaaacctactggtcctgttaagtgcacttgcagctgcagatgcagacacaatatgtataggctaccatgcgaacaattcaaccgacactgttgacacagtactcgagaagaatgtgacagtgacacactctgttaacctgctcgaagacagccacaacggaaaactatgtagattaaaaggaatagccccactacaattggggaaatgtaacatcgccggatggctcttgggaaacccagaatgcgacccactgcttccagtgagatcatggtcctacattgtagaaacaccaaactctgagaatggaatatgttatccaggagatttcatcgactatgaggagctgagggagcaattgagctcagtgtcatcattcgaaagattcgaaatatttcccaaagaaagctcatggcccaaccacaacacaaacggagtaacggcagcatgctcccatgaggggaaaagcagtttttacagaaatttgctatggctgacggagaaggagggctcatacccaaagctgaaaaattcttatgtgaacaaaaaagggaaagaagtccttgtactgtggggtattcatcacccgcctaacagtaaggaacaacagaatatctatcagaatgaaaatgcttatgtctctgtagtgacttcaaattataacaggagatttaccccggaaatagcagaaagacccaaagtaagagatcaagctgggaggatgaactattactggaccttgctaaaacccggagacacaataatatttgaggcaaatggaaatctaatagcaccaatgtatgctttcgcactgagtagaggctttgggtccggcatcatcacctcaaacgcatcaatgcatgagtgtaacacgaagtgtcaaacacccctgggagctataaacagcagtctcccttaccagaatatacacccagtcacaataggagagtgcccaaaatacgtcaggagtgccaaattgaggatggttacaggactaaggaacactccgtccattcaatccagaggtctatttggagccattgccggttttattgaagggggatggactggaatgatagatggatggtatggttatcatcatcagaatgaacagggatcaggctatgcagcggatcaaaaaagcacacaaaatgccattaacgggattacaaacaaggtgaacactgttatcgagaaaatgaacattcaattcacagctgtgggtaaagaattcaacaaattagaaaaaaggatggaaaatttaaataaaaaagttgatgatggatttctggacatttggacatataatgcagaattgttagttctactggaaaatgaaaggactctggatttccatgactcaaatgtgaagaatctgtatgagaaagtaaaaagccaattaaagaataatgccaaagaaatcggaaatggatgttttgagttctaccacaagtgtgacaatgaatgcatggaaagtgtaagaaatgggacttatgattatcccaaatattcagaagagtcaaagttgaacagggaaaaggtagatggagtgaaattggaatcaatggggatctatcagattctggcgatctactcaactgtcgccagttcactggtgcttttggtctccctgggggcaatcagtttctggatgtgttctaatggatctttgcagtgcagaatatgcatctgagattagaatttcagaaatatgaggaaaaacacccttgtttctact

SEQ ID NO: 21 - DNA, 1775 bp, unknown
  synthetic
agcaaaagcaggggaaaataaaaacaaccaaaatgaaggcaaacctactggtcctgttaagtgcacttgcagctgcagatgcagacacaatatgtataggctaccatgcgaacaattcaaccgacactgttgacacagtactcgagaagaatgtgacagtgacacactctgttaacctgttagaggactcacataacggaaagctatgtaggcttaagggaatcgcaccactgcaattgggcaagtgtaatatagccggatggttgttggggaatcccgaatgcgatccactgttacccgttaggtcatggtcatatatagtcgagacacctaatagcgaaaacggaatttgttatcccggcgattttatcgattacgaagagcttagagagcaattgtctagcgttagttcattcgaaagattcgaaatttttccgaaagagtctagttggccaaatcataatactaacggagtgactgccgcatgctcacacgaaggcaagtctagcttttataggaatctgttgtggttgactgagaaagagggatcatatccgaaactgaaaaactcatacgtgaacaaaaagggaaaggaagtgttagtgttgtgggggatacaccatccaccaaatagtaaagagcaacagaatatatatcagaacgaaaacgcatacgttagcgtcgtaactagtaattataatagaaggtttacacccgaaatcgcagagagaccgaaagttagagaccaagccggaagaatgaattattattggacactactgaaacccggcgatacaattatattcgaagcgaacggaaatctgatcgcaccgatgtatgcattcgcactatctagggggttcggatccggaattattactagtaacgctagtatgcacgaatgtaacacgaagtgtcagactccactaggcgcaattaactctagtctgccatatcagaatatacatcccgtaacaatcggcgaatgcccaaaatacgttagatccgctaagcttagaatggttaccggactgagaaatacaccatcaatccaatctagggggttgttcggagcgatagccggatttatcgaaggggggtggacagggatgatagacggttggtacggatatcatcaccaaaacgaacagggatccggatacgcagccgatcagaaatcgacgcaaaacgctattaacggaattactaataaagtgaataccgtaatcgaaaaaatgaatatccaatttaccgcagtcggaaaggaattcaataagcttgagaaaagaatggagaatctgaataaaaaagtcgacgacggatttctagacatatggacttataacgccgaactgttagtgttgctcgaaaacgaaagaacactagactttcacgactcaaacgttaagaatctatacgaaaaagtgaaatcccaattgaaaaataacgctaaagagatagggaacggatgtttcgagttctatcataaatgcgataacgaatgtatggaatccgttaggaacggaacatacgattatcctaagtatagcgaagagtcaaaactgaatagggagaaagtcgacggagtgaaactcgaatcaatggggatatatcagatactggcaatctatagtacagtcgccagctcactggttcttttggtctccctgggggcaatcagtttctggatgtgttctaatggatctttgcagtgcagaatatgcatctgagattagaatttcagaaatatgaggaaaaacacccttgtttctact

SEQ ID NO: 22 - DNA, 1565 bp, Influenza virus
agcaaaagcagggtagataatcactcactgagtgacatcaaaatcatggcgtcccaaggcaccaaacggtcttacgaacagatggagactgatggagaacgccagaatgccactgaaatcagagcatccgtcggaaaaatgattggtggaattggacgattctacatccaaatgtgcaccgaactcaaactcagtgattatgagggacggttgatccaaaacagcttaacaatagagagaatggtgctctctgcttttgacgaaaggagaaataaatacctggaagaacatcccagtgcggggaaagatcctaagaaaactggaggacctatatacaggagagtaaacggaaagtggatgagagaactcatcctttatgacaaagaagaaataaggcgaatctggcgccaagctaataatggtgacgatgcaacggctggtctgactcacatgatgatctggcattccaatttgaatgatgcaacttatcagaggacaagagctcttgttcgcaccggaatggatcccaggatgtgctctctgatgcaaggttcaactctccctaggaggtctggagccgcaggtgctgcagtcaaaggagttggaacaatggtgatggaattggtcaggatgatcaaacgtgggatcaatgatcggaacttctggaggggtgagaatggacgaaaaacaagaattgcttatgaaagaatgtgcaacattctcaaagggaaatttcaaactgctgcacaaaaagcaatgatggatcaagtgagagagagccggaacccagggaatgctgagttcgaagatctcacttttctagcacggtctgcactcatattgagagggtcggttgctcacaagtcctgcctgcctgcctgtgtgtatggacctgccgtagccagtgggtacgactttgaaagagagggatactctctagtcggaatagaccctttcagactgcttcaaaacagccaagtgtacagcctaatcagaccaaatgagaatccagcacacaagagtcaactggtgtggatggcatgccattctgccgcatttgaagatctaagagtattaagcttcatcaaagggacgaaggtgctcccaagagggaagctttccactagaggagttcaaattgcttccaatgaaaatatggagactatggaatcaagtacacttgaactgagaagcaggtactgggccataaggaccagaagtggaggaaacaccaatcaacagagggcatctgcgggccaaatcagcatacaacctacgttctcagtacagagaaatctcccttttgacagaacaaccattatggcagcattcaatgggaatacagagggaagaacatctgacatgaggaccgaaatcataaggatgatggaaagtgcaagaccagaagatgtgtctttccaggggcggggagtcttcgagctctcggacgaaaaggcagcgagcccgatcgtgccttcctttgacatgagtaatgaaggatcttatttcttcggagacaatgcagaggagtacgacaattaaagaaaaatacccttgtttctact

SEQ ID NO: 23 - DNA, 1565 bp, unknown
  synthetic
agcaaaagcagggtagataatcactcactgagtgacatcaaaatcatggcgtcccaaggcaccaaacggtcttacgaacagatggagactgatggagaacgccagaatgccactgaaatcagagctagcgtcggaaaaatgatagggggaatcggaaggttttacatacaaatgtgtaccgaactcaaattgtccgattacgaagggagattgatccaaaatagtctgacaatcgaaagaatggtgttaagcgcattcgacgaaagacggaataagtatctcgaagagcatcctagcgcaggcaaggatccaaaaaaaaccggagggccaatctataggagagtgaacggaaagtggatgcgcgaactgatactgtacgataaagaggagattagacggatatggcgacaagcgaataacggagacgacgctactgccggactgacacatatgatgatatggcactctaatcttaacgacgctacataccaacggactagggcactcgttagaaccggaatggatcctagaatgtgctcacttatgcagggatctacactccctagacgatccggagccgcaggagcagccgttaagggagtcggaactatggttatggaactcgttagaatgataaaaagggggattaacgataggaatttttggagaggcgaaaacggacgtaaaactagaatcgcatacgaaagaatgtgcaatatactcaaagggaaattccaaaccgcagcgcaaaaagctatgatggatcaagttagggagtctaggaatccaggaaatgccgaattcgaagaccttacatttctcgctcggtccgcactaatccttcgcggatcagtcgcacacaaatcttgcttacccgcatgcgtatacggacctgcagtcgctagcggatacgatttcgaacgcgaagggtatagtctagtaggaattgatccatttagattgctccaaaattcgcaagtgtatagtctgattagacctaacgagaatcctgcacacaaatctcaactcgtatggatggcatgccatagtgccgcattcgaagaccttagagtgctatctttcataaagggaacgaaagtgttgcctaggggaaagctatctactaggggagtgcaaatcgctagtaacgagaatatggagactatggagtctagtacactcgaactgagatctagatattgggctattaggactagatccggagggaatacgaatcagcaacgagctagcgccgggcaaatctcaatccaacctacattttccgtgcaacggaatctgccattcgatcggacaacgattatggccgcattcaatgggaataccgagggacggactagcgatatgagaaccgaaattatcagaatgatggaatccgctagaccagaggacgtttcgtttcaaggacggggagtcttcgagctctcggacgaaaaggcagcgagcccgatcgtgccttcctttgacatgagtaatgaaggatcttatttcttcggagacaatgcagaggagtacgacaattaaagaaaaatacccttgtttctact

SEQ ID NO: 24 - DNA, 1413 bp, Influenza virus
agcgaaagcaggggtttaaaatgaatccaaatcagaaaataacaaccattggatcaatctgtctggtagtcggactaattagcctaatattgcaaatagggaatataatctcaatatggattagccattcaattcaaactggaagtcaaaaccatactggaatatgcaaccaaaacatcattacctataaaaatagcacctgggtaaaggacacaacttcagtgatattaaccggcaattcatctctttgtcccatccgtgggtgggctatatacagcaaagacaatagcataagaattggttccaaaggagacgtttttgtcataagagagccctttatttcatgttctcacttggaatgcaggaccttttttctgacccaaggtgccttactgaatgacaagcattcaaatgggactgttaaggacagaagcccttatagggccttaatgagctgccctgtcggtgaagctccgtccccgtacaattcaagatttgaatcggttgcttggtcagcaagtgcatgtcatgatggcatgggctggctaacaatcggaatttcaggtccagataatggagcagtggctgtattaaaatacaacggcataataactgaaaccataaaaagttggaggaagaaaatattgaggacacaagagtctgaatgtgcctgtgtaaatggttcatgttttactataatgactgatggcccgagtgatgggctggcctcgtacaaaattttcaagatcgaaaaggggaaggttactaaatcaatagagttgaatgcacctaattctcactatgaggaatgttcctgttaccctgataccggcaaagtgatgtgtgtgtgcagagacaactggcatggttcgaaccggccatgggtgtctttcgatcaaaacctggattatcaaataggatacatctgcagtggggttttcggtgacaacccgcgtcccgaagatggaacaggcagctgtggtccagtgtatgttgatggagcaaacggagtaaagggattttcatataggtatggtaatggtgtttggataggaaggaccaaaagtcacagttccagacatgggtttgagatgatttgggatcctaatggatggacagagactgatagtaagttctctgttaggcaagatgttgtggcaatgactgattggtcagggtatagcggaagtttcgttcaacatcctgagctaacagggctagactgtatgaggccgtgcttctgggttgaattaatcaggggacgacctaaagaaaaaacaatctggactagtgcgagcagcatttctttttgtggcgtgaatagtgatactgtagattggtcttggccagacggtgctgagttgccattcagcattgacaagtagtctgttcaaaaaactccttgtttctact

SEQ ID NO: 25 - DNA, 1413 bp, unknown
  synthetic
agcgaaagcaggggtttaaaatgaatccaaatcagaaaataacaaccattggatcaatctgtctggtagtcggactaattagcctaatattgcaaatagggaatataatctcaatatggatttcgcattcaatccaaaccggatcacaaaatcatacaggcatatgcaatcagaatataattacttataaaaatagtacatgggtgaaagatactactagcgtgatactaaccggcaattctagtctatgtccgattagggggtgggctatatactctaaagacaatagtatacggatagggtctaagggagacgttttcgtaattagggaaccgtttataagttgttcacatctagagtgtaggaccttttttctgacacaaggcgcactattaaacgataagcattctaacggtacagttaaggataggtcaccttatagggcacttatgtcatgtcccgtaggcgaagcccctagtccatacaatagtagatttgaatccgttgcatggtccgctagcgcatgtcacgacggaatggggtggttgactatagggattagcggacccgataacggagccgttgccgtactgaaatataacggtataattaccgaaactattaagagttggcgtaaaaaaatattgcgtacacaagagtccgaatgcgcatgcgttaacggatcatgttttacaattatgactgacggacctagcgacgggttagcgtcatacaaaatttttaaaatcgaaaaaggcaaggttactaagtcaatcgagttaaacgcacctaattcgcattacgaagagtgttcatgttatcccgataccggaaaggttatgtgcgtttgtagggataattggcacggttcgaacagaccttgggtgtcattcgatcaaaatctagactatcaaatcggatatatatgtagcggagtgttcggcgataatcctagaccagaggacggtacaggcagctgtggaccggtttacgttgacggcgctaacggcgttaaggggtttagttatagatacggcaatggcgtatggatcggtaggactaagtcacatagttctagacacggatttgaaatgatatgggatcctaacggatggaccgaaaccgactcgaagtttagcgttaggcaagacgtagtcgctatgaccgattggtccgggtatagcggatcattcgtgcaacatccagagttaaccggattggattgtatgcgaccatgtttttgggttgagttgattagggggagaccgaaagagaaaactatatggactagcgcgagcagcatttctttttgtggcgtgaatagtgatactgtagattggtcttggccagacggtgctgagttgccattcagcattgacaagtagtctgttcaaaaaactccttgtttctact

SEQ ID NO: 26 - DNA, 1026 bp, Influenza virus
agcgaaagcaggtagatattgaaagatgagtcttctaaccgaggtcgaaacgtacgtactctctatcatcccgtcaggccccctcaaagccgagatcgcacagagacttgaagatgtctttgcagggaagaacactgatcttgaggttctcatggaatggctaaagacaagaccaatcctgtcacctctgactaaggggattttaggatttgtgttcacgctcaccgtgcccagtgagcgaggactgcagcgtagacgctttgtccaaaatgcccttaatgggaacggggatccaaataacatggacaaagcagttaaactgtataggaagctcaagagggagataacattccatggggccaaagaaatctcactcagttattctgctggtgcacttgccagttgtatgggcctcatatacaacaggatgggggctgtgaccactgaagtggcatttggcctggtatgtgcaacctgtgaacagattgctgactcccagcatcggtctcataggcaaatggtgacaacaaccaatccactaatcagacatgagaacagaatggttttagccagcactacagctaaggctatggagcaaatggctggatcgagtgagcaagcagcagaggccatggaggttgctagtcaggctagacaaatggtgcaagcgatgagaaccattgggactcatcctagctccagtgctggtctgaaaaatgatcttcttgaaaatttgcaggcctatcagaaacgaatgggggtgcagatgcaacggttcaagtgatcctctcgctattgccgcaaatatcattgggatcttgcacttgacattgtggattcttgatcgtctttttttcaaatgcatttaccgtcgctttaaatacggactgaaaggagggccttctacggaaggagtgccaaagtctatgagggaagaatatcgaaaggaacagcagagtgctgtggatgctgacgatggtcattttgtcagcatagagctggagtaaaaaactaccttgtttctac

SEQ ID NO: 27 - DNA, 890 bp, Influenza virus
agcaaaagcagggtgacaaagacataatggatccaaacactgtgtcaagctttcaggtagattgctttctttggcatgtccgcaaacgagttgcagaccaagaactaggtgatgccccattccttgatcggcttcgccgagatcagaaatccctaagaggaaggggcagcaccctcggtctggacatcgagacagccacacgtgctggaaagcagatagtggagcggattctgaaagaagaatccgatgaggcacttaaaatgaccatggcctctgtacctgcgtcgcgttacctaactgacatgactcttgaggaaatgtcaagggactggtccatgctcatacccaagcagaaagtggcaggccctctttgtatcagaatggaccaggcgatcatggataagaacatcatactgaaagcgaacttcagtgtgatttttgaccggctggagactctaatattgctaagggctttcaccgaagagggagcaattgttggcgaaatttcaccattgccttctcttccaggacatactgctgaggatgtcaaaaatgcagttggagtcctcatcgggggacttgaatggaatgataacacagttcgagtctctgaaactctacagagattcgcttggagaagcagtaatgagaatgggagacctccactcactccaaaacagaaacgagaaatggcgggaacaattaggtcagaagtttgaagaaataagatggttgattgaagaagtgagacacaaactgaagataacagagaatagttttgagcaaataacatttatgcaagccttacatctattgcttgaagtggagcaagagataagaactttctcgtttcagcttatttaataataaaaaacacccttgtttctact

SEQ ID NO: 28 - DNA, 890 bp, unknown
  synthetic
agcaaaagcagggtgacaaagacataatggatccaaacactgtgtcaagctttcaggtagattgctttctttggcatgtccgcaaacgagttgcagaccaagaactaggtgatgccccattccttgaccgactgagacgggatcagaaatcccttaggggcaggggatcgaccctaggcctagacatcgaaaccgcaactagggccggaaagcagatcgtggagcgtatactgaaagaggagtccgacgaagcgcttaagatgactatggccagcgtacccgctagtcggtaccttaccgatatgacactcgaagagatgtcacgcgattggtctatgctaatccctaagcagaaagtggccggacctctatgtatacggatggaccaggcgattatggacaaaaacattatccttaaagcgaacttttccgtgatattcgatcgcctagagactctgatactgttgcgtgcattcacagaagagggagcaattgttggcgaaatttcaccattgccttctcttccaggacatactgctgaggatgtcaaaaatgcagttggagtcctcatcgggggacttgaatggaatgataacacagttcgagtctctgaaactctacagagattcgcttggagaagcagtaatgagaatgggagacctccactcactccaaaacagaaacgagaaatggcgggaacaattaggtcagaagtttgaagaaataagatggttgattgaagaagtgagacacaaactgaagataacagagaatagttttgagcaaataacatttatgcaagccttacatctattgcttgaagtggagcaagagataagaactttctcgtttcagcttatttaataataaaaaacacccttgtttctact

SEQ ID NO: 29 - DNA, 7152 bp, Human rhinovirus 89
ttaaaactgggagtgggttgttcccactcactccacccatgcggtgttgtactctgttattacggtaactttgtacgccagtttttcccacccttccccataatgtaacttagaagtttgtacaatatgaccaataggtgacaatcatccagactgtcaaaggtcaagcacttctgtttccccggtcaatgaggatatgctttacccaaggcaaaaaccttagagatcgttatccccacactgcctacacagagcccagtaccatttttgatataattgggttggtcgctccctgcaaacccagcagtagacctggcagatgaggctggacattccccactggcgacagtggtccagcctgcgtggctgcctgctcacccttcttgggtgagaagcctaattattgacaaggtgtgaagagccgcgtgtgctcagtgtgcttcctccggcccctgaatgtggctaaccttaaccctgcagccgttgcccataatccaatgggtttgcggtcgtaatgcgtaagtgcgggatgggaccaactactttgggtgtccgtgtttcctgtttttcttttgattgcattttatggtgacaatttatagtgtatagattgtcatcatgggtgcacaagtatctagacaaaatgttgggacacactccacacaaaattcagtgagcaatggatctagcttaaattatttcaacatcaattattttaaagacgcagcttcaagtggtgcttctagattggatttttctcaagaccctagtaaatttactgatcctgttaaagatgtgttagaaaagggtattccaacacttcaatcaccaacagttgaagcttgtggttattcagacagactaatacagataacccgaggagattccactataacatcccaagatactgcaaatgcagttgttgcttatggtgtgtggccatcatacttgactccagatgatgcgactgctattgacaaacccacacaacctgatacatcatccaacagattctacaccttggacagtcgttcttggacatctgcctcatctggatggtggtggaaattgcctgatgcccttaaaaacatgggtatatttggtgaaaatatgttttaccattttctagggagatctggatacacaatacatgtacaatgtaattctagcaagtttcatcagggtttattaatagttgccgccatcccagaacatcaattggcatctgcaacaagtggaaatgtatcagtcgggtacaatcacacccacccaggtgagcaaggtagagaagtagtaccatcacggacatctagtgataataaaagacctagtgatgacagttggttaaattttgatggaacattacttggtaacttacctatttatccccaccaatacattaatctaaggactaacaattcagctacccttattttaccttatgtcaatgctgtaccaatggactctatgcttagacataataattggagcttggttataatcccaatatgccctcttcaggtccaacctggggggacacaatccatacctataacagtatcaattagccctatgttttcagaattttcagggccaagaagtaaggttgtgtttagtaccactcagggtttaccagttatgttaacacctggatctgggcaattcttaacaactgatgatactcaatccccatcagcgtttccatacttccacccgaccaaggaaatatttatacctggacaagttaggaatttaattgaaatgtgccaagttgacacactcattcctgttaacaatacacaggaaaatgtaagatctgtgaatatgtacactgttgatttacgcacacaagttgatttagctaaagaagtcttttctataccagtagatattgcctcacaacctttagccactactctcataggagaacttgcaagctattacacacactggactggtagtctgcgctttagctttatgttttgtggttctgctagctctactttgaaactattaattgcatacactcctcctggtgttggaaaacctaaatccaggagagaagccatgcttggtacacatttagtgtgggatgtggggttgcagtccaccgcctcactagttgtaccatgggttagtgctagccattttagattcactacacctgacacatattcctcagctggttatattacatgctggtaccagaccaactttgtagtacctgatagtactccagataacgccaaaatggtgtgcatggtttctgcatgcaaagatttttgcttaagattagccagagatactaacctacacacacaagaaggagtactcacacaaaacccagttgaaaattatatagatagtgtattaaatgaagttcttgtggtgccaaatatccaacctagcacatctgtgtcaagtcatgcagcgcctgcattggatgctgcggaaaccggacacaccagctctgttcaacctgaagatatgattgaaactagatatgttataactgatcaaacaagggatgaaacaagtattgagagtttcttaggtaggtcagggtgtatcgctatgatagaatttaatacaagtagtgataaaactgaacatgataaaattggtaaaggattcaaaacatggaaggttagtcttcaagaaatggcacaaatcagaagaaaatatgaattattcacatatacaagatttgattcagagataacaatagtcactgcagccgcagctcaaggaaatgatagtggacatatagtattgcaatttatgtatgtacccccaggagcacctgtccccgaaaaacgtgatgattacacatggcaatcaggaacaaatgcatctgtgttctggcaagaaggacaaccataccccagattcacaatcccttttatgagcattgcatcagcctattacatgttttatgatggttatgatggtgatagtgcagcatcaaaatacggttctgtagtcactaatgatatgggaaccatatgtgttagaatagtgacatccaaccaaaaacacgattcaaatattgtgtgccgcatttaccacaaggccaaacatataaaagcatggtgtcctcgcccaccaagggctgttgcctatcaacacacacactcaaccaattacataccatccaatggtgaggccacaactcagattaaaaccagacctgatgtttttaccgttacaaacgtcggaccatctagtatgtttgtacatgtgggtaacttaatctatagaaatcttcatctctttaattctgatcttgatgattctattcttgtatcatactccagtgatctaatcatatatcgaacaaacactgaaggtaatgatgtgatccctaattgtgattgcactgaatgtacatattactgccaccacaaagataggtattttcctatcagagttactgcacatgattggtatgagattcaagaatcagaatattacccaaaacatatccaatataatctcctgattggagagggtccttgtgaaccaggagattgtggaggaaaactattgtgtaaacatggtgttataggtatgattacagctggaggtgaaggtcacgttgcttttattgacctgagaaaattccagtgtgctgaggagcaagggttatctgattatgtggaacatcttggtcaagtctttggtgtaggcttcgtagacagcatcaaacaacaggtaaactttatcaaccccactagtaaaattggttcaaaagtgattaaatggttgttgaggatagtttcagctatgataataatggtaaggaatagttctgatccacaaactgtaattgccactctcacccttctaggttgttcaggctcaccatggaggtttcttaaagagaaactctgtgcgtggctccagcttagctatgtacataagcagtctgattcatggctcaagaaatttactgaagcgtgtaacgcagcacgtgggctagagtggattggacaaaagatatctaaatttatagattggataaagagtatgttaccacaggctcaattgaaaattgattacctaaccaaattaaaacaacttaatctcttagagaaacaaatagaaacaattagacttgcacctgctagtgttcaggagaaaattttcattgaaataaacacccttcatgatttatccttaaaattcttaccactgtatgcatctgaagcacgtagaattaagaatttatatatcaaatgcagtaatgttattaaagggggaaagaggaatgaaccagttgcagttctaatacatggttctcctggtactggaaaatctcttgccacttctgttcttgctcgaatgctaactgttgagactgatatatattctttgcccccagatcctaaatattttgatgggtatgatcaacagagtgttgttatcatggatgatatcatgcaaaatcctagtggtgaagacatgactttgttttgccaaatggtatcgagtgtccctttcatacctcctatggcagatcttccagataaaggaaaaccatttacatccaagtttgtacttgcaagcactaatcacactctactaacaccaccaacagtatcttcattaccagcaatggcaagaaggttttactttgatctagacattcaagttaagaaagagtatcttttagatggcaaactagatatagcaaaaagctttcgaccatgtgatgttaatattaaaataggcaatgctaagtgctgtccatttatctgtggaaaagctgtagagtttaaagatagaaattcatgtacaaccttgtctttatctcaattgtatagtcatataaaggaagaagataggagaagaagcagtgcagcacaagcaatggaggctatatttcaaggtatagacctccaatctcctccacctccagccatagctgacctccttaggtctgtgaaaacaccagagatcattaagtattgccaagataataattggattgttccagcagagtgttctattgaaagagatttagggatagcaaatatgactataggtataatagctaatgtggtctctatagtaggtgttatctatataatttataaattgttctgtacacttcagggtccatactcaggggaacctaaacccaaaagcagagctccagagagaagagtagttactcagggcccagaggaagagtttggtcgctcactactcaaacataattgctgtgttgtgacaaccgacaaaggcaaattcacaggtcttggcatatatgaccaagtcatggtacttccaacacattctgacccaggctctgagatcttggtagatggagtaaaagttaaggtctctgattcctatgatttgcataaccatgagggtgttaagctagagatcacagttgtgaaattaattagaaatgagaagtttaaagacatcagaaaatatttaccctcacgtgaagatgactatcctgcttgtaaccttgccttactagctaatcaagatgagccaacaataataagtgttggtgatgcagtatcttatggtaacatcttattgagtggtaccaatactgcacgaatgatcaagtaccattacccgacaaaagctggatattgtgggggtgttttgtacaaggttggctctattcttggtatacatgttggtggcaatggtagagatggattttctgcaatgcttctcaaatcttattttggtgaaacccagggtttaatcactaaagaacttcctgtatctgtaaagaacttaccatccgtacatgtttcatctaaaacccgactacaacctagtgtttttcatgatgttttccctggaacaaaagagcctgcagttcttagtagtaatgatccaagactagaaactgactttgactcagcacttttctccaaatataaaggtaatcctgcttgtcaagtgaccccacacatgaaaattgctgtagcacattatgcagcacagttatctacactagacataaatcctcaacccctttcattggaagagagtgtgtttggtattgagggattagaagctttggatttaaatactagtgcaggatttccttatgtttcactgggaataaagaagaaagatcttatagataaaaagaccaaagacatcacaaaacttaggaaagcaattgatgaatatggtattgatttgcctatggttacttttctgaaagatgaacttagaaagaaggaaaaaataaaagatggaaagactagagtcatagaagctaatagtgtgaatgatactgtgttattcagaagtgtatttggaaatcttttctctgctttccacaaaaacccaggtatagtcactggttcagcagtagggtgtgaccctgaagtattctggtcaactatacctctcatgctagatggagaatgtttaatggcttttgattattcaaactatgatggtagcctacatcccgtttggtttaaatgtcttagtatgctcttagaagacataggtttctcctctcaacttattaaccagatctgtaactctaaacatatatacaaatctaagtattatgaagtggaaggaggtatgccatctggatgtgctggtactagtatttttaatacaataatcaacaatattatcattagaactttggtactagatgcttataagaacatagatctagataaactgaaaatcttagcatatggggatgatgtcatcttttcttataattttaaacttgacatggcagttcttgccaaagaaggagaaaaatatggactaacaatcacccctgctgataagtctgatgttttccaagaattgacctataaaaatgtaacttttcttaaaagaggattcagagctgatgagcgccactctttccttatacaccctacctttcctgtggctgagattcatgactccatcagatggaccaaaaacccttcatgtatgcaggaacacgtgctatctttgtgtcatttaatgtggcataatggtagacatgcataccaggaattcattaaaggtatacgcagtgtatctgccggtcgggcactgtatataccagcttatgaagttcttgaacatgaatggtatgaaaaattttagatataaaactgttaaatatagctagtttattagttttat

SEQ ID NO: 30 - DNA, 7152 bp, unknown
  synthetic
ttaaaactgggagtgggttgttcccactcactccacccatgcggtgttgtactctgttattacggtaactttgtacgccagtttttcccacccttccccataatgtaacttagaagtttgtacaatatgaccaataggtgacaatcatccagactgtcaaaggtcaagcacttctgtttccccggtcaatgaggatatgctttacccaaggcaaaaaccttagagatcgttatccccacactgcctacacagagcccagtaccatttttgatataattgggttggtcgctccctgcaaacccagcagtagacctggcagatgaggctggacattccccactggcgacagtggtccagcctgcgtggctgcctgctcacccttcttgggtgagaagcctaattattgacaaggtgtgaagagccgcgtgtgctcagtgtgcttcctccggcccctgaatgtggctaaccttaaccctgcagccgttgcccataatccaatgggtttgcggtcgtaatgcgtaagtgcgggatgggaccaactactttgggtgtccgtgtttcctgtttttcttttgattgcattttatggtgacaatttatagtgtatagattgtcatcatgggagcacaagtgtctagacaaaacgtaggtacacatagtacacaaaactcagtgtctaacggatctagtcttaattattttaatattaattattttaaagacgctgcatctagcggagctagtagacttgattttagtcaggatccatctaaatttaccgatccagttaaagacgtactcgaaaaaggtatacctacattgcaatcacctacagtcgaagcatgcggatactctgatagattgatacaaattactaggggggatagtactattactagtcaggataccgctaacgccgtagtcgcatacggagtttggccatcttatcttacacctgatgacgcaaccgcaatcgataaacctacacaacctgatactagttctaatagattctatacacttgattctagatcatggactagtgctagttcaggttggtggtggaaattgcctgacgcacttaaaaatatgggtatattcggtgagaatatgttttatcatttcttaggtaggtcagggtatactatacacgttcaatgtaatagttctaaatttcaccaaggtctattaatcgttgccgctatacccgaacaccaattagctagcgctacatcaggtaacgttagcgtagggtataatcatacacatccaggcgaacagggtagggaagtcgtaccatctagaacatctagcgataataaacgaccatctgacgatagttggcttaatttcgatggtacactattaggtaatctacctatatatccacatcaatatattaatcttagaactaataattccgctacacttatactgccatacgttaacgcagtgcctatggatagtatgcttagacataataattggtcattagtgattataccgatatgtccattgcaagtgcaacctggaggtacacaatctatacctattaccgttagtattagtcctatgtttagcgaatttagcggacctagatctaaggtagtgtttagtactacacaggggttacccgttatgcttacacctggatcaggtcaatttttgactactgacgatacacaatcacctagtgcattcccatattttcaccctactaaagagatttttatacccggtcaggttaggaatctaatcgaaatgtgtcaagtcgatacacttatacccgttaataatacacaggaaaacgttagatccgttaatatgtataccgttgatttgcgtacacaagtcgatctagctaaagaggttttttcgataccagtcgatatcgctagtcaaccattagctactacacttataggcgaactcgcatcatattatacacattggaccggatcacttagattttcttttatgttttgcggatccgctagtagtacacttaaactgttaatcgcatatacacctccaggagtgggtaagcctaaatctagacgcgaagctatgttaggtacacatctagtttgggacgtagggttacaatctaccgctagtttagtcgtaccatgggttagcgcatcacattttagatttactacacctgatacttattctagtgccggatatataacatgttggtatcaaactaatttcgtagtgccagatagtacacctgataacgctaaaatggtttgtatggttagcgcatgtaaagatttttgtcttagattagctagggatactaatttgcatacacaagagggagtgcttacacaaaatccagtcgaaaattatatcgatagcgtacttaacgaagtgttagtcgtacctaatatacaacctagtactagtgtgtcatctcacgctgcaccagcattagacgcagccgaaaccggacatacatctagtgtgcaacctgaggatatgatagagactagatacgttattaccgatcagactagagacgaaacatcaatcgaatcattcttaggtaggtcagggtgtatcgctatgatagagtttaatactagttccgataaaaccgaacacgataagataggtaaggggtttaaaacttggaaagtgtcattgcaggaaatggcacaaattagacgtaaatacgaattgtttacatatactagattcgatagtgagattactatcgttaccgcagccgcagcacaaggtaacgattcaggtcatatagtgttacaatttatgtacgtaccaccaggtgcaccagtacccgaaaaacgcgatgattatacatggcaatccggtactaacgctagcgttttttggcaagagggacaaccatatcctagatttactataccttttatgtcaatcgctagtgcatattatatgttttacgacggatacgatggcgattctgccgcatctaaatacggatctgtagtgactaacgatatgggtactatatgcgttagaatcgttacatctaatcaaaaacacgattctaatatcgtttgtagaatatatcataaagctaaacatattaaggcatggtgtcctagaccacctagagccgttgcatatcaacatacacatagtactaattatataccatctaacggtgaggctactacacaaattaaaactagacctgacgtttttaccgttactaacgtaggtccatctagtatgttcgtacacgtaggtaatctgatatatagaaatttgcatctattcaattccgatttagacgattctatactcgttagttattctagcgatctgattatatatagaactaataccgaaggtaacgatgtgatacctaattgcgattgtaccgaatgtacttattattgtcatcataaagataggtattttccgatacgcgttaccgcacacgattggtacgaaatacaggaatctgagtattatcctaaacatatacaatataatctgttaataggcgaaggtccatgcgaaccaggcgattgcggaggtaagttattgtgtaaacacggagtgataggtatgattaccgcagggggagagggacacgttgcgtttatcgatttgcgaaaatttcaatgcgcagaggaacaggggttatccgattacgttgagcatttagggcaagtgttcggagtcggattcgttgattcaattaaacaacaggttaattttattaatcctacatctaaaatcggatctaaagtgataaaatggttacttagaatcgttagcgctatgataattatggttaggaattctagcgatccacaaaccgtaatcgctacacttacactattagggtgttcaggttcaccttggcgatttcttaaagagaaattatgcgcatggttgcaattgtcatacgttcataaacaatccgatagttggcttaaaaaatttaccgaagcatgtaacgccgctaggggactcgaatggatagggcaaaaaatatctaaatttatcgattggattaaatctatgttaccacaagcgcaattgaaaatcgattatcttactaagcttaaacaattgaacttactcgaaaaacaaatcgaaactattagactcgcaccagctagtgtgcaagagaaaatttttatagagattaatacattacacgatctatcacttaaattcttaccattatacgctagcgaagctagacggattaaaaatctatatattaagtgttctaacgtaattaagggaggtaagcgtaacgaacccgttgccgtacttatacacggatcaccaggtaccggtaagtcattagcgactagcgtactcgctagaatgcttacagtcgaaaccgatatatactctttaccacctgatcctaaatatttcgacggatacgatcaacaatccgtagtgattatggacgatattatgcaaaatcctagtggtgaggatatgacattgttttgtcaaatggtatctagcgtaccatttataccacctatggccgatttacccgataagggtaagccttttacatctaaattcgtactcgcatcaactaatcatacattgcttacaccacctaccgttagttcactaccagctatggctagacggttttatttcgatctagatatacaggttaaaaaagagtatctgttagacggtaagttagatatcgctaaatcttttagaccatgcgatgttaatattaaaatcggtaacgctaaatgttgtccatttatatgcggtaaggcagtcgaatttaaagataggaattcatgtactacactatcactatcacaattgtattcacatattaaggaagaggatagacgtagatctagtgccgcacaagctatggaagctatttttcagggtatcgatctgcaatcaccaccaccaccagctatagccgatctacttagatccgttaaaacacctgagataattaagtattgtcaggataataattggatcgtaccagccgaatgttcaatcgaacgcgatttagggatagcgaatatgacaatcggtataatcgctaacgtagtgtcaatcgtaggcgttatatatattatatataaattgttttgtacattgcagggaccatactctggcgaacctaaacctaaatctagagcacctgaaagacgcgtagtgacacagggacctgaagaggaattcggtaggtcattgcttaaacataattgttgcgtagtgactaccgataagggtaagtttaccggattaggtatatacgatcaggttatggtgttacctacacattccgatccaggatctgagatactcgtagacggagttaaggttaaggttagcgattcatacgatctacataatcacgaaggcgttaagttagagattaccgtagttaagcttatacgtaacgaaaaatttaaagatatacgaaaatatctaccatcacgcgaagacgattatcctgcatgtaatctcgcactattagcgaatcaagacgaacctacaattattagcgtaggcgatgccgtatcatacggtaatatactgttatccggtactaataccgctagaatgattaagtatcattatcctactaaagccggatattgcggaggagtgttatataaagtcggatctatactcggtatacacgtaggcggtaacggtagggacggattttccgctatgttacttaaatcttatttcggtgagacacagggattgattactaaagagttacccgtatccgttaaaaatctacctagcgtacacgttagttctaaaactagattgcaacctagtgtgtttcacgacgtttttccaggtactaaggaacctgccgtactatcttctaacgatcctagactcgaaaccgatttcgatagtgcattattctctaaatataagggtaatcctgcatgtcaggttacaccacatatgaaaatcgcagtcgcacattacgctgcacaattgtctacacttgatattaatccacaaccactatcacttgaggaatccgtattcggtatcgaagggttagaggcacttgatcttaatactagtgccggattcccatacgttagtctaggtattaaaaaaaaagatctaatcgataaaaaaactaaggatattactaaattgcgaaaagcgatagacgaatacggtatcgatctacctatggttacattccttaaagacgaacttagaaaaaaagagaaaattaaagacggtaagactagggttatcgaagctaactctgttaacgataccgtactttttagatccgtattcggtaatctattttccgcattccataaaaatccaggtatcgttaccggatccgcagtcggatgcgatccagaagtgttttggtctactataccacttatgttagacggtgagtgtcttatggcattcgattattctaattacgatgggtcattgcatcccgtatggtttaaatgtctatctatgttactcgaagatatagggtttagttcacaattgattaatcagatttgtaactctaaacatatatataaatctaaatattacgaagtcgaagggggtatgccatcaggttgcgcaggtacatctatttttaatactataattaataatattataattagaacattagtgttagacgcatataaaaatatcgatctagataagcttaagatactcgcatacggagatgacgttatattctcatataattttaaacttgatatggccgtactcgctaaagagggagaaaaatacggacttacaattacacctgccgataagtctgacgtttttcaggaattgacttataaaaacgttacattccttaaaagggggtttcgcgcagacgaacgacattcttttcttatacatcctacatttcccgttgccgaaatacacgattcaattagatggactaaaaatcctagttgtatgcaagaacacgtacttagtctatgtcatcttatgtggcataacggtagacacgcttatcaggaatttattaagggtattagatccgttagtgccggtagggcactatatatacccgcatacgaagtactcgaacacgaatggtacgaaaaattttagatataaaactgttaaatatagctagtttattagttttat

SEQ ID NO: 31 - DNA, 7212 bp, Human rhinovirus 14
ttaaaacagcggatgggtatcccaccattcgacccattgggtgtagtactctggtactatgtacctttgtacgcctgtttctccccaaccacccttccttaaaattcccacccatgaaacgttagaagcttgacattaaagtacaataggtggcgccatatccaatggtgtctatgtacaagcacttctgtttcccaggagcgaggtataggctgtacccactgccaaaagcctttaaccgttatccgccaaccaactacgtaacagttagtaccatcttgttcttgactggacgttcgatcaggtggattttccctccactagtttggtcgatgaggctaggaattccccacgggtgaccgtgtcctagcctgcgtggcggccaacccagcttatgctgggacgcccttttaaggacatggtgtgaagactcgcatgtgcttggttgtgagtcctccggcccctgaatgcggctaaccttaaccctagagccttatgccacgatccagtggttgtaaggtcgtaatgagcaattccgggacgggaccgactactttgggtgtccgtgtttctcatttttcttcatattgtcttatggtcacagcatatatatacatatactgtgatcatgggcgctcaggtttctacacagaaaagtggatctcacgaaaatcaaaacattttgaccaatggatcaaatcagactttcacagttataaattactataaggatgcagcaagtacatcatcagctggtcaatcactgtcaatggacccatctaagtttacagaaccagttaaagatctcatgcttaagggtgcaccagcattgaattcacccaatgttgaggcctgtggttatagtgatagagtacaacaaatcacactcgggaattcaacaataacaacacaagaagcagccaacgctgttgtgtgttatgctgaatggccagagtaccttccagatgtggacgctagtgatgtcaataaaacttcaaaaccagacacttctgtctgtaggttttacacattggatagtaagacatggacaacaggttctaaaggctggtgctggaaattaccagatgcactcaaggatatgggtgtgttcgggcaaaacatgtttttccactcactaggaagatcaggttacacagtacacgttcagtgcaatgccacaaaattccatagcggttgtctacttgtagttgtaataccagaacaccaactggcttcacatgagggtggcaatgtttcagttaaatacacattcacgcatccaggtgaacgtggtatagatttatcatctgcaaatgaagtgggagggcctgtcaaggatgtcatatacaatatgaatggtactttattaggaaatctgctcattttccctcaccagttcattaatctaagaaccaataatacagccacaatagtgataccatacataaactcagtacccattgattcaatgacacgtcacaacaatgtctcactgatggtcatccctattgcccctcttacagtaccaactggagcaactccctcactccctataacagtcacaatagcacctatgtgcactgagttctctgggataaggtccaagtcaattgtgccacaaggtttgccaactacaactttgccggggtcaggacaattcttgaccacagatgacaggcaatcccccagtgcactgccaaattatgagccaactccaagaatacacatactagggaaagttcataacttgctagaaattatacaggtagatacactcattcctatgaacaacacgcatacaaaagatgaggttaacagttacctcataccactaaatgcaaacaggcaaaatgagcaggtttttgggacaaacctgtttattggtgatggggtcttcaaaactactcttctgggtgaaattgttcagtactatacacattggtctggatcacttagattctcttcgatgtatactggtcctgccttgtccagtgctaaactcactctagcatacaccccgcctggtgctcgtggtccacaggacaggagagaagcaatgctaggtactcatgttgtctgggatattggtctgcaatccaccatagtaatgacaataccatggacatcaggggtgcagtttagatatactgatccagatacatacaccagtgctggctttctatcatgttggtatcaaacttctcttatacttcccccagaaacgaccggccaggtctacttattatcattcataagtgcatgtccagattttaagcttaggctgatgaaagatactcaaactatctcacagactgttgcactcactgaaggcttaggtgatgaattagaagaagtcatcgttgagaaaacgaaacagacggtggcctcaatctcatctggtccaaaacacacacaaaaagtccccatactaactgcaaacgaaacaggggccacaatgcctgttcttccatcagacagcatagaaaccagaactacctacatgcactttaatggttcagaaactgatgtagaatgctttttgggtcgtgcagcttgtgtgcatgtaactgaaatacaaaacaaagatgctactggaatagataatcacagagaagcaaaattgttcaatgattggaaaatcaacctgtccagccttgtccaacttagaaagaaactggaactcttcacttatgttaggtttgattctgagtataccatactggccactgcatctcaacctgattcagcaaactattcaagcaatttggtggtccaagccatgtatgttccacatggtgccccgaaatccaaaagagtgggcgattacacatggcaaagtgcttcaaaccccagtgtattcttcaaggtgggggatacatcaaggtttagtgtgccttatgtaggattggcatcagcatataattgtttttatgatggttactcacatgatgatgcagaaactcagtatggcataactgttctaaaccatatgggtagtatggcattcagaatagtaaatgaacatgatgaacacaaaactcttgtcaagatcagagtttatcacagggcaaagctcgttgaagcatggattccaagagcacccagagcactaccctacacatcaatagggcgcacaaattatcctaagaatacagaaccagtaattaagaagaggaaaggtgacattaaatcctatggtttaggacctaggtacggtgggatttatacatcaaatgttaaaataatgaattaccacttgatgacaccagaagaccaccataatctgatagcaccctatccaaatagagatttagcaatagtctcaacaggaggacatggtgcagaaacaataccacactgtaaccgtacatcaggtgtttactattccacatattacagaaagtattaccccataatttgcgaaaagcccaccaacatctggattgaaggaagcccttattacccaagtagatttcaagcaggagtgatgaaaggggttgggccggcagagctaggagactgcggtgggattttgagatgcatacatggtcccattggattgttaacagctgaaggtagtggatatgtttgttttgctgacatacgacagttggagtgtatcgcagaggaacaggggctgagtgattacatcacaggtttgggtagagcttttggtgtcgggttcactgaccaaatctcaacaaaagtcacagaactacaagaagtggcgaaagatttcctcaccacaaaagttttgtccaaagtggtcaaaatggtttcagctttagtgatcatttgcagaaatcatgatgacttggtcactgttacggccactctagcactacttggatgtgatggatctccttggagatttctgaagatgtacatttccaaacactttcaggtgccttacattgaaagacaagcaaatgatggatggttcagaaagtttaatgatgcatgtaatgctgcaaagggattggaatggattgctaataagatttccaaactgattgaatggataaaaaacaaagtacttccccaagccaaagaaaaactagaattttgtagtaaactcaaacaacttgatatactagagagacaaataaccaccatgcatatctcgaatccaacacaggaaaaacgagagcagttgttcaataacgtattgtggttggaacaaatgtcgcaaaagtttgccccattttatgccgttgaatcaaaaagaatcagggaactcaagaacaaaatggtaaattatatgcaatttaaaagtaaacaaagaactgaaccagtgtgtgtattaatccatggtacacccggttctggtaaatcattaacaacatccattgtgggacgtgcaattgcagaacacttcaattcagcagtatattcacttccaccagatcccaagcactttgatggttatcagcaacaggaagttgtgattatggatgatctgaaccaaaatccagatggacaggatataagcatgttttgtcaaatggtttcttcagtggatttcttgcctccaatggctagtttagataacaagggcatgttattcaccagtaattttgttctagcctccacaaattctaacacactaagccccccaacaatcttgaatcctgaagctttagtcaggagatttggttttgacctagatatatgtttgcatactacctacacaaagaatggaaaactcaatgcaggcatgtcaaccaagacatgcaaagattgccatcaaccatctaatttcaagaaatgttgccccctagtctgtggaaaagctattagcttggtagacagaactaccaacgttaggtatagtgtggatcaactggtcacggctattataagtgatttcaagagcaaaatgcaaattacagattccctagaaacactgtttcaaggaccagtgtataaagatttagagattgatgtttgcaacacaccaccttcagaatgtatcaacgatttactgaaatctgtagattcagaagagattagggaatattgtaagaagaagaaatggattatacctgaaattcctaccaacatagaaagggctatgaatcaagccagcatgattattaatactattctgatgtttgtcagtacattaggtattgtttatgtcatttataaattgtttgctcaaactcaaggaccatattctggtaacccgcctcacaataaactaaaagccccaactttacgcccagttgttgtgcaaggaccaaacacagaatttgcactatccctgttaaggaaaaacataatgactataacaacctcaaagggagagttcacagggttaggcatacatgatcgtgtctgtgtgatacccacacacgcacagcctggtgatgatgtactagtgaatggtcagaaaattagagttaaggataagtacaaattagtagatccagagaacattaatctagagcttacagtgttgactttagatagaaatgaaaaattcagagatatcaggggatttatatcagaagatctagaaggtgtggatgccactttggtagtacattcaaataactttaccaacactatcttagaagttggccctgtaacaatggcaggacttattaatttgagtagcacccccactaacagaatgattcgttatgattatgcaacaaaaactgggcagtgtggaggtgtgctgtgtgctactggtaagatctttggtattcatgttggcggtaatggaagacaaggattttcagctcaacttaaaaaacaatattttgtagagaaacaaggccaagtaatagctagacataaggttagggagtttaacataaatccagtcaacacggcaactaagtcaaaattacatcccagtgtattttatgatgtttttccaggtgacaaggaacctgctgtattgagtgacaatgatcccagactggaagttaaattgactgaatcattattctctaagtacaaggggaatgtaaatacggaacccactgaaaatatgcttgtggctgtagaccattatgcagggcaactattatcactagatatccccacttctgaacttacactaaaagaagcattatatggagtagatggactagaacctatagatattacaaccagtgcaggatttccctatgtgagtcttgggatcaaaaagagagacattctgaataaagagacccaggacacagaaaagatgaagttttatctagacaagtatggcattgacttgcctctagttacatatattaaggatgaattaagaagtgttgacaaagtccgattagggaaaagtagattaattgaagcctccagtttgaatgattctgttaacatgagaatgaaactaggcaacctttacaaagcattccatcaaaatcccggtgttctgactggatcagcagtgggttgtgatcctgatgtgttttggtctgtcatcccttgcttaatggatgggcacctgatggcatttgattactctaattttgatgcctctttgtcaccagtttggtttgtctgtctagagaaggttttgaccaagttaggctttgcaggctcttcattaattcaatcaatttgtaatacccatcatatctttagggatgaaatatatgtggttgaaggtggcatgccctcagggtgttcaggaaccagcatattcaattccatgatcaacaacataatcattaggactttgatattagatgcatataaaggaatagatttagacaaacttaaaatcttagcttacggtgatgatttgattgtttcttatccttatgaactggatccacaagtgttggcaactcttggtaaaaattatggactaaccatcacacccccagacaaatctgaaacttttacaaaaatgacatgggaaaacttgacatttttaaagagatacttcaagcctgatcaacaatttccctttttggttcacccagttatgcccatgaaagatatacatgagtcaatcagatggacaaaggatcctaaaaacacacaggatcacgtccgatcattatgcatgttagcatggcactcaggagaaaaagagtacaatgaattcattcagaagatcagaactactgacattggaaaatgtctaattctcccagaatacagcgtacttaggaggcgctggttggacctcttttaggttaacaatatagacacttaatttgagtagaagtaggagtttat

SEQ ID NO: 32 - DNA, 7212 bp, unknown
  synthetic
ttaaaacagcggatgggtatcccaccattcgacccattgggtgtagtactctggtactatgtacctttgtacgcctgtttctccccaaccacccttccttaaaattcccacccatgaaacgttagaagcttgacattaaagtacaataggtggcgccatatccaatggtgtctatgtacaagcacttctgtttcccaggagcgaggtataggctgtacccactgccaaaagcctttaaccgttatccgccaaccaactacgtaacagttagtaccatcttgttcttgactggacgttcgatcaggtggattttccctccactagtttggtcgatgaggctaggaattccccacgggtgaccgtgtcctagcctgcgtggcggccaacccagcttatgctgggacgcccttttaaggacatggtgtgaagactcgcatgtgcttggttgtgagtcctccggcccctgaatgcggctaaccttaaccctagagccttatgccacgatccagtggttgtaaggtcgtaatgagcaattccgggacgggaccgactactttgggtgtccgtgtttctcatttttcttcatattgtcttatggtcacagcatatatatacatatactgtgatcatgggcgcacaagtgtcaacgcaaaaatccggatcacacgaaaaccaaaacatactgactaacggatctaatcagacttttacagtgattaattattataaagacgccgctagtactagttcagccggtcaatcactatctatggatccatctaaatttaccgaacccgttaaggatcttatgcttaaaggcgcaccagcacttaactcacctaacgttgaggcatgcggatactctgatagagtgcaacaaattacattgggtaatagtacaattactacacaggaagccgctaacgcagtcgtttgttacgccgaatggcccgaatacttacccgatgtcgacgcatcagacgttaataagacatctaaacccgatactagcgtatgtagattctatacactcgatagtaagacttggactaccggtagtaagggatggtgttggaaattgcctgacgcacttaaggatatgggcgtattcggtcagaatatgttttttcactcattgggtaggtcagggtatacagtacacgttcaatgtaacgctactaaatttcactcagggtgtctgttagtcgttgtgatacccgaacaccaattggcatcacacgaagggggtaacgttagcgttaagtatacatttacacatccaggcgaaagaggtatcgatctatcatccgctaacgaagtggggggacccgttaaagacgttatatacaatatgaacggtacactgttaggtaatctgttaatttttccacatcaatttattaatctgagaactaataataccgctacaatcgttataccatatattaactcagtgccaatcgatagtatgactagacataataacgttagtcttatggtgataccaatcgcaccattgacagtgccaaccggtgcaacacctagtctaccaattacggttacaatcgcacctatgtgtactgagttttccggtattaggtctaaatcaatcgtaccacaagggttacctactactacattgcccggatccggtcaatttttgactactgacgataggcaatcacctagcgcattgcctaattacgaacctacaccacgtatacatatactcggtaaggtgcataatctgttagagattatacaggtcgatacactgatacctatgaataatacacatacaaaagacgaagtgaattcgtatctgataccgttaaacgctaataggcaaaacgaacaggtattcggtacgaatctgtttataggcgatggcgtattcaaaactacactgttaggcgaaatcgttcaatactatacacattggtcagggtcacttagattctcatctatgtatacaggtccagcactatctagcgctaaattgacactcgcatatacacctcccggtgctaggggaccacaggataggagagaggctatgttaggtacacacgtagtgtgggatatcggattgcaatcgacaatcgttatgactataccatggacatcaggcgtacaatttagatataccgatcccgatacatatacatcagccggattcctatcatgttggtatcagactagtctgatactgccacccgaaactaccggtcaagtgtatctattgtcattcatatccgcatgtcccgattttaaacttagattgatgaaagatacacaaacaatttcgcaaacagtcgcactaaccgaagggttaggcgacgaattagaggaagtgatagtcgaaaaaactaagcaaacagtcgcatcaattagttccggacctaaacatacacaaaaagtgccaatattgaccgctaacgaaacaggcgcaactatgcccgtactgccatccgattcaatcgaaacacgaactacttatatgcattttaacggatccgaaaccgatgtcgaatgctttctaggtagggccgcatgcgtacacgttacagagatacagaataaagacgcaaccggtatcgataatcatagagaggctaaattgtttaacgattggaaaattaatctatctagtctagtgcaattgcgtaaaaaactcgaattgtttacatacgttagattcgatagcgaatatactatactcgcaaccgcatcacaacccgattccgctaattatagttctaacttagtcgttcaggctatgtacgtaccacacggtgcacctaaatctaaaagagtcggcgattatacatggcaatccgcatctaatccatcagtgttttttaaggtaggcgatactagtagattctcagtgccatacgtagggttagctagcgcatataattgtttttacgacggatactcacacgacgatgccgaaacacaatacggtattacggtactgaatcatatggggtcaatggcatttagaatcgttaacgaacacgacgaacataaaacactagttaagattagagtgtatcatagggctaagttagtcgaagcatggatacctagagcacctagagcactaccatatacatcaatcggtaggactaattatcctaaaaataccgaacccgttattaaaaaacgtaaaggcgatattaagtcatacggattagggcctagatacggaggtatatatacatctaacgttaagattatgaattatcatcttatgacaccagaggatcatcataacttaatcgcaccataccctaatagggatctagcaatcgttagtacagggggacacggagccgaaactataccgcattgtaatagaacatcaggcgtatactatagtacatattatagaaagtattatcctattatatgcgaaaaacctactaatatttggatcgaagggtcaccatattatcctagtagattccaagccggagtgatgaaaggcgtaggtccagccgaattaggcgattgcggaggtatactgagatgtatacacggtccaatcggactgttaactgccgaagggtcaggatacgtttgtttcgccgatattaggcaattggagtgtatagccgaagaacagggactatccgattatattaccggattgggtagggcattcggagtggggtttacggatcagattagtactaaggttaccgaattgcaggaagtcgctaaggattttttgactactaaagtgctatctaaagtcgttaaaatggttagcgcattagtgataatttgtaggaatcacgacgatctagttacggttaccgctacactcgcactattagggtgcgatgggtcaccatggagattccttaaaatgtatattagtaagcattttcaagtgccatatatcgaaagacaggctaacgacggatggtttagaaaatttaacgatgcatgtaacgccgctaagggactcgaatggatcgctaataagattagtaagttaatcgaatggattaaaaataaagtgttaccacaagctaaagagaaactcgaattttgtagtaagcttaagcaattggatatactcgaaagacagattacgactatgcatatatctaaccctacacaagagaaacgcgaacaattgtttaataacgtattgtggttagagcaaatgtcacaaaaattcgcaccattttacgcagtcgaatctaaacgtatacgcgaactgaaaaataaaatggttaactatatgcaatttaaatctaaacaacgaaccgaacccgtatgcgtactgatacacggtacacccggtagcggtaagtcattgactacatcaatcgtaggtagggctatagccgaacactttaactcagccgtatatagtctaccacccgatccaaaacatttcgatgggtatcaacaacaggaagtcgttattatggacgatctgaatcagaatcccgatggtcaggatattagtatgttttgtcaaatggtgtcatcagtcgattttctaccacctatggcatcactcgataataagggtatgttgtttacatctaatttcgtactcgcatcaactaactctaatacactatcaccacctactatactgaatcccgaagcattagtgcgtagattcggattcgatctagatatatgcttgcatacaacttatactaaaaacggtaagcttaacgccggtatgtcaactaagacatgtaaggattgtcaccaacctagtaattttaaaaaatgttgtccactagtttgcggtaaggcaattagtctagtcgatagaactactaacgttaggtattcagtcgatcaattggttaccgcaattatatccgattttaaatctaaaatgcaaattaccgattcactcgaaacattgtttcagggaccagtgtataaggatcttgagatagacgtatgcaatacaccacctagtgagtgtattaacgatctgttaaaatcagtcgatagcgaagagatacgcgaatattgtaaaaaaaaaaaatggattatacccgaaataccgactaatatcgaaagagctatgaatcaggctagtatgattattaatactatacttatgttcgttagtacattgggtatcgtttacgttatatacaaattgttcgcacaaacacagggaccatactcaggtaatccaccacataataagcttaaggcacctacacttagacccgtagtcgttcagggacctaataccgaattcgcactatcactattgcgtaaaaatattatgacaattactacatctaaaggcgaatttacagggttagggatacacgatagggtatgcgttataccgacacacgctcaacccggtgatgacgtactggttaacggtcaaaaaattagggttaaggataagtataagttagtcgatccagagaatattaacttagagttaaccgtactgacactcgatagaaacgaaaaatttagggatattagggggtttatatccgaagatcttgagggagtcgacgctacattagtcgtacactctaataattttacgaatactatactcgaagtcggacccgttactatggccggattgattaatctatctagtacacctactaatagaatgattaggtacgattacgctactaagacagggcaatgcggaggggtgttatgcgcaaccggtaagatattcggtatacacgtagggggtaacggtagacaggggtttagcgcacaattgaaaaaacagtatttcgtcgaaaaacagggtcaggtaatcgctagacataaggttagagagtttaatattaatcccgttaataccgctactaagtctaaattgcatccatcagtgttttacgacgtattcccaggcgataaggaaccagccgtactatccgataacgatcctagacttgaggttaagttaaccgaatcactattctctaagtataagggtaacgttaataccgaacctaccgaaaatatgttagtcgcagtcgatcattacgccggtcaattgctatcacttgatataccgactagcgaattgacacttaaagaggcactatacggagtcgacggactcgaaccaatcgatattactacatcagccggattcccatacgttagtctaggtattaaaaaaagggatatacttaacaaagagacacaggataccgaaaaaatgaaattttatctagataaatacggtatcgatctaccattagtgacttatattaaagacgaattgcgatcagtcgataaggttaggttaggtaagtctagattgatcgaagctagttcacttaacgatagcgttaatatgcgtatgaaattgggtaatctgtataaggcatttcaccaaaatcccggagtgttaaccggatccgcagtcggatgcgatccagacgttttttggtcagtgataccatgtcttatggacggacatcttatggcattcgattactctaatttcgatgcatcactatcacccgtttggttcgtatgtcttgagaaagtgttaactaagttagggttcgcaggatctagtctgatacaatcaatttgtaatacacatcatatttttagagacgaaatatacgtagtcgaagggggtatgcctagcggatgttccggtacatcaatttttaactctatgattaacaatattattattagaacattgatacttgacgcatataagggtatcgatctagataagcttaagatactcgcatacggagacgatctaatcgttagttatccatacgaactcgatccacaagtgttagcgacattgggtaagaattacggattgactattacacctcccgataaatccgaaacttttacgaaaatgacatgggagaatctgacatttctgaaacgatattttaaacccgatcagcaatttccattcttagtgcatcccgttatgcctatgaaagatatacacgaatcaattagatggactaaggatccaaaaaatacacaggatcacgttaggtcactatgtatgttagcatggcattcaggcgaaaaagagtataacgaattcatacaaaaaattagaactaccgatatcggtaagtgtctgatattgcccgaatactcagtgcttagacgtagatggttagatctattctaggttaacaatatagacacttaatttgagtagaagtaggagtttat

SEQ ID NO: 33 - DNA, 10735 bp, Dengue virus type 1
agttgttagtctacgtggaccgacaagaacagtttcgaatcggaagcttgcttaacgtagttctaacagttttttattagagagcagatctctgatgaataatcaacgtaaaaaaacgggtcgtccgtcgtttaatatgttaaaacgtgcgcgtaatcgtgtatcgacggtatcgcaattagcgaaacgtttttcgaaaggtttattatcgggtcaaggtccgatgaaattagtaatggcgtttatagcgtttttacgttttttagcgataccgccgacggcgggtatattagcgcgttggggttcgtttaaaaaaaatggtgcgataaaagtattacgtggttttaaaaaagaaatatcgaatatgttaaatataatgaatcgtcgtaaacgttcggtaacgatgttattaatgttattaccgacggcgttagcgtttcatttaacgacgcgtggtggtgaaccgcatatgatagtatcgaaacaagaacgtggtaaatcgttattatttaaaacgtcggcgggtgtaaatatgtgtacgttaatagcgatggatttaggtgaattatgtgaagatacgatgacgtataaatgtccgcgtataacggaaacggaaccggatgatgtagattgttggtgtaatgcgacggaaacgtgggtaacgtatggtacgtgttcgcaaacgggtgaacatcgtcgtgataaacgttcggtagcgttagcgccgcatgtaggtttaggtttagaaacgcgtacggaaacgtggatgtcgtcggaaggtgcgtggaaacaaatacaaaaagtagaaacgtgggcgttacgtcatccgggttttacggtaatagcgttatttttagcgcatgcgataggtacgtcgataacgcaaaaaggtataatatttatattattaatgttagtaacgccgtcgatggcgatgcgttgtgtaggtataggtaatcgtgattttgtagaaggtttatcgggtgcgacgtgggtagatgtagtattagaacatggttcgtgtgtaacgacgatggcgaaagataaaccgacgttagatatagaattattaaaaacggaagtaacgaatccggcggtattacgtaaattatgtatagaagcgaaaatatcgaatacgacgacggattcgcgttgtccgacgcaaggtgaagcgacgttagtagaagaacaagatacgaattttgtatgtcgtcgtacgtttgtagatcgtggttggggtaatggttgtggtttatttggtaaaggttcgttaataacgtgtgcgaaatttaaatgtgtaacgaaattagaaggtaaaatagtacaatatgaaaatttaaaatattcggtaatagtaacggtacatacgggtgatcaacatcaagtaggtaatgaaacgacggaacatggtacgacggcgacgataacgccgcaagcgccgacgtcggaaatacaattaacggattatggtgcgttaacgttagattgttcgccgcgtacgggtttagattttaatgaaatggtattattaacgatgaaaaaaaaatcgtggttagtacataaacaatggtttttagatttaccgttaccgtggacgtcgggtgcgtcgacgtcgcaagaaacgtggaatcgtcaagatttattagtaacgtttaaaacggcgcatgcgaaaaaacaagaagtagtagtattaggttcgcaagaaggtgcgatgcatacggcgttaacgggtgcgacggaaatacaaacgtcgggtacgacgacgatatttgcgggtcatttaaaatgtcgtttaaaaatggataaattaatattaaaaggtatgtcgtatgtaatgtgtacgggttcgtttaaattagaaaaagaagtagcggaaacgcaacatggtacggtattagtacaagtaaaatatgaaggtacggatgcgccgtgtaaaataccgttttcgtcgcaagatgaaaaaggtgtaacgcaaaatggtcgtttaataacggcgaatccgatagtaacggataaagaaaaaccggtaaatatagaagcggaaccgccgtttggtgaatcgtatatagtagtaggtgcgggtgaaaaagcgttaaaattatcgtggtttaaaaaaggttcgtcgataggtaaaatgtttgaagcgacggcgcgtggtgcgcgtcgtatggcgatattaggtgatacggcgtgggattttggttcgataggtggtgtatttacgtcggtaggtaaattaatacatcaaatatttggtacggcgtatggtgtattattttcgggtgtatcgtggacgatgaaaataggtataggtatattattaacgtggttaggtttaaattcgcgttcgacgtcgttatcgatgacgtgtatagcggtaggtatggtaacgttatatttaggtgtaatggtacaagcggattcgggttgtgtaataaattggaaaggtcgtgaattaaaatgtggttcgggtatatttgtaacgaatgaagtacatacgtggacggaacaatataaatttcaagcggattcgccgaaacgtttatcggcggcgataggtaaagcgtgggaagaaggtgtatgtggtatacgttcggcgacgcgtttagaaaatataatgtggaaacaaatatcgaatgaattaaatcatatattattagaaaatgatatgaaatttacggtagtagtaggtgatgtatcgggtatattagcgcaaggtaaaaaaatgatacgtccgcaaccgatggaacataaatattcgtggaaatcgtggggtaaagcgaaaataataggtgcggatgtacaaaatacgacgtttataatagatggtccgaatacgccggaatgtccggataatcaacgtgcgtggaatatatgggaagtagaagattatggttttggtatatttacgacgaatatatggttaaaattacgtgattcgtatacgcaagtatgtgatcatcgtttaatgtcggcggcgataaaagattcgaaagcggtacatgcggatatgggttattggatagaatcggaaaaaaatgaaacgtggaaattagcgcgtgcgtcgtttatagaagtaaaaacgtgtatatggccgaaatcgcatacgttatggtcgaatggtgtattagaatcggaaatgataataccgaaaatatatggtggtccgatatcgcaacataattatcgtccgggttattttacgcaaacggcgggtccgtggcatttaggtaaattagaattagattttgatttatgtgaaggtacgacggtagtagtagatgaacattgtggtaatcgtggtccgtcgttacgtacgacgacggtaacgggtaaaacgatacatgaatggtgttgtcgttcgtgtacgttaccgccgttacgttttaaaggtgaagatggttgttggtatggtatggaaatacgtccggtaaaagaaaaagaagaaaatttagtaaaatcgatggtatcggcgggttcgggtgaagtagattcgttttcgttaggtttattatgtatatcgataatgatagaagaagtaatgcgttcgcgttggtcgcgtaaaatgttaatgacgggtacgttagcggtatttttattattaacgatgggtcaattaacgtggaatgatttaatacgtttatgtataatggtaggtgcgaatgcgtcggataaaatgggtatgggtacgacgtatttagcgttaatggcgacgtttcgtatgcgtccgatgtttgcggtaggtttattatttcgtcgtttaacgtcgcgtgaagtattattattaacggtaggtttatcgttagtagcgtcggtagaattaccgaattcgttagaagaattaggtgatggtttagcgatgggtataatgatgttaaaattattaacggattttcaatcgcatcaattatgggcgacgttattatcgttaacgtttgtaaaaacgacgttttcgttacattatgcgtggaaaacgatggcgatgatattatcgatagtatcgttatttccgttatgtttatcgacgacgtcgcaaaaaacgacgtggttaccggtattattaggttcgttaggttgtaaaccgttaacgatgtttttaataacggaaaataaaatatggggtcgtaaatcgtggccgttaaatgaaggtataatggcggtaggtatagtatcgatattattatcgtcgttattaaaaaatgatgtaccgttagcgggtccgttaatagcgggtggtatgttaatagcgtgttatgtaatatcgggttcgtcggcggatttatcgttagaaaaagcggcggaagtatcgtgggaagaagaagcggaacattcgggtgcgtcgcataatatattagtagaagtacaagatgatggtacgatgaaaataaaagatgaagaacgtgatgatacgttaacgatattattaaaagcgacgttattagcgatatcgggtgtatatccgatgtcgataccggcgacgttatttgtatggtatttttggcaaaaaaaaaaacaacgttcgggtgtattatgggatacgccgtcgccgccggaagtagaacgtgcggtattagatgatggtatatatcgtatattacaacgtggtttattaggtcgttcgcaagtaggtgtaggtgtatttcaagaaggtgtatttcatacgatgtggcatgtaacgcgtggtgcggtattaatgtatcaaggtaaacgtttagaaccgtcgtgggcgtcggtaaaaaaagatttaatatcgtatggtggtggttggcgttttcaaggttcgtggaatgcgggtgaagaagtacaagtaatagcggtagaaccgggtaaaaatccgaaaaatgtacaaacggcgccgggtacgtttaaaacgccggaaggtgaagtaggtgcgatagcgttagattttaaaccgggtacgtcgggttcgccgatagtaaatcgtgaaggtaaaatagtaggtttatatggtaatggtgtagtaacgacgtcgggtacgtatgtatcggcgatagcgcaagcgaaagcgtcgcaagaaggtccgttaccggaaatagaagatgaagtatttcgtaaacgtaatttaacgataatggatttacatccgggttcgggtaaaacgcgtcgttatttaccggcgatagtacgtgaagcgataaaacgtaaattacgtacgttagtattagcgccgacgcgtgtagtagcgtcggaaatggcggaagcgttaaaaggtatgccgatacgttatcaaacgacggcggtaaaatcggaacatacgggtaaagaaatagtagatttaatgtgtcatgcgacgtttacgatgcgtttattatcgccggtacgtgtaccgaattataatatgataataatggatgaagcgcattttacggatccggcgtcgatagcggcgcgtggttatatatcgacgcgtgtaggtatgggtgaagcggcggcgatatttatgacggcgacgccgccgggttcggtagaagcgtttccgcaatcgaatgcggtaatacaagatgaagaacgtgatataccggaacgttcgtggaattcgggttatgattggataacggattttccgggtaaaacggtatggtttgtaccgtcgataaaatcgggtaatgatatagcgaattgtttacgtaaaaatggtaaacgtgtagtacaattatcgcgtaaaacgtttgatacggaatatcaaaaaacgaaaaataatgattgggattatgtagtaacgacggatatatcggaaatgggtgcgaattttcgtgcggatcgtgtaatagatccgcgtcgttgtttaaaaccggtaatattaaaagatggtccggaacgtgtaatattagcgggtccgatgccggtaacggtagcgtcggcggcgcaacgtcgtggtcgtataggtcgtaatcaaaataaagaaggtgatcaatatatatatatgggtcaaccgttaaataatgatgaagatcatgcgcattggacggaagcgaaaatgttattagataatataaatacgccggaaggtataataccggcgttatttgaaccggaacgtgaaaaatcggcggcgatagatggtgaatatcgtttacgtggtgaagcgcgtaaaacgtttgtagaattaatgcgtcgtggtgatttaccggtatggttatcgtataaagtagcgtcggaaggttttcaatattcggatcgtcgttggtgttttgatggtgaacgtaataatcaagtattagaagaaaatatggatgtagaaatatggacgaaagaaggtgaacgtaaaaaattacgtccgcgttggttagatgcgcgtacgtattcggatccgttagcgttacgtgaatttaaagaatttgcggcgggtcgtcgttcggtatcgggtgatttaatattagaaataggtaaattaccgcaacatttaacgcaacgtgcgcaaaatgcgttagataatttagtaatgttacataattcggaacaaggtggtaaagcgtatcgtcatgcgatggaagaattaccggatacgatagaaacgttaatgttattagcgttaatagcggtattaacgggtggtgtaacgttattttttttatcgggtcgtggtttaggtaaaacgtcgataggtttattatgtgtaatagcgtcgtcggcgttattatggatggcgtcggtagaaccgcattggatagcggcgtcgataatattagaattttttttaatggtattattaataccggaaccggatcgtcaacgtacgccgcaagataatcaattagcgtatgtagtaataggtttattatttatgatattaacggtagcggcgaatgaaatgggtttattagaaacgacgaaaaaagatttaggtataggtcatgcggcggcggaaaatcatcatcatgcggcgatgttagatgtagatttacatccggcgtcggcgtggacgttatatgcggtagcgacgacgataataacgccgatgatgcgtcatacgatagaaaatacgacggcgaatatatcgttaacggcgatagcgaatcaagcggcgatattaatgggtttagataaaggttggccgatatcgaaaatggatataggtgtaccgttattagcgttaggttgttattcgcaagtaaatccgttaacgttaacggcggcggtattaatgttagtagcgcattatgcgataataggtccgggtttacaagcgaaagcgacgcgtgaagcgcaaaaacgtacggcggcgggtataatgaaaaatccgacggtagatggtatagtagcgatagatttagatccggtagtatatgatgcgaaatttgaaaaacaattaggtcaaataatgttattaatattatgtacgtcgcaaatattattaatgcgtacgacgtgggcgttatgtgaatcgataacgttagcgacgggtccgttaacgacgttatgggaaggttcgccgggtaaattttggaatacgacgatagcggtatcgatggcgaatatatttcgtggttcgtatttagcgggtgcgggtttagcgttttcgttaatgaaatcgttaggtggtggtcgtcgtggtacgggtgcgcaaggtgaaacgttaggtgaaaaatggaaacgtcaattaaatcaattatcgaaatcggaatttaatacgtataaacgttcgggtataatagaagtagatcgttcggaagcgaaagaaggtttaaaacgtggtgaaacgacgaaacatgcggtatcgcgtggtacggcgaaattacgttggtttgtagaacgtaatttagtaaaaccggaaggtaaagtaatagatttaggttgtggtcgtggtggttggtcgtattattgtgcgggtttaaaaaaagtaacggaagtaaaaggttatacgaaaggtggtccgggtcatgaagaaccgataccgatggcgacgtatggttggaatttagtaaaattatattcgggtaaagatgtattttttacgccgccggaaaaatgtgatacgttattatgtgatataggtgaatcgtcgccgaatccgacgatagaagaaggtcgtacgttacgtgtattaaaaatggtagaaccgtggttacgtggtaatcaattttgtataaaaatattaaatccgtatatgccgtcggtagtagaaacgttagaacaaatgcaacgtaaacatggtggtatgttagtacgtaatccgttatcgcgtaattcgacgcatgaaatgtattgggtatcgtgtggtacgggtaatatagtatcggcggtaaatatgacgtcgcgtatgttattaaatcgttttacgatggcgcatcgtaaaccgacgtatgaacgtgatgtagatttaggtgcgggtacgcgtcatgtagcggtagaaccggaagtagcgaatttagatataataggtcaacgtatagaaaatataaaaaatgaacataaatcgacgtggcattatgatgaagataatccgtataaaacgtgggcgtatcatggttcgtatgaagtaaaaccgtcgggttcggcgtcgtcgatggtaaatggtgtagtacgtttattaacgaaaccgtgggatgtaataccgatggtaacgcaaatagcgatgacggatacgacgccgtttggtcaacaacgtgtatttaaagaaaaagtagatacgcgtacgccgaaagcgaaacgtggtacggcgcaaataatggaagtaacggcgcgttggttatggggttttttatcgcgtaataaaaaaccgcgtatatgtacgcgtgaagaatttacgcgtaaagtacgttcgaatgcggcgataggtgcggtatttgtagatgaaaatcaatggaattcggcgaaagaagcggtagaagatgaacgtttttgggatttagtacatcgtgaacgtgaattacataaacaaggtaaatgtgcgacgtgtgtatataatatgatgggtaaacgtgaaaaaaaattaggtgaatttggtaaagcgaaaggttcgcgtgcgatatggtatatgtggttaggtgcgcgttttttagaatttgaagcgttaggttttatgaatgaagatcattggttttcgcgtgaaaattcgttatcgggtgtagaaggtgaaggtttacataaattaggttatatattacgtgatatatcgaaaataccgggtggtaatatgtatgcggatgatacggcgggttgggatacgcgtataacggaagatgatttacaaaatgaagcgaaaataacggatataatggaaccggaacatgcgttattagcgacgtcgatatttaaattaacgtatcaaaataaagtagtacgtgtacaacgtccggcgaaaaatggtacggtaatggatgtaatatcgcgtcgtgatcaacgtggttcgggtcaagtaggtacgtatggtttaaatacgtttacgaatatggaagcgcaattaatacgtcaaatggaatcggaaggtatattttcgccgtcggaattagaaacgccgaatttagcggaacgtgtattagattggttaaaaaaacatggtacggaacgtttaaaacgtatggcgatatcgggtgatgattgtgtagtaaaaccgatagatgatcgttttgcgacggcgttaacggcgttaaatgatatgggtaaagtacgtaaagatataccgcaatgggaaccgtcgaaaggttggaatgattggcaacaagtaccgttttgttcgcatcattttcatcaattaataatgaaagatggtcgtgaaatagtagtaccgtgtcgtaatcaagatgaattagtaggtcgtgcgcgtgtatcgcaaggtgcgggttggtcgttacgtgaaacggcgtgtttaggtaaatcgtatgcgcaaatgtggcaattaatgtattttcatcgtcgtgatttacgtttagcggcgaatgcgatatgttcggcggtaccggtagattgggtaccgacgtcgcgtacgacgtggtcgatacatgcgcatcatcaatggatgacgacggaagatatgttatcggtatggaatcgtgtatggatagaagaaaatccgtggatggaagataaaacgcatgtatcgtcgtgggaagatgtaccgtatttaggtaaacgtgaagatcaatggtgtggttcgttaataggtttaacggcgcgtgcgacgtgggcgacgaatatacaagtagcgataaatcaagtacgtcgtttaataggtaatgaaaattatttagattttatgacgtcgatgaaacgttttaaaaatgaatcggatccggaaggtgcgttatggtaagccaactcattcacaaaataaaggaaaataaaaaatcaaacaaggcaagaagtcaggccggattaagccatagcacggtaagagctatgctgcctgtgagccccgtccaaggacgtaaaatgaagtcaggccgaaagccacggttcgagcaagccgtgctgcctgtagctccatcgtggggatgtaaaaacccgggaggctgcaaaccatggaagctgtacgcatggggtagcagactagtggttagaggagacccctcccaagacacaacgcagcagcggggcccaacaccaggggaagctgtaccctggtggtaaggactagaggttagaggagaccccccgcacaacaacaaacagcatattgacgctgggagagaccagagatcctgctgtctctacagcatcattccaggcacagaacgccaaaaaatggaatggtgctgttgaatcaacaggttct

SEQ ID NO: 34 - DNA, 10735 bp, Unknown
  synthetic
agttgttagtctacgtggaccgacaagaacagtttcgaatcggaagcttgcttaacgtagttctaacagttttttattagagagcagatctctgatgaataaccaacgaaaaaaaaccggacgaccatcattcaatatgcttaaacgcgctaggaatagggtgtcaaccgtatcgcaattggctaagagattctctaagggactgttaagcggacagggaccaatgaaactggttatggcattcatagcgtttctgagatttctcgcaataccgccaaccgccggaatactcgctagatgggggtcattcaaaaaaaacggcgcaattaaagtgcttagggggttcaaaaaagagatatcgaatatgcttaacattatgaatagacgtaagagatccgttacaatgctattgatgctattgccaaccgcactagcctttcacctaacgactagggggggggaaccacatatgatagtgagtaagcaagagagaggtaagtcactattgttcaaaacatccgccggagtgaatatgtgtacactaatcgctatggacttaggcgaattgtgcgaagacactatgacatataagtgtcctaggattaccgaaaccgaaccagacgacgtcgattgttggtgtaacgcaaccgaaacatgggtgacatacggaacatgttcgcaaaccggagagcatagacgcgataagagatcagtcgcactcgcaccacacgtcggattggggttagagactagaaccgaaacatggatgtctagcgaaggcgcatggaaacagatacagaaagtcgagacatgggcccttagacacccagggtttaccgtaatcgcactatttctcgcacacgcaatcggaacgtcaattacgcaaaaagggattatattcatactgcttatgttagtgacaccatctatggctatgagatgcgtcggaatcggaaatagggatttcgttgagggactatccggagcgacatgggtcgacgtagtgctcgaacacggatcatgcgttacgactatggccaaagacaaaccgacacttgacatagagttactgaaaaccgaagtgactaacccagccgtactgagaaagttgtgtatcgaagctaagatatcgaatacgactaccgatagtaggtgtccaacgcaaggcgaagcgacactagtcgaagagcaggatacgaatttcgtatgtagacgtacattcgtcgatagggggtggggaaacggatgcggattgttcggtaagggatcactgattacatgcgctaaattcaaatgcgttacgaaactcgagggtaagatagtgcaatacgagaatctgaaatatagcgtaatcgttacagtgcataccggagaccaacaccaagtgggaaacgagactaccgaacacggaactaccgcaacgattacgccacaagcccctactagcgaaatccaattgaccgattacggcgcactaacactcgattgttcacctagaaccggattggactttaacgaaatggtgctattgactatgaaaaaaaaatcatggttagtgcataagcaatggttcttagacctaccactaccatggactagcggagctagtacgtcacaggagacatggaatagacaggatctgttagtgacattcaaaaccgcacacgctaaaaaacaggaggtcgtagtgttagggtcacaagagggagctatgcataccgcactaacaggcgcaaccgagatacagactagcggaacgactacgatattcgccggacaccttaagtgtagactgaaaatggacaaactgatactgaaaggtatgtcatacgttatgtgtaccggatcattcaaactcgaaaaagaggtcgccgaaacgcaacacggaacagtgttagtgcaagtgaaatacgagggaactgacgcaccatgtaagataccgttttcgtcacaggacgaaaaaggcgttacgcaaaacggtagactgattaccgctaacccaatcgttaccgataaagagaaaccggttaatatcgaagccgaaccaccattcggcgaatcatatatcgtagtcggagccggagagaaagcccttaagctatcatggtttaaaaaagggtcatcaatcggtaagatgttcgaagcaaccgctagaggcgctagacgtatggccatactaggcgataccgcatgggatttcggatcaatcggaggagtgtttacgtcagtcggaaaactgatacaccaaattttcggaaccgcatacggagtgttgtttagcggagtgtcatggactatgaaaatcggaatcggaatactgttgacatggttagggttgaactctagatcgactagtctatctatgacatgtatcgcagtcggaatggtgacactatacttaggcgtaatggtgcaagccgatagcggatgcgttattaattggaaagggagagagcttaaatgcggatccggaatattcgttacgaacgaagtgcatacatggaccgaacagtataaattccaagccgatagtccgaaaagactatctgccgcaatcggtaaggcatgggaggagggagtgtgcggaattaggtcagcgactagactcgaaaacattatgtggaaacagatatctaacgaactgaatcacatactgttagagaacgatatgaaatttacagtcgtagtcggagacgttagcggaatactcgcacagggtaagaaaatgattagaccgcaacctatggagcataagtatagttggaaatcatggggaaaagcgaaaattatcggagccgacgtgcaaaatacgacattcataatcgacggaccgaatacgccagagtgtccagacaatcagagagcatggaacatatgggaggtcgaagactacggattcggaatttttacgactaacatatggcttaagcttagagactcatatacacaggtatgcgatcatagattgatgtctgccgcaatcaaagactctaaagccgtacacgccgatatggggtattggatcgaatccgaaaaaaacgagacatggaaactcgctagagcgtcattcatagaggttaagacatgtatttggcctaagtcacatacattgtggtctaacggagtgcttgagtctgagatgataatccctaagatatacggcggaccgatatcgcaacataactatagaccagggtattttacgcaaacagccggaccatggcatctcggtaagcttgagttagacttcgatctatgcgaagggactaccgtagtggtcgacgaacattgcggtaataggggacctagtctgagaacgactaccgttaccggtaagactatacacgaatggtgttgtaggtcatgtacactaccaccacttagattcaaaggcgaagacggatgttggtacggaatggagattagaccagtgaaagagaaagaggaaaacctagtgaaatctatggtgtcagccggatcaggcgaagtcgactcattctcactcggactgttatgcatatcgattatgatcgaagaggttatgcgatctagatggtcacgaaaaatgcttatgaccggaacactagccgtttttctgttactgactatggggcaattgacatggaacgatctgattaggttgtgtattatggtcggagctaacgctagcgataagatgggtatgggaacgacatacttagcccttatggctacatttagaatgcgaccaatgttcgccgtagggttactgtttagacggttgactagtagggaagtgctattgttgacagtcggactgtcactagtcgctagcgttgagttgcctaactcactcgaagagttaggcgacggactcgcaatggggattatgatgcttaagctattgaccgatttccaatctcaccaattgtgggctacactattgtcactgacattcgttaagactacattctcattgcattacgcatggaaaactatggctatgatactgtcaatcgttagtctattcccactatgtctatctacaactagtcagaaaactacatggttgccagtgctattggggtcactagggtgtaaaccattgactatgtttctgattaccgaaaacaaaatttgggggagaaagtcatggccacttaacgagggaattatggccgtagggatagtgtcaatactgctatctagtctgcttaaaaacgacgtgccactagccggaccactgatagccggaggtatgctaatcgcatgttacgtgatatccggatctagcgccgatctgtcactcgaaaaagccgccgaagtgtcatgggaagaggaagccgaacactctggcgcatcacataacatactagtcgaagtgcaagacgacggaactatgaaaattaaagacgaagagagagacgatacacttacgatactgcttaaagcgacactgttagcgatatccggagtgtatcctatgtcaatacccgctacactattcgtttggtatttttggcaaaaaaaaaaacagagatccggagtgttgtgggatacacctagtccacccgaagtcgagagagccgtactcgacgacggaatatataggatactgcaacggggattgctcggtaggtcacaggtcggagtgggagtgtttcaggagggagtgtttcacactatgtggcacgttacgagaggcgccgtactgatgtatcagggtaagagactcgaacctagttgggctagcgttaaaaaagacctaatctcatacggaggggggtggagatttcaggggtcatggaacgccggagaggaagtgcaagtgatagccgtcgaacccggtaagaaccctaaaaacgtgcaaaccgcacccggaacgtttaagacacccgaaggcgaagtgggcgcaatcgcactcgactttaaacccggaactagcggatcaccaatcgttaatagagagggtaagatagtcggattgtacggaaacggagtggttacgactagcggaacatacgttagcgcaatagcgcaagcgaaagcgtcacaagagggaccactaccagagatagaggacgaagtgtttagaaagcgtaatctgacaattatggacctacatcccggatccggtaagactagacggtatctgccagcaatcgttagggaggcaattaagagaaagttgcgtacactagtgttagccccaactagagtggtcgctagcgaaatggccgaagcccttaagggaatgccaattaggtatcagactaccgccgttaagtccgaacataccggtaaggagatagtcgaccttatgtgtcacgctacattcacaatgagactgctatcaccagtgagagtgcctaactataatatgataattatggacgaagcccattttacagacccagcctcaatcgccgctagggggtatattagtactagggtgggaatgggcgaagccgccgcaatttttatgacagcgacaccacccggatccgtcgaagcgtttccgcaatctaacgccgttatacaggacgaagagagagacatacccgaacggtcatggaatagcggatacgattggataaccgattttcccggtaagacagtgtggttcgtaccgtcaattaagtccggaaacgatatcgctaattgtcttagaaaaaacggtaagagagtggtgcaattgtctagaaagacattcgataccgaataccaaaaaactaagaataacgattgggattacgtagtgacaaccgacatatccgaaatgggcgctaactttagagccgatagggtgatagaccctagacggtgtctgaaaccagtgatactgaaagacggaccagagagagtgatactagccggaccaatgccagtgacagtcgcatccgccgcacaacgtaggggacggatagggagaaaccaaaacaaagagggagaccaatacatatatatgggacagccactgaataacgacgaagaccacgcacattggaccgaagcgaaaatgctattagacaatattaacacacccgaagggattatacccgcactattcgaacccgaacgcgaaaaatccgccgcaatcgacggcgaatatagactgagaggcgaagctagaaagacattcgttgagcttatgcgtagaggcgatctacccgtatggttgtcatacaaagtcgctagcgaagggtttcagtattccgataggagatggtgtttcgacggcgaacggaataaccaagtgctcgaagagaatatggacgttgagatatggactaaagagggcgaacgaaaaaaactgagacctagatggttagacgcacgtacatattccgatccgttagcccttagagagtttaaagagttcgcagccggtaggagatccgttagcggagatctgatactcgaaatcggtaagctaccacaacacctaacgcaacgagcccaaaacgcactagacaatctggttatgttgcataactccgaacagggcggtaaggcatatagacacgctatggaagagttacccgatacaatcgaaacacttatgctactcgcactgatagccgtactgacaggcggagtgacactattctttctatccggtagggggttaggtaagacatcaatcggactgttatgcgtaatcgcatctagcgcactattgtggatggctagcgtcgaaccacattggatagccgcatcaattatactcgaattctttcttatggtgttactgatacccgaacccgataggcaacgaacaccacaggataaccaattggcatacgtcgtaatcggactattgtttatgatactgacagtcgccgctaacgaaatgggattgctcgagacaacgaaaaaagacctagggatcggacacgccgcagccgaaaatcaccatcacgccgcaatgttagacgtcgatctgcatcccgctagcgcatggacactatacgcagtcgcaacgacaattattacgcctatgatgcgacatacaatcgagaatactaccgctaacatatcgctaaccgctatagcgaatcaggccgcaatactgatggggttagacaaagggtggccaattagtaagatggatatcggagtgccactgttagccttagggtgttatagtcaggttaacccattgacattgaccgcagccgtacttatgctagtcgcacattacgctataatcggaccaggactgcaagcgaaagcgacacgcgaagcgcaaaaaagaaccgcagccggaattatgaaaaaccctacagtcgacggaatagtcgcaatcgacttagacccagtggtgtacgacgctaaattcgaaaaacagttgggacagattatgctactgatactgtgtacgtcacagatactgcttatgcgaactacatgggcactatgcgaatcaattacactcgcaaccggaccattgactacattgtgggagggatcacccggtaagttttggaatacgactatagccgttagtatggctaacatttttagggggtcatatctagccggagccggactcgcattctcacttatgaaatcactcggagggggacgtagggggacaggcgcacagggagagacactaggcgaaaaatggaaacgacaattgaaccaattgtctaaatccgaatttaacacttataagagatccggaataatcgaagtcgatagatccgaagcgaaagagggactgaaacgcggagagacaacgaaacacgccgttagtaggggaaccgctaagcttagatggttcgttgagcgtaacttagtgaaaccagagggtaaggtaatcgatctcggatgcggtaggggggggtggtcatactattgcgccggactgaaaaaagtgaccgaagtgaaagggtatactaagggcggacccggacacgaagagccaataccgatggcaacatacggatggaacctagtgaaactgtattccggtaaggacgtattctttacaccacccgaaaaatgcgatacactgttatgcgatataggcgaatctagtcctaaccctacaatcgaagagggacgtacacttagagtgcttaaaatggtcgaaccatggttgagggggaatcagttttgtattaagatactgaatccatatatgcctagcgtagtcgagacactcgaacagatgcaacgaaaacacggcggaatgctagtgagaaacccactatctaggaattcgacacacgaaatgtattgggtgtcatgcggaaccggaaacatagtgtcagccgttaatatgactagtagaatgctactgaatcggtttacaatggcccatagaaaaccgacatacgaaagagacgtcgacctaggagccggaactagacacgttgccgtcgaacccgaagtcgctaacttagacataatcggacagagaatcgagaatattaaaaacgaacacaaatcgacatggcattacgacgaagacaatccgtataagacatgggcatatcacggatcatacgaagtgaaacctagcggatccgctagttctatggttaacggagtggtgagactgttgactaagccatgggacgtgataccgatggtgacacaaatcgctatgaccgatacgacaccattcggacagcaaagagtgtttaaagagaaagtcgacactagaacacctaaagcgaaacgcggaaccgcacagattatggaggttaccgctagatggttgtgggggttcctatctagaaacaaaaaacctaggatttgtacacgcgaagagtttacacgaaaagtgagatctaacgccgcaatcggagccgtattcgtagacgaaaaccaatggaattccgctaaagaggccgtcgaagacgaacggttttgggacttagtgcatagggaacgcgaattgcataaacagggtaagtgcgcaacatgcgtatacaatatgatgggtaagcgcgaaaaaaagttaggcgaattcggtaaggctaagggatctagagcgatatggtatatgtggttaggcgctaggtttctcgaattcgaagcactcggatttatgaacgaagaccattggttttctagagagaatagtctatccggagtcgagggagagggattgcataaactcggatatatactgagagacatatctaagatacccggagggaatatgtacgccgacgatacagccggatgggatacacgaattaccgaagacgatctgcaaaacgaagcgaaaattaccgatattatggaacccgaacacgcactgttagcgacatctatttttaagttgacatatcagaataaggtcgttagggtgcaacgacccgctaaaaacggaacggttatggacgtgattagtaggagagaccaacgcggatccggacaggtcggaacatacggactgaatacgtttacgaatatggaagcgcaattgattagacagatggagtctgaggggatattctcacctagcgaactcgagacacctaacctagccgaacgggtactcgattggttgaaaaaacacggaaccgaaagactgaaaagaatggcaattagcggagacgattgcgtagtgaaaccaatcgacgatagattcgcaaccgcactaaccgcacttaacgatatgggtaaggtgagaaaagacataccgcaatgggagccatctaagggatggaacgattggcaacaggtgccattttgctcacatcactttcaccaattgattatgaaagacggtagggagatagtcgtgccatgtaggaatcaggacgaactcgtaggtagggctagagtgtcacagggagccggatggtcacttagggaaaccgcatgcctaggtaagtcatacgctcaaatgtggcaattgatgtatttccatagacgcgatctgagactagccgctaacgctatatgctctgccgtaccagtcgattgggtgccaactagtagaacgacatggtctatacacgcacatcaccaatggatgacaaccgaagacatgctatccgtttggaatagggtgtggatcgaagagaatccatggatggaggataagacacacgtgtctagttgggaggacgtgccatatctcggaaaacgcgaagaccaatggtgcggatcactaatcggattgaccgctagagcgacatgggcaactaacatacaggtcgcaattaaccaagtgagacgattgatcggaaacgagaattatctcgactttatgacatctatgaaaagattcaaaaacgaatccgatcccgaaggcgcactatggtaagccaactcattcacaaaataaaggaaaataaaaaatcaaacaaggcaagaagtcaggccggattaagccatagcacggtaagagctatgctgcctgtgagccccgtccaaggacgtaaaatgaagtcaggccgaaagccacggttcgagcaagccgtgctgcctgtagctccatcgtggggatgtaaaaacccgggaggctgcaaaccatggaagctgtacgcatggggtagcagactagtggttagaggagacccctcccaagacacaacgcagcagcggggcccaacaccaggggaagctgtaccctggtggtaaggactagaggttagaggagaccccccgcacaacaacaaacagcatattgacgctgggagagaccagagatcctgctgtctctacagcatcattccaggcacagaacgccaaaaaatggaatggtgctgttgaatcaacaggttct

SEQ ID NO: 35 - DNA, 9181 bp, Human immunodeficiency virus type 1
ggtctctctggttagaccagatctgagcctgggagctctctggctaactagggaacccactgcttaagcctcaataaagcttgccttgagtgcttcaagtagtgtgtgcccgtctgttgtgtgactctggtaactagagatccctcagacccttttagtcagtgtggaaaatctctagcagtggcgcccgaacagggacctgaaagcgaaagggaaaccagaggagctctctcgacgcaggactcggcttgctgaagcgcgcacggcaagaggcgaggggcggcgactggtgagtacgccaaaaattttgactagcggaggctagaaggagagagatgggtgcgcgtgcgtcggtattatcgggtggtgaattagatcgttgggaaaaaatacgtttacgtccgggtggtaaaaaaaaatataaattaaaacatatagtatgggcgtcgcgtgaattagaacgttttgcggtaaatccgggtttattagaaacgtcggaaggttgtcgtcaaatattaggtcaattacaaccgtcgttacaaacgggttcggaagaattacgttcgttatataatacggtagcgacgttatattgtgtacatcaacgtatagaaataaaagatacgaaagaagcgttagataaaatagaagaagaacaaaataaatcgaaaaaaaaagcgcaacaagcggcggcggatacgggtcattcgaatcaagtatcgcaaaattatccgatagtacaaaatatacaaggtcaaatggtacatcaagcgatatcgccgcgtacgttaaatgcgtgggtaaaagtagtagaagaaaaagcgttttcgccggaagtaataccgatgttttcggcgttatcggaaggtgcgacgccgcaagatttaaatacgatgttaaatacggtaggtggtcatcaagcggcgatgcaaatgttaaaagaaacgataaatgaagaagcggcggaatgggatcgtgtacatccggtacatgcgggtccgatagcgccgggtcaaatgcgtgaaccgcgtggttcggatatagcgggtacgacgtcgacgttacaagaacaaataggttggatgacgaataatccgccgataccggtaggtgaaatatataaacgttggataatattaggtttaaataaaatagtacgtatgtattcgccgacgtcgatattagatatacgtcaaggtccgaaagaaccgtttcgtgattatgtagatcgtttttataaaacgttacgtgcggaacaagcgtcgcaagaagtaaaaaattggatgacggaaacgttattagtacaaaatgcgaatccggattgtaaaacgatattaaaagcgttaggtccggcggcgacgttagaagaaatgatgacggcgtgtcaaggtgtaggtggtccgggtcataaagcgcgtgtattagcggaagcgatgtcgcaagtaacgaattcggcgacgataatgatgcaacgtggtaattttcgtaatcaacgtaaaatagtaaaatgttttaattgtggtaaagaaggtcatacggcgcgtaattgtcgtgcgccgcgtaaaaaaggttgttggaaatgtggtaaagaaggtcatcaaatgaaagattgtacggaacgtcaagcgaattttttagggaagatctggccttcctacaagggaaggccagggaattttcttcagagcagaccagagccaacagccccaccagaagagagcttcaggtctggggtagagacaacaactccccctcagaagcaggagccgatagacaaggaactgtatcctttaacttccctcaggtcactctttggcaacgacccctcgtcacaataaagataggtggtcaattaaaagaagcgttattagatacgggtgcggatgatacggtattagaagaaatgtcgttaccgggtcgttggaaaccgaaaatgataggtggtataggtggttttataaaagtacgtcaatatgatcaaatattaatagaaatatgtggtcataaagcgataggtacggtattagtaggtccgacgccggtaaatataataggtcgtaatttattaacgcaaataggttgtacgttaaattttccgatatcgccgatagaaacggtaccggtaaaattaaaaccgggtatggatggtccgaaagtaaaacaatggccgttaacggaagaaaaaataaaagcgttagtagaaatatgtacggaaatggaaaaagaaggtaaaatatcgaaaataggtccggaaaatccgtataatacgccggtatttgcgataaaaaaaaaagattcgacgaaatggcgtaaattagtagattttcgtgaattaaataaacgtacgcaagatttttgggaagtacaattaggtataccgcatccggcgggtttaaaaaaaaaaaaatcggtaacggtattagatgtaggtgatgcgtatttttcggtaccgttagatgaagattttcgtaaatatacggcgtttacgataccgtcgataaataatgaaacgccgggtatacgttatcaatataatgtattaccgcaaggttggaaaggttcgccggcgatatttcaatcgtcgatgacgaaaatattagaaccgtttcgtaaacaaaatccggatatagtaatatatcaatatatggatgatttatatgtaggttcggatttagaaataggtcaacatcgtacgaaaatagaagaattacgtcaacatttattacgttggggtttaacgacgccggataaaaaacatcaaaaagaaccgccgtttttatggatgggttatgaattacatccggataaatggacggtacaaccgatagtattaccggaaaaagattcgtggacggtaaatgatatacaaaaattagtaggtaaattaaattgggcgtcgcaaatatatccgggtataaaagtacgtcaattatgtaaattattacgtggtacgaaagcgttaacggaagtaataccgttaacggaagaagcggaattagaattagcggaaaatcgtgaaatattaaaagaaccggtacatggtgtatattatgatccgtcgaaagatttaatagcggaaatacaaaaacaaggtcaaggtcaatggacgtatcaaatatatcaagaaccgtttaaaaatttaaaaacgggtaaatatgcgcgtatgcgtggtgcgcatacgaatgatgtaaaacaattaacggaagcggtacaaaaaataacgacggaatcgatagtaatatggggtaaaacgccgaaatttaaattaccgatacaaaaagaaacgtgggaaacgtggtggacggaatattggcaagcgacgtggataccggaatgggaatttgtaaatacgccgccgttagtaaaattatggtatcaattagaaaaagaaccgatagtaggtgcggaaacgttttatgtagatggtgcggcgaatcgtgaaacgaaattaggtaaagcgggttatgtaacgaatcgtggtcgtcaaaaagtagtaacgttaacggatacgacgaatcaaaaaacggaattacaagcgatatatttagcgttacaagattcgggtttagaagtaaatatagtaacggattcgcaatatgcgttaggtataatacaagcgcaaccggatcaatcggaatcggaattagtaaatcaaataatagaacaattaataaaaaaagaaaaagtatatttagcgtgggtaccggcgcataaaggtataggtggtaatgaacaagtagataaattagtatcggcgggtatacgtaaagtattatttttagatggtatagataaagcgcaagatgaacatgaaaaatatcattcgaattggcgtgcgatggcgtcggattttaatttaccgccggtagtagcgaaagaaatagtagcgtcgtgtgataaatgtcaattaaaaggtgaagcgatgcatggtcaagtagattgttcgccgggtatatggcaattagattgtacgcatttagaaggtaaagtaatattagtagcggtacatgtagcgtcgggttatatagaagcggaagtaataccggcggaaacgggtcaagaaacggcgtattttttattaaaattagcgggtcgttggccggtaaaaacgatacatacggataatggttcgaattttacgggtgcgacggtacgtgcggcgtgttggtgggcgggtataaaacaagaatttggtataccgtataatccgcaatcgcaaggtgtagtagaatcgatgaataaagaattaaaaaaaataataggtcaagtacgtgatcaagcggaacatttaaaaacggcggtacaaatggcggtatttatacataattttaaacgtaaaggtggtataggtggttattcggcgggtgaacgtatagtagatataatagcgacggatatacaaacgaaagaattacaaaaacaaataacgaaaatacaaaattttcgtgtatattatcgtgattcgcgtaatccgttatggaaaggtccggcgaaattattatggaaaggtgaaggtgcggtagtaatacaagataattcggatataaaagtagtaccgcgtcgtaaagcgaaaataatacgtgattatggaaaacagatggcaggtgatgattgtgtggcaagtagacaggatgaggattagaacgtggaaatcgttagtaaaacatcatatgtatgtatcgggtaaagcgcgtggttggttttatcgtcatcattatgaatcgccgcatccgcgtatatcgtcggaagtacatataccgttaggtgatgcgcgtttagtaataacgacgtattggggtttacatacgggtgaacgtgattggcatttaggtcaaggtgtatcgatagaatggcgtaaaaaacgttattcgacgcaagtagatccggaattagcggatcaattaatacatttatattattttgattgtttttcggattcggcgatacgtaaagcgttattaggtcatatagtatcgccgcgttgtgaatatcaagcgggtcataataaagtaggttcgttacaatatttagcgttagcggcgttaataacgccgaaaaaaataaaaccgccgttaccgtcggtaacgaaattaacggaagatagatggaacaagccccagaagaccaagggccacagagggagccacacaatgaatggacactagagcttttagaggagcttaagaatgaagctgttagacattttcctaggatttggctccatggcttagggcaacatatctatgaaacttatggggatacttgggcaggagtggaagccataataagaattctgcaacaactgctgtttatccattttcagaattgggtgtcgacatagcagaataggcgttactcgacagaggagagcaagaaatggagccagtagatcctagactagagccctggaagcatccaggaagtcagcctaaaactgcttgtaccaattgctattgtaaaaagtgttgctttcattgccaagtttgtttcataacaaaagccttaggcatctcctatggcaggaagaagcggagacagcgacgaagagctcatcagaacagtcagactcatcaagcttctctatcaaagcagtaagtagtacatgtaatgcaacctataccaatagtagcaatagtagcattagtagtagcaataataatagcaatagttgtgtggtccatagtaatcatagaatataggaaaatattaagacaaagaaaaatagacaggttaattgatagactaatagaaagagcagaagacagtggcaatgagagtgaaggagaaatatcagcacttgtggagatgggggtggagatggggcaccatgctccttgggatgttgatgatctgtagtgcgacggaaaaattatgggtaacggtatattatggtgtaccggtatggaaagaagcgacgacgacgttattttgtgcgtcggatgcgaaagcgtatgatacggaagtacataatgtatgggcgacgcatgcgtgtgtaccgacggatccgaatccgcaagaagtagtattagtaaatgtaacggaaaattttaatatgtggaaaaatgatatggtagaacaaatgcatgaagatataatatcgttatgggatcaatcgttaaaaccgtgtgtaaaattaacgccgttatgtgtatcgttaaaatgtacggatttaaaaaatgatacgaatacgaattcgtcgtcgggtcgtatgataatggaaaaaggtgaaataaaaaattgttcgtttaatatatcgacgtcgatacgtggtaaagtacaaaaagaatatgcgtttttttataaattagatataataccgatagataatgatacgacgtcgtataaattaacgtcgtgtaatacgtcggtaataacgcaagcgtgtccgaaagtatcgtttgaaccgataccgatacattattgtgcgccggcgggttttgcgatattaaaatgtaataataaaacgtttaatggtacgggtccgtgtacgaatgtatcgacggtacaatgtacgcatggtatacgtccggtagtatcgacgcaattattattaaatggttcgttagcggaagaagaagtagtaatacgttcggtaaattttacggataatgcgaaaacgataatagtacaattaaatacgtcggtagaaataaattgtacgcgtccgaataataatacgcgtaaacgtatacgtatacaacgtggtccgggtcgtgcgtttgtaacgataggtaaaataggtaatatgcgtcaagcgcattgtaatatatcgcgtgcgaaatggaataatacgttaaaacaaatagcgtcgaaattacgtgaacaatttggtaataataaaacgataatatttaaacaatcgtcgggtggtgatccggaaatagtaacgcattcgtttaattgtggtggtgaatttttttattgtaattcgacgcaattatttaattcgacgtggtttaattcgacgtggtcgacggaaggttcgaataatacggaaggttcggatacgataacgttaccgtgtcgtataaaacaaataataaatatgtggcaaaaagtaggtaaagcgatgtatgcgccgccgatatcgggtcaaatacgttgttcgtcgaatataacgggtttattattaacgcgtgatggtggtaattcgaataatgaatcggaaatatttcgtccgggtggtggtgatatgcgtgataattggcgttcggaattatataaatataaagtagtaaaaatagaaccgttaggtgtagcgccgacgaaagcgaaacgtcgtgtagtacaacgtgaaaaacgtgcggtaggtataggtgcgttatttttaggttttttaggtgcggcgggttcgacgatgggtgcggcgtcgatgacgttaacggtacaagcgcgtcaattattatcgggtatagtacaacaacaaaataatttattacgtgcgatagaagcgcaacaacatttattacaattaacggtatggggtataaaacaattacaagcgcgtatattagcggtagaacgttatttaaaagatcaacaattattaggtatatggggttgttcgggtaaattaatatgtacgacggcggtaccgtggaatgcgtcgtggtcgaataaatcgttagaacaaatatggaatcatacgacgtggatggaatgggatcgtgaaataaataattatacgtcgttaatacattcgttaatagaagaatcgcaaaatcaacaagaaaaaaatgaacaagaattattagaattagataaatgggcgtcgttatggaattggtttaatataacgaattggttatggtatataaaattatttataatgatagtaggtggtttagtaggtttacgtatagtatttgcggtattatcgatagtaaatcgtgtacgtcaaggttattcgccgttatcgtttcaaacccacctcccaaccccgaggggacccgacaggcccgaaggaatagaagaagaaggtggagagagagacagagacagatccattcgattagtgaacggatccttggcacttatctgggacgatctgcggagcctgtgcctcttcagctaccaccgcttgagagacttactcttgattgtaacgaggattgtggaacttctgggacgcagggggtgggaagccctcaaatattggtggaatctcctacagtattggagtcaggaactaaagaatagtgctgttagcttgctcaatgccacagccatagcagtagctgaggggacagatagggttatagaagtagtacaaggagcttgtagagctattcgccacatacctagaagaataagacagggcttggaaaggattttgctataagatgggtggtaaatggtcgaaatcgtcggtaataggttggccgacggtacgtgaacgtatgcgtcgtgcggaaccggcggcggatcgtgtaggtgcggcgtcgcgtgatttagaaaaacatggtgcgataacgtcgtcgaatacggcggcgacgaatgcggcgtgtgcgtggttagaagcgcaagaagaagaagaagtaggttttccggtaacgccgcaagtaccgttacgtccgatgacgtataaagcggcggtagatttatcgcattttttaaaagaaaaaggtggtttagaaggtttaatacattcgcaacgtcgtcaagatatattagatttatggatatatcatacgcaaggttattttccggattaacaaaattatacgccgggtccgggtgtacgttatccgttaacgtttggttggtgttataaattagtaccggtagaaccggataaaatagaagaagcgaataaaggtgaaaatacgtcgttattacatccggtatcgttacatggtatggatgatccggaacgtgaagtattagaatggcgttttgattcgcgtttagcgtttcatcatgtagcgcgtgaattacatccggaatattttaaaaattgttaacatcgagcttgctacaagggactttccgctggggactttccagggaggcgtggcctgggcgggactggggagtggcgagccctcagatcctgcatataagcagctgctttttgcctgtactgggtctctctggttagaccagatctgagcctgggagctctctggctaactagggaacccactgcttaagcctcaataaagcttgccttgagtgcttc

SEQ ID NO: 36 - DNA, 9181 bp, unknown
  synthetic
ggtctctctggttagaccagatctgagcctgggagctctctggctaactagggaacccactgcttaagcctcaataaagcttgccttgagtgcttcaagtagtgtgtgcccgtctgttgtgtgactctggtaactagagatccctcagacccttttagtcagtgtggaaaatctctagcagtggcgcccgaacagggacctgaaagcgaaagggaaaccagaggagctctctcgacgcaggactcggcttgctgaagcgcgcacggcaagaggcgaggggcggcgactggtgagtacgccaaaaattttgactagcggaggctagaaggagagagatgggagctagagctagcgtacttagcggaggcgaactcgatagatgggaaaaaattagactgagaccagggggaaaaaaaaaatataaactgaaacatatagtatgggctagtagagagttagagagattcgcagtaaacccagggttactcgaaactagcgaagggtgtagacagatactgggacaattgcaacctagtctgcaaaccggatccgaagagcttagatcactatataatacagtcgcaacactatattgtgtacaccaacgaatcgaaattaaggatacgaaagaggcattagacaaaatcgaagaggaacagaataagtctaaaaaaaaagcgcaacaggcagcagccgataccggacatagtaatcaggtatcgcaaaattatccaatcgtacagaatatacagggacaaatggtacaccaagcgatatcacctagaacacttaacgcatgggttaaggtagtcgaagagaaagcatttagtccagaggtaatacctatgtttagcgcattaagcgaaggcgcaacaccacaggatctgaatactatgcttaataccgtaggggggcatcaagccgcaatgcaaatgcttaaagagacaattaacgaagaggcagccgaatgggatagagtgcatcccgtacacgcaggaccaatcgcaccaggacaaatgagagaacctaggggatccgatatagccggaactactagtacattgcaggaacagatagggtggatgactaataatccacctatacccgtaggcgaaatatacaaaagatggataatactgggactgaataagatagttagaatgtatagtccaactagtatactcgatattagacagggacctaaagaaccttttagggattacgtagatagattctataaaacacttagagccgaacaggctagtcaagaggttaagaattggatgacagagacactattagtgcaaaacgctaatcccgattgtaaaactatacttaaggcactaggaccagcagcaacactcgaagaaatgatgacagcatgtcagggagtagggggaccaggacataaagctagagtgttagccgaagctatgtcacaggtaacgaatagcgcaacaattatgatgcaaagaggtaattttagaaaccaacgaaaaatcgttaagtgttttaattgcggaaaagagggacataccgctagaaattgtagggcacctagaaaaaaagggtgttggaaatgcggaaaagagggacatcaaatgaaagattgtaccgaaagacaggctaattttttagggaagatctggccttcctacaagggaaggccagggaattttcttcagagcagaccagagccaacagccccaccagaagagagcttcaggtctggggtagagacaacaactccccctcagaagcaggagccgatagacaaggaactgtatcctttaacttccctcaggtcactctttggcaacgacccctcgtcacaataaagatagggggacaattgaaagaggcactattagacacaggagcagacgatacagtactcgaagaaatgtcactaccaggtagatggaaacctaaaatgataggggggataggggggtttataaaggtaagacaatacgatcagatactaatcgaaatttgcggacataaagcaatcggaacagtgttagtcggacctacacccgtaaacataatcggtaggaatctgttaacacagatagggtgtacattgaattttccaattagtccaatcgaaaccgtacccgtaaaactgaaaccaggtatggacggacctaaggttaagcaatggccattaaccgaagagaaaattaaggcattagtcgaaatttgtaccgaaatggaaaaagagggtaagattagtaagataggaccagagaatccatataatacacccgtattcgcaattaaaaaaaaagatagtacgaaatggagaaagttagtcgattttagagagttaaacaaaagaacacaagacttttgggaggtacagttagggataccacatccagcaggactgaaaaaaaaaaaaagcgtaaccgtattagacgtaggagacgcatactttagcgtaccattagacgaagactttagaaagtataccgcatttacgatacctagtattaataacgaaacaccaggaattaggtatcaatataacgtactgccacagggatggaaagggtcaccagctatattccaatctagtatgactaagatactcgaaccttttagaaaacagaatccagacatagtgatataccaatatatggacgatctatacgtaggtagcgatctagagatagggcaacatagaacgaaaatcgaagagcttagacagcatctgttaagatggggattgactacacctgacaaaaaacaccaaaaagaaccaccattcttatggatgggatacgaattgcatcccgataaatggacagtgcaacctatagtgttacccgaaaaagactcatggacagtaaacgatatacaaaaactggtaggtaagttgaattgggctagtcagatatatcccggaattaaggttaggcaattgtgtaaactgttaaggggaactaaggcactaaccgaagtgataccgttaaccgaagaggcagagttagagttagccgaaaatagagagatacttaaggaacccgtacacggagtgtattacgatcctagtaaggatctgatagccgaaatacaaaaacagggacagggacaatggacatatcagatatatcaggaaccttttaaaaatctgaaaaccggtaagtacgctagaatgaggggagcacatacaaacgacgttaagcaattgaccgaagccgtacaaaaaattacaaccgaatcaatcgtaatttggggtaagacacctaaatttaaattgcctatacaaaaagagacatgggaaacatggtggactgagtattggcaagctacatggatacccgaatgggaattcgtaaatacaccaccattagtgaaattgtggtatcaactcgaaaaagaaccaatcgtaggagccgaaacattttacgtagacggagcagctaatagggaaactaagttaggtaaggcaggatacgttacgaatagggggagacagaaagtcgttacactaaccgatacaactaaccaaaaaaccgaactgcaagcgatatacttagcgttacaggatagcggattagaggtaaacatagtgacagactcacaatacgcattagggattatacaggcacaacccgatcaatccgaaagcgaactagttaatcagataatcgaacaattgattaaaaaagagaaagtgtatctagcatgggtaccagcacataagggaatagggggaaacgaacaggtagataagttagttagcgcaggaattagaaaggtactgtttttagacggaatagacaaagcgcaagacgaacacgaaaaatatcatagtaattggagagctatggctagcgattttaatctaccacccgtagtcgctaaagagatagtcgcatcatgtgataagtgtcaattgaaaggcgaagctatgcacggacaggtcgattgtagtccagggatatggcaattggattgtacacacttagagggtaaggtaatactagtcgcagtacacgtagctagcggatatatcgaagccgaagtgataccagccgaaaccggacaggaaaccgcatactttctgttaaagttagccggtagatggccagttaagactatacataccgataacggatctaattttacaggagcaaccgttagggcagcatgttggtgggcaggaattaaacaggaattcggaataccatataatccacaatcacagggagtagtcgaatctatgaataaagagttaaaaaaaattatcggacaggttagagaccaagccgaacaccttaaaaccgcagtgcaaatggccgtattcatacataattttaaaagaaaaggggggataggggggtatagcgcaggcgaaagaatcgtagacataatcgcaactgacatacagactaaagagttacagaaacagattactaagatacagaattttagagtgtattatagagactctagaaatccattatggaaaggaccagctaaactgttatggaaaggcgaaggcgcagtagtgatacaggataatagcgatattaaggtagtgcctagacgaaaagcgaaaattattagggattatggaaaacagatggcaggtgatgattgtgtggcaagtagacaggatgaggattagaacatggaaatcactagttaagcatcatatgtacgttagcggtaaggctaggggatggttttatagacatcattacgaatcaccacatcctagaatatctagcgaagtgcatataccgttaggcgacgctagattagtgataactacatattggggattgcatacaggcgaaagggattggcatctaggacagggagtgtcaatcgaatggcgaaaaaaaagatatagtacacaggtagacccagagttagccgatcaattgatacacctatattatttcgattgttttagcgatagcgcaattagaaaggcactattagggcatatagtgtcacctagatgcgaatatcaagccggacataataaggtagggtcactgcaatatctagcattagccgcactaattacacctaaaaaaattaaaccaccactacctagcgtaactaagttaaccgaagacagatggaacaagccccagaagaccaagggccacagagggagccacacaatgaatggacactagagcttttagaggagcttaagaatgaagctgttagacattttcctaggatttggctccatggcttagggcaacatatctatgaaacttatggggatacttgggcaggagtggaagccataataagaattctgcaacaactgctgtttatccattttcagaattgggtgtcgacatagcagaataggcgttactcgacagaggagagcaagaaatggagccagtagatcctagactagagccctggaagcatccaggaagtcagcctaaaactgcttgtaccaattgctattgtaaaaagtgttgctttcattgccaagtttgtttcataacaaaagccttaggcatctcctatggcaggaagaagcggagacagcgacgaagagctcatcagaacagtcagactcatcaagcttctctatcaaagcagtaagtagtacatgtaatgcaacctataccaatagtagcaatagtagcattagtagtagcaataataatagcaatagttgtgtggtccatagtaatcatagaatataggaaaatattaagacaaagaaaaatagacaggttaattgatagactaatagaaagagcagaagacagtggcaatgagagtgaaggagaaatatcagcacttgtggagatgggggtggagatggggcaccatgctccttgggatgttgatgatctgtagtgcaaccgaaaaattgtgggttacggtatattacggagtacccgtatggaaagaggcaactactacactattttgcgctagcgacgctaaagcatacgataccgaagtgcataacgtatgggctacacacgcatgcgtacctaccgatcctaatccacaagaggtagtgttagttaacgtaaccgaaaattttaatatgtggaaaaacgatatggtcgaacaaatgcacgaagacataattagcttatgggaccaatcacttaaaccatgtgttaagttgacaccactatgcgtaagtcttaagtgtacagaccttaaaaacgatactaatactaactctagtagcggaagaatgattatggaaaagggagagataaaaaattgttcattcaatattagtacatcaattaggggtaaggtacaaaaagaatacgcatttttttataagttagacataataccaatcgataacgatacaacatcatataagttaactagttgtaatactagcgtaattacacaggcatgtcctaaggtatcattcgaacctataccgatacactattgtgcaccagccggattcgcaatactgaaatgtaataataagacatttaacggaaccggaccatgtactaacgtaagtacagtgcaatgtacacacggaattagacccgtagtgagtacgcaattactgttaaacggatcattagccgaagaggaagtggtaattagatccgttaattttaccgataacgctaaaacaattatagtgcaattgaatactagcgtagagattaattgtactagacctaataataatactagaaaacggattaggatacaaaggggaccaggtagggcattcgtaacaatcggtaagatagggaatatgagacaggcacattgtaatattagtagggctaaatggaataatacacttaaacagatagctagtaagcttagagagcaattcggtaataataagacaattatattcaaacaatctagcggaggggatccagaaatcgtaacacatagttttaattgcggaggcgaatttttttattgtaatagtacacaattgttcaatagtacatggtttaatagtacatggtcaaccgaaggatctaataatacagagggatccgatacaattacactaccatgtaggattaaacagataattaatatgtggcaaaaggtaggtaaggcaatgtacgcaccacctattagcggacaaattagatgtagttcgaatataaccggattactgttaactagagacggagggaattcgaataacgaatccgaaatttttagaccaggggggggagatatgagagacaattggagatccgaattgtataagtataaagtcgttaaaatcgaaccattaggcgtagcacctacaaaagcgaaaagacgggtagtgcaacgcgaaaaaagagccgtagggataggcgcactattcttagggtttttaggcgcagccggatcaactatgggagcagctagtatgacattgacagtgcaagctagacaactgttaagcggaatagtgcaacaacagaataatctgttaagggcaatcgaagcacaacagcatctgttacaattgacagtatgggggattaagcaattgcaggctagaatactcgcagtcgaacggtatctgaaagaccaacaactgttagggatatggggatgtagcggtaagttgatatgtacaaccgcagtaccatggaacgctagttggtctaataaatcactcgaacagatatggaatcatacaacatggatggaatgggatagagagattaacaattatactagtctgatacactcactaatcgaagagtcacaaaaccaacaggaaaaaaacgaacaggaactgttagagttagacaaatgggctagcttatggaattggtttaatattactaattggttatggtatataaaactgtttattatgatagtaggggggttagtcggattgagaatcgtattcgcagtactatcaatcgttaatagggttagacagggatatagtccactatcattccaaacccacctcccaaccccgaggggacccgacaggcccgaaggaatagaagaagaaggtggagagagagacagagacagatccattcgattagtgaacggatccttggcacttatctgggacgatctgcggagcctgtgcctcttcagctaccaccgcttgagagacttactcttgattgtaacgaggattgtggaacttctgggacgcagggggtgggaagccctcaaatattggtggaatctcctacagtattggagtcaggaactaaagaatagtgctgttagcttgctcaatgccacagccatagcagtagctgaggggacagatagggttatagaagtagtacaaggagcttgtagagctattcgccacatacctagaagaataagacagggcttggaaaggattttgctataagatgggaggtaagtggtctaaatctagcgtaatcggatggcctacagttagggaaagaatgcgtagagccgaacctgcagccgatagggtaggcgcagctagtagggatctcgaaaaacacggagcaattactagtagtaatacagccgcaactaacgcagcatgcgcatggttagaggcacaggaagaggaagaggtagggtttcccgtaacaccacaggtaccacttagacctatgacatataaagccgcagtcgatctatcacattttctgaaagagaaaggggggttagagggactgatacattcacagagacgacaagacatactagacttatggatatatcatacacagggatattttccagactagcaaaattatacaccaggaccaggcgtaagatatccattgacattcggatggtgttataaactggtaccagtcgaaccagacaaaatcgaagaggctaacaaaggcgaaaatactagtctgttacatcccgtaagcttacacggaatggacgatccagaaagagaggtactcgaatggagattcgatagtagactcgcattccatcacgtagctagggaattgcatccagagtattttaaaaattgttgacatcgagcttgctacaagggactttccgctggggactttccagggaggcgtggcctgggcgggactggggagtggcgagccctcagatcctgcatataagcagctgctttttgcctgtactgggtctctctggttagaccagatctgagcctgggagctctctggctaactagggaacccactgcttaagcctcaataaagcttgccttgagtgcttc

SEQ ID NO: 37 - DNA, 3309 bp, Rotavirus C
ggctaaaaaaaatggcgcaatcgatagtagtagatggtgattatgatgcgttagcgtcgcgttatttaaaatttgtatatgattttgaaaatgtaacgtatcaaaataattattttgcgacggataaatttaaaaaagatatagaacaatatttaaaatcgatacatgatggtgaaaaaataacgcaatcgaaaatagatgaaaaagaaaaaatattattagatcgtgtaccggcggaagaacgttgtttaatatcgaaattagtatttgcgtatggtaaacatggtaatgtagaaaataaattagtaaaatatggtgtaaaagatgcgttatcgcatgcgccgcaaaaagatgcgaaaccgtatgaaaataatataataacgtcggaaatatttaaagaaaaatcggaatatacggatatatatatggatccgtcgataaatacgtcgtgtcaatcgaattgtcaagcgatgatgtttacgatatcggaaatgaaattaaataatataaaaaatgcggcgcgtttagaaaaattatttacgataatagcggcgacgataaataaatatggtatgccgcgtcataatacgcgttatcgttatgaatgggaaacgatgaaaaataaaccgtatcatttagcggcgtggataaattcgtcgatagaaatgatagcgtgtgtagtagatcatcatacgtatatgatagcgcgtgaattaatagtaaaatcgtttacgaatcgtacgtcgttagcgaaattagtatcgtcgccgatgacggtattaacggcgatgttaccgatacgtggtacgtttataacgacggaaaatttagaattagaatattcgaataaatcgataaattatttaatatcgaaagaaatggcggaagattttatgcaagcgataaaacaattacgtgatgaaggtttagaatatataccggattattatgaaaaatggtttaaatcgccggatccgttaacgtttccgaatatagcgttaatatattcgttttcgtttcatgtaggttatcgtaaacaagcgttatcggatgcggtatatgatcaaataacggtaacgtattcggataatgtaaatatggaaatgtataaagaatattcggaacgtatagaaaatgaaatatttacgatattaaaagataaaataatacatgaagataaacgtttagaagaatatgaattatcggcgttattatcgatgtcgtcggcgtcgaatggtatattacgtgaaataaattttggtggtcaaaaagtacgttcgacgaaaaaaaatatgcatgtaatagatgatatatatcataaaaaatatacgacggatataccgccggtagatgcgcgtaatccgataccgttaggtcgtcgtgatgtaccgggtcgtcgtacgcgtgcgatatttatattaccgtatcaatattttatagcgcaacattcgtttgcggaaataatgttaaattatgcgaaacgtgaacgtgaatattcggaattttattcgcaagcgaatcaagtattatcgtatggtgatgtaacgcgttatttagattcgaattcgatattatgttttacggatgtatcgcaatgggatgcgtcgcaacataatacgaaagtattacgtcgttcgataatacgtgcgatgaaacgtttaaaacaattaacgcataatataaatatacataaagcgataaatatatatatacaatcgcaagaaaatttagaaaattcgtatgtattaatagataaaaaagcgatacaatatggtgcgacggcgtcgggtgaaaaacaaacgaaaataatgaattcgatagcgaataaagcgttaatacaaacggtattaggtaaattaatgacggattatacgtttgatgtaaaaatgatacgtgtagatggtgatgataattatgcgatagtacgttttccgatagcgataacggaaaaattattatcggaatttacgtcgaaattacgttcgtattattcggaaatgaatgtaaaagtaaaagcgttagcgtcgttaacgggttgtgaaatagcgaaacgttatgtagcgggtggtatgttattttttcgtgcgggtgtaaatatattacatcatgaaaaacgtaatcaagattcggcgtatgatatggcggcgacgttatatgcgaattatatagtaaatgcgttacgtggtttaacgatgtcgcgtacgtttatattaacgaaaatatgtcaaatgacgtcgataaaaataacgggtacgttacgtttatttccgatgaaatcgatattagcgttaaattcggcgtttaaagtatttgatgaagtagattatgtaataaattatccgatatcgaatttatttatacaattacaacgtaaattatcgtcgataaaagcgaaatcgaaaatagcggataatatagcgaaatcgccgcaatttaaatcgtatgtagaattattaaataaatcgttaacgacggatgaaaatccgatagtatcggatggtatacgtttaacggaaaaagcgaaattaaattcgtatgcgccgatagcgttagaaaaacgtcgtgatcaattttcgataatggtatcgtttttacaaaatccgacgacgtttaaatcggaaacggtagtaacgataaatgatgtattatattttatatcgggttttataaaaatagattcgtcgacggtattaccgaaagaagaaaataatacgatgccgttattaccggcgataataaaacgtacgttatcgtattttggtttacgtacgcatgattatgatataaaaggttcgtcgtcgacggtatcgaaaataataaaacaatattcggtatatacgccgggtatagaagaattatatgaaatagtaaataaatcggtagatacgatacgtggttattttgcgtcgtttaatgtaccgaaagcggatgtagatacgtatatatcgacgcaaatgtataaacatgatcgttttaaaatattacaagcgtatatatataatttattatcggtaaattatggtatgtatcaattagtagatttaaattcggcgcgtttttttgatcatgtaatacatacgccgatggcgaaaacgccgacggcggtatttatgatagatttagcgttacgtttaaaaataataaatcattgtatagaaaaaggtgaaataataacggtatcggtacatgcgaataaaacggattatttaaaattatggcgtatgttatggaatgtaaaaacgatgaattcgccgtattcgaaaaattcgatgtttgatgaataagagaagtggattgcatattgtggct

SEQ ID NO: 38 - DNA, 3309 bp, Unknown
  synthetic
ggctaaaaaaaatggcacaatcaatcgtagttgacggagattatgatgcattagctagtagatatctaaaattcgtatacgatttcgaaaacgtaacttatcagaataattatttcgcaactgataaatttaaaaaagatatcgaacaatatcttaaatcaatacacgatggagaaaaaattacgcaatctaagatagacgaaaaagaaaaaatactgttagatagagtaccagctgaagaaagatgtctaatatctaagttagtattcgcatatggtaagcatggtaacgttgagaataagttagttaagtatggagttaaggatgcactatcacatgcaccacaaaaagacgctaaaccatacgaaaataatataattactagcgaaatttttaaagaaaaatccgaatatactgatatatatatggatccatcaattaatacatcatgtcaatctaattgtcaagctatgatgtttacgatatccgaaatgaaattgaataatataaaaaacgctgctagactcgaaaaattgtttacaattatagccgctacaattaataagtatggtatgcctagacataatactagatatagatatgaatgggaaactatgaaaaataaaccatatcatttagccgcatggattaattcgtcaatcgaaatgatagcatgcgtagtcgatcatcatacatatatgatagctagagagttaatcgttaaatcatttactaatagaacatcattagcgaaattagtgtcatcacctatgacagtgttaaccgctatgttaccaattagaggtacatttataactactgaaaatctcgaactcgaatattctaataaatcaattaattatctgatatcgaaagaaatggctgaagattttatgcaagctataaaacaattgagagacgaaggattagagtatataccagattattacgaaaaatggtttaaatcaccagatccattaacttttcctaatatagcgttaatatattcattttcatttcacgtagggtatagaaaacaggcactatctgatgcagtatacgatcagattacggttacatattcagataacgttaatatggaaatgtataaagagtattcagaaagaatcgaaaacgaaatttttacgatactgaaagataaaattatacacgaagataaacggttagaggaatacgaactatcagcattactatctatgtcatcagcatcaaacggaatacttagagaaattaatttcggaggacaaaaagttagatcaactaaaaaaaatatgcatgtaatcgatgatatatatcataaaaaatatactactgatataccaccagtagacgctagaaatccgataccattaggtagaagagacgtaccaggtagacgaactagagctatttttatactaccatatcaatattttatagcgcaacattcattcgcagaaattatgcttaattatgctaaaagagaacgcgaatatagcgaattttattcacaggctaatcaggtactatcatacggagatgtaactagatatctagattctaattcgatactatgttttacggatgtatcacaatgggatgctagtcagcataatactaaggtacttagacgatcaattattagagctatgaaaagattgaaacaattgacacataatattaatatacataaagcgataaatatatatatacaatcacaggaaaatctcgaaaattcatatgtgttaatcgataaaaaagcgatacaatacggagctactgcatcaggcgaaaaacagactaaaattatgaattcaatcgctaataaggcattgatacagacagtgttaggtaagttaatgactgattatacattcgatgttaaaatgattagagtagacggagatgataattatgctatagttagatttccgatagcgataaccgaaaaactgttaagcgaatttacatctaaattgcgatcatattattcagaaatgaacgttaaggttaaggcattagcgtcattaacgggatgtgagatagcgaaaagatatgtagccggaggtatgttattttttagagccggagtgaatatattgcatcatgaaaaacgtaatcaggatagtgcatacgatatggcagctacattatacgctaattatatagttaacgcacttagagggttaactatgtcacgaacttttatattgactaagatatgtcaaatgacatcaattaaaattacgggaacacttagattgtttccaatgaaatcaatactcgcacttaatagtgcatttaaggtattcgatgaggtagattatgtaattaattatcctatatctaatctatttatacaattgcaacgaaaactatcatcaattaaagcgaaatctaagatagccgataatatagcgaaatcaccacaatttaaatcatacgttgagttactgaataaatcattgactactgacgaaaatccgatagtgtcagacggaatacggttaacggaaaaagctaaattgaattcatacgcaccaatcgcattagaaaaacgtagagatcaattttcaattatggtatcatttttacagaatcctactacttttaaatccgaaacagtagttacaattaacgatgtattgtattttatatcaggatttataaaaatcgattctagtacagtgttacctaaagaggaaaataatactatgccactattaccagctataattaaacgtacactatcatatttcggattgcgtacacatgattatgatattaagggatcatctagtacagtatcgaaaattataaaacagtattcagtatatacaccaggaatcgaagagttatacgaaatcgttaataaatcagtagatacaattaggggatattttgctagttttaacgtacctaaagctgatgtagatacatatatatcgacacaaatgtataaacatgatagatttaaaatactgcaagcatatatatataatctgttatcagttaattatggtatgtatcaattagtcgatctgaattcagctagattttttgatcatgtaatacatacacctatggctaaaacacctacagcagtttttatgatagatttagcgttaagattgaaaattataaatcattgtatcgaaaaaggcgaaattataacagttagcgtacacgctaataaaactgattatcttaagttatggcgtatgttatggaacgttaagactatgaatagtccatattctaaaaattcaatgtttgacgaataagagaagtggattgcatattgtggct

SEQ ID NO: 39 - DNA, 2736 bp, Rotavirus C
ggcttaaaaagatcagttgaggacaaatcgttcaagatgatatcgcgtaatcgtcgtcgtaataatcaacaaaaaaatatagaaaaagaaaaacaattagaaacgataataaataaagaagtaaaagaaaataaagattcgatgaaagaagataaattagtagtaacggaagaatcgaatggtgatgtaacgacggcgaaagaacaatcgaataatataaatttacaaaaaaatgatttagtaaaagaagtaatgaatatacaaaatcaaacgttaaatacggtagtaacggaaaataaagtagaaatagaagaaatagtaaaaaaatatataccgtcgtataatacggattcgttaatagtaaaaaaattaacggaaatacaagaatcgtcggcgaaaacgtataatacgttatttcgtttatttacgccggtaaaatcgtatttatatgatataaatggtgaaaaaaaattatcgacgcgttggtattggaaattattaaaagatgatttaccggcgggtgattattcggtacgtcaattttttttatcgttatatttaaatgtattagaagaaatgccggattatataatgttacgtgatatggcggtagataatccgtattcggcggaagcgggtaaaatagtagatggtaaatcgaaagaaatattaatagaattatatcaagatcaaatgacggaaggttatatacgtcgttatatgtcggaattacgtcataaaatatcgggtgaaacgaatacggcgaaatatccggcgatattacatccggtagataatgaattaaatcaatattttttagaacatcaattaatacaaccgttaacgacgcgtaatatagcggaattaataccgacgcaattatatcatgatccgaattatgtatttaatatagatgcggcgtttttaacgaattcgcgttttgtaccgccgtatttaacgcaagatcgtataggtttacatgatggttttgaatcgatatgggattcgaaaacgcatgcggattatgtatcggcgcgtcgttttataccggatttaacggaattagtagatgcggaaaaacaaataaaagaaatggcggcgcatttacaattagaagcgataacggtacaagtagaatcgcaatttttagcgggtatatcggcggcggcggcgaatgaagcgtttaaatttataataggttcggtattatcgacgcgtacgatagcggtagaatttataacgtcgaattatatgtcgttagcgtcgtgtatgtatttaatgacgataatgccgtcggaaatatttttacgtgaatcgttagtagcgatgcaattagcgataataaatacgttaatatatccggcgttaggtttagcgcaaatgcattatcaagcgggtgaagtacgtacgccgtttgaattagcggaaatgcaagtagcgaatcgttcgatacgtcaatggttacatcattgtaatacgttacaatttggtcgtcaaataacggaaggtataatacatttacgttttacgaatgatataatgacgggtcgtatagtaaatttattttcgacgatgttagtagcgttatcgtcgcaaccgtttgcgacgtatccgttagattataaacgttcggtacaacgtgcgttacaattattatcgaatcgtacggcgcaaatagcggatttaacgcgtttaatagtatataattatacgacgttatcggcgtgtatagtaatgaatatgcatttagtaggtacgttaacggtagaacgtatacaagcgacgtcgttaacgtcgttaatgatgttaatatcgaataaaacggtaataccggaaccgtcgtcgttattttcgtatttttcgtcgaatataaattttttaacgaattataatgaacaaatagataatgtagtagcggaaataatggcggcgtatcgtttaaatttatatcaacaaaaaatgttaatgttagtaacgcgttttgtatcgaaattatatatatttgatgcgccgaaaataccgccggatcaaatgtatcgtttacgtaatcgtttacgtaatataccggtagaacgtcgtcgtgcggatgtatttcgtataataatgaataatcgtgatttaatagaaaaaacgtcggaacgtatatgtcaaggtgtattattatcgtatacgccgatgccgttaacgtatgtagaagatgtaggtttaacgaatgtaataaatgatacgaattcgtttcaaataataaatatagaagaaatagaaaaaacgggtgattattcggcgataacgaatgcgttattacgtgatacgccgataatattaaaaggtgcgataccgtatgtaacgaattcgtcggtaatagatgtattatcgaaagtagatacgacggtatttgcgtcgatagtaaaagatcgtgatatatcgaaattaaaaccgataaaatttataataaattcggattcgtcggaatattatttagtacataataataaatggacgccgacgacgacgacggcggtatataaagcgcgttcgcaacaatttgatatacaacattcggtatcgatgttagaatcgaatttattttttgtagtatataatgatttatttaaatatataaaaacgacgacggtattaccgataaatgcggtatcgtatgatggtgcgcgtataatgcaagaaacgtaaatgattgtatagtatcatcttgtgacgacctcaaactttgtggct

SEQ ID NO: 40 - DNA, 2736 bp, Unknown
  synthetic
ggcttaaaaagatcagttgaggacaaatcgttcaagatgatatctagaaatagacgtagaaataatcagcaaaaaaatatcgaaaaagaaaaacagttagagacaattattaataaagaggttaaagagaataaggattcaatgaaagaggataagttagtggtaaccgaagaatctaacggagacgttacaaccgctaaagagcaatctaataatattaatctgcaaaaaaacgatttagttaaagaggttatgaatatacagaatcagacacttaatacagtagttaccgaaaataaggttgagatagaagagatagttaaaaaatatataccgtcatataatactgattcattaatcgttaaaaaattaaccgaaatacaggaatctagtgctaaaacttataatacactatttagattgtttacaccagttaaatcatacttatacgatattaatggcgaaaaaaaactatctactagatggtattggaaactgttaaaagacgatctaccagcaggtgattactcagttagacaattttttctatcattatacttaaacgtattagaggaaatgccagattatattatgcttagagatatggcagttgataatccatactcagctgaagcaggtaagatagttgacggtaagtctaaagagatattaatcgaattgtatcaggatcaaatgacagagggatatattagacggtatatgtcagaacttagacataaaatttcaggcgaaactaataccgctaaatatccagctatactgcatccagtagataacgaattgaatcaatattttctcgaacatcaattgatacaaccattaactactagaaatatagccgaattgataccgacacaattgtatcatgatcctaattacgtttttaatatagacgctgcatttttaactaattctagattcgtaccaccatacttaacgcaagataggatagggttacatgacggattcgaatcaatttgggattctaaaacacatgctgattacgtatcagctagacgatttatacccgatttaaccgaattagttgacgctgaaaaacagattaaggaaatggctgcacatttacaactcgaagctattacggtacaggttgaatcacaatttttagccggtattagcgcagcagcagctaacgaagcatttaaatttattataggatcagtgttatcaactagaactatagcagtcgaatttattacatctaattatatgtcattagctagttgtatgtatcttatgacaattatgcctagcgaaatttttttacgcgaatcattagtcgctatgcaattagctattattaatacacttatatatccagcattagggttagcgcaaatgcattatcaggcaggtgaggttagaacaccattcgaattagccgaaatgcaagttgcgaatagatcaattagacaatggttacatcattgtaatacattacaattcggtaggcaaattaccgaaggtattatacatcttagatttactaacgatattatgacaggtaggatagttaatctattttcgactatgttagttgcgttatcatcacaaccattcgctacatatccattagattataaaagatcagtgcaacgagcattacaattgttatctaatagaaccgctcaaatagctgatttaactagactgatagtgtataattatactacattatccgcatgcatagttatgaatatgcatttagtgggtacacttacagtcgaacgtatacaggctacatcattaacatcattaatgatgttaatttctaataaaacagttatacccgaaccatcatcattattttcatatttttcatctaatattaattttttaactaattataacgaacagatagataacgtagttgcggaaattatggctgcatatagattgaatctatatcaacaaaaaatgttaatgttagtgactagattcgtaagtaagttatatatattcgatgcacctaaaattccaccagatcaaatgtatagacttagaaatagacttagaaatataccagtcgaaagacgtagagcagacgtatttagaattattatgaataatagggatttaatcgaaaaaactagcgaaagaatttgtcagggagtgttactatcatatacacctatgccattaacatacgttgaagacgtaggattaactaacgtaattaacgatactaattcgtttcaaattattaatatcgaagaaatcgaaaaaacaggtgattactcagctattactaatgcactattaagggatacacctattatacttaagggagctataccatacgttacgaattcgtcagtgatagacgtactatctaaggtagatactacagtattcgctagtatagttaaggatagggatatatctaagttaaaaccaattaaatttataattaattctgattctagcgaatattatttagtgcataataataaatggacacctactactactactgcagtgtataaagctagatcacaacaattcgatatacaacatagcgtatctatgctcgaatctaatctatttttcgtagtgtataacgatctatttaaatatattaaaactactacagtgttaccaattaacgctgtatcatacgatggagctagaattatgcaagaaacataaatgattgtatagtatcatcttgtgacgacctcaaactttgtggct

SEQ ID NO: 41 - DNA, 29751 bp, coronavirus
atattaggtttttacctacccaggaaaagccaaccaacctcgatctcttgtagatctgttctctaaacgaactttaaaatctgtgtagctgtcgctcggctgcatgcctagtgcacctacgcagtataaacaataataaattttactgtcgttgacaagaaacgagtaactcgtccctcttctgcagactgcttacggtttcgtccgtgttgcagtcgatcatcagcatacctaggtttcgtccgggtgtgaccgaaaggtaagatggaatcgttagtattaggtgtaaatgaaaaaacgcatgtacaattatcgttaccggtattacaagtacgtgatgtattagtacgtggttttggtgattcggtagaagaagcgttatcggaagcgcgtgaacatttaaaaaatggtacgtgtggtttagtagaattagaaaaaggtgtattaccgcaattagaacaaccgtatgtatttataaaacgttcggatgcgttatcgacgaatcatggtcataaagtagtagaattagtagcggaaatggatggtatacaatatggtcgttcgggtataacgttaggtgtattagtaccgcatgtaggtgaaacgccgatagcgtatcgtaatgtattattacgtaaaaatggtaataaaggtgcgggtggtcattcgtatggtatagatttaaaatcgtatgatttaggtgatgaattaggtacggatccgatagaagattatgaacaaaattggaatacgaaacatggttcgggtgcgttacgtgaattaacgcgtgaattaaatggtggtgcggtaacgcgttatgtagataataatttttgtggtccggatggttatccgttagattgtataaaagattttttagcgcgtgcgggtaaatcgatgtgtacgttatcggaacaattagattatatagaatcgaaacgtggtgtatattgttgtcgtgatcatgaacatgaaatagcgtggtttacggaacgttcggataaatcgtatgaacatcaaacgccgtttgaaataaaatcggcgaaaaaatttgatacgtttaaaggtgaatgtccgaaatttgtatttccgttaaattcgaaagtaaaagtaatacaaccgcgtgtagaaaaaaaaaaaacggaaggttttatgggtcgtatacgttcggtatatccggtagcgtcgccgcaagaatgtaataatatgcatttatcgacgttaatgaaatgtaatcattgtgatgaagtatcgtggcaaacgtgtgattttttaaaagcgacgtgtgaacattgtggtacggaaaatttagtaatagaaggtccgacgacgtgtggttatttaccgacgaatgcggtagtaaaaatgccgtgtccggcgtgtcaagatccggaaataggtccggaacattcggtagcggattatcataatcattcgaatatagaaacgcgtttacgtaaaggtggtcgtacgcgttgttttggtggttgtgtatttgcgtatgtaggttgttataataaacgtgcgtattgggtaccgcgtgcgtcggcggatataggttcgggtcatacgggtataacgggtgataatgtagaaacgttaaatgaagatttattagaaatattatcgcgtgaacgtgtaaatataaatatagtaggtgattttcatttaaatgaagaagtagcgataatattagcgtcgttttcggcgtcgacgtcggcgtttatagatacgataaaatcgttagattataaatcgtttaaaacgatagtagaatcgtgtggtaattataaagtaacgaaaggtaaaccggtaaaaggtgcgtggaatataggtcaacaacgttcggtattaacgccgttatgtggttttccgtcgcaagcggcgggtgtaatacgttcgatatttgcgcgtacgttagatgcggcgaatcattcgataccggatttacaacgtgcggcggtaacgatattagatggtatatcggaacaatcgttacgtttagtagatgcgatggtatatacgtcggatttattaacgaattcggtaataataatggcgtatgtaacgggtggtttagtacaacaaacgtcgcaatggttatcgaatttattaggtacgacggtagaaaaattacgtccgatatttgaatggatagaagcgaaattatcggcgggtgtagaatttttaaaagatgcgtgggaaatattaaaatttttaataacgggtgtatttgatatagtaaaaggtcaaatacaagtagcgtcggataatataaaagattgtgtaaaatgttttatagatgtagtaaataaagcgttagaaatgtgtatagatcaagtaacgatagcgggtgcgaaattacgttcgttaaatttaggtgaagtatttatagcgcaatcgaaaggtttatatcgtcaatgtatacgtggtaaagaacaattacaattattaatgccgttaaaagcgccgaaagaagtaacgtttttagaaggtgattcgcatgatacggtattaacgtcggaagaagtagtattaaaaaatggtgaattagaagcgttagaaacgccggtagattcgtttacgaatggtgcgatagtaggtacgccggtatgtgtaaatggtttaatgttattagaaataaaagataaagaacaatattgtgcgttatcgccgggtttattagcgacgaataatgtatttcgtttaaaaggtggtgcgccgataaaaggtgtaacgtttggtgaagatacggtatgggaagtacaaggttataaaaatgtacgtataacgtttgaattagatgaacgtgtagataaagtattaaatgaaaaatgttcggtatatacggtagaatcgggtacggaagtaacggaatttgcgtgtgtagtagcggaagcggtagtaaaaacgttacaaccggtatcggatttattaacgaatatgggtatagatttagatgaatggtcggtagcgacgttttatttatttgatgatgcgggtgaagaaaatttttcgtcgcgtatgtattgttcgttttatccgccggatgaagaagaagaagatgatgcggaatgtgaagaagaagaaatagatgaaacgtgtgaacatgaatatggtacggaagatgattatcaaggtttaccgttagaatttggtgcgtcggcggaaacggtacgtgtagaagaagaagaagaagaagattggttagatgatacgacggaacaatcggaaatagaaccggaaccggaaccgacgccggaagaaccggtaaatcaatttacgggttatttaaaattaacggataatgtagcgataaaatgtgtagatatagtaaaagaagcgcaatcggcgaatccgatggtaatagtaaatgcggcgaatatacatttaaaacatggtggtggtgtagcgggtgcgttaaataaagcgacgaatggtgcgatgcaaaaagaatcggatgattatataaaattaaatggtccgttaacggtaggtggttcgtgtttattatcgggtcataatttagcgaaaaaatgtttacatgtagtaggtccgaatttaaatgcgggtgaagatatacaattattaaaagcggcgtatgaaaattttaattcgcaagatatattattagcgccgttattatcggcgggtatatttggtgcgaaaccgttacaatcgttacaagtatgtgtacaaacggtacgtacgcaagtatatatagcggtaaatgataaagcgttatatgaacaagtagtaatggattatttagataatttaaaaccgcgtgtagaagcgccgaaacaagaagaaccgccgaatacggaagattcgaaaacggaagaaaaatcggtagtacaaaaaccggtagatgtaaaaccgaaaataaaagcgtgtatagatgaagtaacgacgacgttagaagaaacgaaatttttaacgaataaattattattatttgcggatataaatggtaaattatatcatgattcgcaaaatatgttacgtggtgaagatatgtcgtttttagaaaaagatgcgccgtatatggtaggtgatgtaataacgtcgggtgatataacgtgtgtagtaataccgtcgaaaaaagcgggtggtacgacggaaatgttatcgcgtgcgttaaaaaaagtaccggtagatgaatatataacgacgtatccgggtcaaggttgtgcgggttatacgttagaagaagcgaaaacggcgttaaaaaaatgtaaatcggcgttttatgtattaccgtcggaagcgccgaatgcgaaagaagaaatattaggtacggtatcgtggaatttacgtgaaatgttagcgcatgcggaagaaacgcgtaaattaatgccgatatgtatggatgtacgtgcgataatggcgacgatacaacgtaaatataaaggtataaaaatacaagaaggtatagtagattatggtgtacgtttttttttttatacgtcgaaagaaccggtagcgtcgataataacgaaattaaattcgttaaatgaaccgttagtaacgatgccgataggttatgtaacgcatggttttaatttagaagaagcggcgcgttgtatgcgttcgttaaaagcgccggcggtagtatcggtatcgtcgccggatgcggtaacgacgtataatggttatttaacgtcgtcgtcgaaaacgtcggaagaacattttgtagaaacggtatcgttagcgggttcgtatcgtgattggtcgtattcgggtcaacgtacggaattaggtgtagaatttttaaaacgtggtgataaaatagtatatcatacgttagaatcgccggtagaatttcatttagatggtgaagtattatcgttagataaattaaaatcgttattatcgttacgtgaagtaaaaacgataaaagtatttacgacggtagataatacgaatttacatacgcaattagtagatatgtcgatgacgtatggtcaacaatttggtccgacgtatttagatggtgcggatgtaacgaaaataaaaccgcatgtaaatcatgaaggtaaaacgttttttgtattaccgtcggatgatacgttacgttcggaagcgtttgaatattatcatacgttagatgaatcgtttttaggtcgttatatgtcggcgttaaatcatacgaaaaaatggaaatttccgcaagtaggtggtttaacgtcgataaaatgggcggataataattgttatttatcgtcggtattattagcgttacaacaattagaagtaaaatttaatgcgccggcgttacaagaagcgtattatcgtgcgcgtgcgggtgatgcggcgaatttttgtgcgttaatattagcgtattcgaataaaacggtaggtgaattaggtgatgtacgtgaaacgatgacgcatttattacaacatgcgaatttagaatcggcgaaacgtgtattaaatgtagtatgtaaacattgtggtcaaaaaacgacgacgttaacgggtgtagaagcggtaatgtatatgggtacgttatcgtatgataatttaaaaacgggtgtatcgataccgtgtgtatgtggtcgtgatgcgacgcaatatttagtacaacaagaatcgtcgtttgtaatgatgtcggcgccgccggcggaatataaattacaacaaggtacgtttttatgtgcgaatgaatatacgggtaattatcaatgtggtcattatacgcatataacggcgaaagaaacgttatatcgtatagatggtgcgcatttaacgaaaatgtcggaatataaaggtccggtaacggatgtattttataaagaaacgtcgtatacgacgacgataaaaccggtatcgtataaattagatggtgtaacgtatacggaaatagaaccgaaattagatggttattataaaaaagataatgcgtattatacggaacaaccgatagatttagtaccgacgcaaccgttaccgaatgcgtcgtttgataattttaaattaacgtgttcgaatacgaaatttgcggatgatttaaatcaaatgacgggttttacgaaaccggcgtcgcgtgaattatcggtaacgttttttccggatttaaatggtgatgtagtagcgatagattatcgtcattattcggcgtcgtttaaaaaaggtgcgaaattattacataaaccgatagtatggcatataaatcaagcgacgacgaaaacgacgtttaaaccgaatacgtggtgtttacgttgtttatggtcgacgaaaccggtagatacgtcgaattcgtttgaagtattagcggtagaagatacgcaaggtatggataatttagcgtgtgaatcgcaacaaccgacgtcggaagaagtagtagaaaatccgacgatacaaaaagaagtaatagaatgtgatgtaaaaacgacggaagtagtaggtaatgtaatattaaaaccgtcggatgaaggtgtaaaagtaacgcaagaattaggtcatgaagatttaatggcggcgtatgtagaaaatacgtcgataacgataaaaaaaccgaatgaattatcgttagcgttaggtttaaaaacgatagcgacgcatggtatagcggcgataaattcggtaccgtggtcgaaaatattagcgtatgtaaaaccgtttttaggtcaagcggcgataacgacgtcgaattgtgcgaaacgtttagcgcaacgtgtatttaataattatatgccgtatgtatttacgttattatttcaattatgtacgtttacgaaatcgacgaattcgcgtatacgtgcgtcgttaccgacgacgatagcgaaaaattcggtaaaatcggtagcgaaattatgtttagatgcgggtataaattatgtaaaatcgccgaaattttcgaaattatttacgatagcgatgtggttattattattatcgatatgtttaggttcgttaatatgtgtaacggcggcgtttggtgtattattatcgaattttggtgcgccgtcgtattgtaatggtgtacgtgaattatatttaaattcgtcgaatgtaacgacgatggatttttgtgaaggttcgtttccgtgttcgatatgtttatcgggtttagattcgttagattcgtatccggcgttagaaacgatacaagtaacgatatcgtcgtataaattagatttaacgatattaggtttagcggcggaatgggtattagcgtatatgttatttacgaaatttttttatttattaggtttatcggcgataatgcaagtattttttggttattttgcgtcgcattttatatcgaattcgtggttaatgtggtttataatatcgatagtacaaatggcgccggtatcggcgatggtacgtatgtatatattttttgcgtcgttttattatatatggaaatcgtatgtacatataatggatggttgtacgtcgtcgacgtgtatgatgtgttataaacgtaatcgtgcgacgcgtgtagaatgtacgacgatagtaaatggtatgaaacgttcgttttatgtatatgcgaatggtggtcgtggtttttgtaaaacgcataattggaattgtttaaattgtgatacgttttgtacgggttcgacgtttatatcggatgaagtagcgcgtgatttatcgttacaatttaaacgtccgataaatccgacggatcaatcgtcgtatatagtagattcggtagcggtaaaaaatggtgcgttacatttatattttgataaagcgggtcaaaaaacgtatgaacgtcatccgttatcgcattttgtaaatttagataatttacgtgcgaataatacgaaaggttcgttaccgataaatgtaatagtatttgatggtaaatcgaaatgtgatgaatcggcgtcgaaatcggcgtcggtatattattcgcaattaatgtgtcaaccgatattattattagatcaagcgttagtatcggatgtaggtgattcgacggaagtatcggtaaaaatgtttgatgcgtatgtagatacgttttcggcgacgttttcggtaccgatggaaaaattaaaagcgttagtagcgacggcgcattcggaattagcgaaaggtgtagcgttagatggtgtattatcgacgtttgtatcggcggcgcgtcaaggtgtagtagatacggatgtagatacgaaagatgtaatagaatgtttaaaattatcgcatcattcggatttagaagtaacgggtgattcgtgtaataattttatgttaacgtataataaagtagaaaatatgacgccgcgtgatttaggtgcgtgtatagattgtaatgcgcgtcatataaatgcgcaagtagcgaaatcgcataatgtatcgttaatatggaatgtaaaagattatatgtcgttatcggaacaattacgtaaacaaatacgttcggcggcgaaaaaaaataatataccgtttcgtttaacgtgtgcgacgacgcgtcaagtagtaaatgtaataacgacgaaaatatcgttaaaaggtggtaaaatagtatcgacgtgttttaaattaatgttaaaagcgacgttattatgtgtattagcggcgttagtatgttatatagtaatgccggtacatacgttatcgatacatgatggttatacgaatgaaataataggttataaagcgatacaagatggtgtaacgcgtgatataatatcgacggatgattgttttgcgaataaacatgcgggttttgatgcgtggttttcgcaacgtggtggttcgtataaaaatgataaatcgtgtccggtagtagcggcgataataacgcgtgaaataggttttatagtaccgggtttaccgggtacggtattacgtgcgataaatggtgattttttacattttttaccgcgtgtattttcggcggtaggtaatatatgttatacgccgtcgaaattaatagaatattcggattttgcgacgtcggcgtgtgtattagcggcggaatgtacgatatttaaagatgcgatgggtaaaccggtaccgtattgttatgatacgaatttattagaaggttcgatatcgtattcggaattacgtccggatacgcgttatgtattaatggatggttcgataatacaatttccgaatacgtatttagaaggttcggtacgtgtagtaacgacgtttgatgcggaatattgtcgtcatggtacgtgtgaacgttcggaagtaggtatatgtttatcgacgtcgggtcgttgggtattaaataatgaacattatcgtgcgttatcgggtgtattttgtggtgtagatgcgatgaatttaatagcgaatatatttacgccgttagtacaaccggtaggtgcgttagatgtatcggcgtcggtagtagcgggtggtataatagcgatattagtaacgtgtgcggcgtattattttatgaaatttcgtcgtgtatttggtgaatataatcatgtagtagcggcgaatgcgttattatttttaatgtcgtttacgatattatgtttagtaccggcgtattcgtttttaccgggtgtatattcggtattttatttatatttaacgttttattttacgaatgatgtatcgtttttagcgcatttacaatggtttgcgatgttttcgccgatagtaccgttttggataacggcgatatatgtattttgtatatcgttaaaacattgtcattggttttttaataattatttacgtaaacgtgtaatgtttaatggtgtaacgttttcgacgtttgaagaagcggcgttatgtacgtttttattaaataaagaaatgtatttaaaattacgttcggaaacgttattaccgttaacgcaatataatcgttatttagcgttatataataaatataaatatttttcgggtgcgttagatacgacgtcgtatcgtgaagcggcgtgttgtcatttagcgaaagcgttaaatgatttttcgaattcgggtgcggatgtattatatcaaccgccgcaaacgtcgataacgtcggcggtattacaatcgggttttcgtaaaatggcgtttccgtcgggtaaagtagaaggttgtatggtacaagtaacgtgtggtacgacgacgttaaatggtttatggttagatgatacggtatattgtccgcgtcatgtaatatgtacggcggaagatatgttaaatccgaattatgaagatttattaatacgtaaatcgaatcattcgtttttagtacaagcgggtaatgtacaattacgtgtaataggtcattcgatgcaaaattgtttattacgtttaaaagtagatacgtcgaatccgaaaacgccgaaatataaatttgtacgtatacaaccgggtcaaacgttttcggtattagcgtgttataatggttcgccgtcgggtgtatatcaatgtgcgatgcgtccgaatcatacgataaaaggttcgtttttaaatggttcgtgtggttcggtaggttttaatatagattatgattgtgtatcgttttgttatatgcatcatatggaattaccgacgggtgtacatgcgggtacggatttagaaggtaaattttatggtccgtttgtagatcgtcaaacggcgcaagcggcgggtacggatacgacgataacgttaaatgtattagcgtggttatatgcggcggtaataaatggtgatcgttggtttttaaatcgttttacgacgacgttaaatgattttaatttagtagcgatgaaatataattatgaaccgttaacgcaagatcatgtagatatattaggtccgttatcggcgcaaacgggtatagcggtattagatatgtgtgcggcgttaaaagaattattacaaaatggtatgaatggtcgtacgatattaggttcgacgatattagaagatgaatttacgccgtttgatgtagtacgtcaatgttcgggtgtaacgtttcaaggtaaatttaaaaaaatagtaaaaggtacgcatcattggatgttattaacgtttttaacgtcgttattaatattagtacaatcgacgcaatggtcgttatttttttttgtatatgaaaatgcgtttttaccgtttacgttaggtataatggcgatagcggcgtgtgcgatgttattagtaaaacataaacatgcgtttttatgtttatttttattaccgtcgttagcgacggtagcgtattttaatatggtatatatgccggcgtcgtgggtaatgcgtataatgacgtggttagaattagcggatacgtcgttatcgggttatcgtttaaaagattgtgtaatgtatgcgtcggcgttagtattattaatattaatgacggcgcgtacggtatatgatgatgcggcgcgtcgtgtatggacgttaatgaatgtaataacgttagtatataaagtatattatggtaatgcgttagatcaagcgatatcgatgtgggcgttagtaatatcggtaacgtcgaattattcgggtgtagtaacgacgataatgtttttagcgcgtgcgatagtatttgtatgtgtagaatattatccgttattatttataacgggtaatacgttacaatgtataatgttagtatattgttttttaggttattgttgttgttgttattttggtttattttgtttattaaatcgttattttcgtttaacgttaggtgtatatgattatttagtatcgacgcaagaatttcgttatatgaattcgcaaggtttattaccgccgaaatcgtcgatagatgcgtttaaattaaatataaaattattaggtataggtggtaaaccgtgtataaaagtagcgacggtacaatcgaaaatgtcggatgtaaaatgtacgtcggtagtattattatcggtattacaacaattacgtgtagaatcgtcgtcgaaattatgggcgcaatgtgtacaattacataatgatatattattagcgaaagatacgacggaagcgtttgaaaaaatggtatcgttattatcggtattattatcgatgcaaggtgcggtagatataaatcgtttatgtgaagaaatgttagataatcgtgcgacgttacaagcgatagcgtcggaattttcgtcgttaccgtcgtatgcggcgtatgcgacggcgcaagaagcgtatgaacaagcggtagcgaatggtgattcggaagtagtattaaaaaaattaaaaaaatcgttaaatgtagcgaaatcggaatttgatcgtgatgcggcgatgcaacgtaaattagaaaaaatggcggatcaagcgatgacgcaaatgtataaacaagcgcgttcggaagataaacgtgcgaaagtaacgtcggcgatgcaaacgatgttatttacgatgttacgtaaattagataatgatgcgttaaataatataataaataatgcgcgtgatggttgtgtaccgttaaatataataccgttaacgacggcggcgaaattaatggtagtagtaccggattatggtacgtataaaaatacgtgtgatggtaatacgtttacgtatgcgtcggcgttatgggaaatacaacaagtagtagatgcggattcgaaaatagtacaattatcggaaataaatatggataattcgccgaatttagcgtggccgttaatagtaacggcgttacgtgcgaattcggcggtaaaattacaaaataatgaattatcgccggtagcgttacgtcaaatgtcgtgtgcggcgggtacgacgcaaacggcgtgtacggatgataatgcgttagcgtattataataattcgaaaggtggtcgttttgtattagcgttattatcggatcatcaagatttaaaatgggcgcgttttccgaaatcggatggtacgggtacgatatatacggaattagaaccgccgtgtcgttttgtaacggatacgccgaaaggtccgaaagtaaaatatttatattttataaaaggtttaaataatttaaatcgtggtatggtattaggttcgttagcggcgacggtacgtttacaagcgggtaatgcgacggaagtaccggcgaattcgacggtattatcgttttgtgcgtttgcggtagatccggcgaaagcgtataaagattatttagcgtcgggtggtcaaccgataacgaattgtgtaaaaatgttatgtacgcatacgggtacgggtcaagcgataacggtaacgccggaagcgaatatggatcaagaatcgtttggtggtgcgtcgtgttgtttatattgtcgttgtcatatagatcatccgaatccgaaaggtttttgtgatttaaaaggtaaatatgtacaaataccgacgacgtgtgcgaatgatccggtaggttttacgttacgtaatacggtatgtacggtatgtggtatgtggaaaggttatggttgttcgtgtgatcaattacgtgaaccgttaatgcaatcggcggatgcgtcgacgtttttaaatgggtttgcggtgtaagtgcggcgcgtttaacgccgtgtggtacgggtacgtcgacggatgtagtatatcgtgcgtttgatatatataatgaaaaagtagcgggttttgcgaaatttttaaaaacgaattgttgtcgttttcaagaaaaagatgaagaaggtaatttattagattcgtattttgtagtaaaacgtcatacgatgtcgaattatcaacatgaagaaacgatatataatttagtaaaagattgtccggcggtagcggtacatgatttttttaaatttcgtgtagatggtgatatggtaccgcatatatcgcgtcaacgtttaacgaaatatacgatggcggatttagtatatgcgttacgtcattttgatgaaggtaattgtgatacgttaaaagaaatattagtaacgtataattgttgtgatgatgattattttaataaaaaagattggtatgattttgtagaaaatccggatatattacgtgtatatgcgaatttaggtgaacgtgtacgtcaatcgttattaaaaacggtacaattttgtgatgcgatgcgtgatgcgggtatagtaggtgtattaacgttagataatcaagatttaaatggtaattggtatgattttggtgattttgtacaagtagcgccgggttgtggtgtaccgatagtagattcgtattattcgttattaatgccgatattaacgttaacgcgtgcgttagcggcggaatcgcatatggatgcggatttagcgaaaccgttaataaaatgggatttattaaaatatgattttacggaagaacgtttatgtttatttgatcgttattttaaatattgggatcaaacgtatcatccgaattgtataaattgtttagatgatcgttgtatattacattgtgcgaattttaatgtattattttcgacggtatttccgccgacgtcgtttggtccgttagtacgtaaaatatttgtagatggtgtaccgtttgtagtatcgacgggttatcattttcgtgaattaggtgtagtacataatcaagatgtaaatttacattcgtcgcgtttatcgtttaaagaattattagtatatgcggcggatccggcgatgcatgcggcgtcgggtaatttattattagataaacgtacgacgtgtttttcggtagcggcgttaacgaataatgtagcgtttcaaacggtaaaaccgggtaattttaataaagatttttatgattttgcggtatcgaaaggtttttttaaagaaggttcgtcggtagaattaaaacattttttttttgcgcaagatggtaatgcggcgatatcggattatgattattatcgttataatttaccgacgatgtgtgatatacgtcaattattatttgtagtagaagtagtagataaatattttgattgttatgatggtggttgtataaatgcgaatcaagtaatagtaaataatttagataaatcggcgggttttccgtttaataaatggggtaaagcgcgtttatattatgattcgatgtcgtatgaagatcaagatgcgttatttgcgtatacgaaacgtaatgtaataccgacgataacgcaaatgaatttaaaatatgcgatatcggcgaaaaatcgtgcgcgtacggtagcgggtgtatcgatatgttcgacgatgacgaatcgtcaatttcatcaaaaattattaaaatcgatagcggcgacgcgtggtgcgacggtagtaataggtacgtcgaaattttatggtggttggcataatatgttaaaaacggtatattcggatgtagaaacgccgcatttaatgggttgggattatccgaaatgtgatcgtgcgatgccgaatatgttacgtataatggcgtcgttagtattagcgcgtaaacataatacgtgttgtaatttatcgcatcgtttttatcgtttagcgaatgaatgtgcgcaagtattatcggaaatggtaatgtgtggtggttcgttatatgtaaaaccgggtggtacgtcgtcgggtgatgcgacgacggcgtatgcgaattcggtatttaatatatgtcaagcggtaacggcgaatgtaaatgcgttattatcgacggatggtaataaaatagcggataaatatgtacgtaatttacaacatcgtttatatgaatgtttatatcgtaatcgtgatgtagatcatgaatttgtagatgaattttatgcgtatttacgtaaacatttttcgatgatgatattatcggatgatgcggtagtatgttataattcgaattatgcggcgcaaggtttagtagcgtcgataaaaaattttaaagcggtattatattatcaaaataatgtatttatgtcggaagcgaaatgttggacggaaacggatttaacgaaaggtccgcatgaattttgttcgcaacatacgatgttagtaaaacaaggtgatgattatgtatatttaccgtatccggatccgtcgcgtatattaggtgcgggttgttttgtagatgatatagtaaaaacggatggtacgttaatgatagaacgttttgtatcgttagcgatagatgcgtatccgttaacgaaacatccgaatcaagaatatgcggatgtatttcatttatatttacaatatatacgtaaattacatgatgaattaacgggtcatatgttagatatgtattcggtaatgttaacgaatgataatacgtcgcgttattgggaaccggaattttatgaagcgatgtatacgccgcatacggtattacaagcggtaggtgcgtgtgtattatgtaattcgcaaacgtcgttacgttgtggtgcgtgtatacgtcgtccgtttttatgttgtaaatgttgttatgatcatgtaatatcgacgtcgcataaattagtattatcggtaaatccgtatgtatgtaatgcgccgggttgtgatgtaacggatgtaacgcaattatatttaggtggtatgtcgtattattgtaaatcgcataaaccgccgatatcgtttccgttatgtgcgaatggtcaagtatttggtttatataaaaatacgtgtgtaggttcggataatgtaacggattttaatgcgatagcgacgtgtgattggacgaatgcgggtgattatatattagcgaatacgtgtacggaacgtttaaaattatttgcggcggaaacgttaaaagcgacggaagaaacgtttaaattatcgtatggtatagcgacggtacgtgaagtattatcggatcgtgaattacatttatcgtgggaagtaggtaaaccgcgtccgccgttaaatcgtaattatgtatttacgggttatcgtgtaacgaaaaattcgaaagtacaaataggtgaatatacgtttgaaaaaggtgattatggtgatgcggtagtatatcgtggtacgacgacgtataaattaaatgtaggtgattattttgtattaacgtcgcatacggtaatgccgttatcggcgccgacgttagtaccgcaagaacattatgtacgtataacgggtttatatccgacgttaaatatatcggatgaattttcgtcgaatgtagcgaattatcaaaaagtaggtatgcaaaaatattcgacgttacaaggtccgccgggtacgggtaaatcgcattttgcgataggtttagcgttatattatccgtcggcgcgtatagtatatacggcgtgttcgcatgcggcggtagatgcgttatgtgaaaaagcgttaaaatatttaccgatagataaatgttcgcgtataataccggcgcgtgcgcgtgtagaatgttttgataaatttaaagtaaattcgacgttagaacaatatgtattttgtacggtaaatgcgttaccggaaacgacggcggatatagtagtatttgatgaaatatcgatggcgacgaattatgatttatcggtagtaaatgcgcgtttacgtgcgaaacattatgtatatataggtgatccggcgcaattaccggcgccgcgtacgttattaacgaaaggtacgttagaaccggaatattttaattcggtatgtcgtttaatgaaaacgataggtccggatatgtttttaggtacgtgtcgtcgttgtccggcggaaatagtagatacggtatcggcgttagtatatgataataaattaaaagcgcataaagataaatcggcgcaatgttttaaaatgttttataaaggtgtaataacgcatgatgtatcgtcggcgataaatcgtccgcaaataggtgtagtacgtgaatttttaacgcgtaatccggcgtggcgtaaagcggtatttatatcgccgtataattcgcaaaatgcggtagcgtcgaaaatattaggtttaccgacgcaaacggtagattcgtcgcaaggttcggaatatgattatgtaatatttacgcaaacgacggaaacggcgcattcgtgtaatgtaaatcgttttaatgtagcgataacgcgtgcgaaaataggtatattatgtataatgtcggatcgtgatttatatgataaattacaatttacgtcgttagaaataccgcgtcgtaatgtagcgacgttacaagcggaaaatgtaacgggtttatttaaagattgttcgaaaataataacgggtttacatccgacgcaagcgccgacgcatttatcggtagatataaaatttaaaacggaaggtttatgtgtagatataccgggtataccgaaagatatgacgtatcgtcgtttaatatcgatgatgggttttaaaatgaattatcaagtaaatggttatccgaatatgtttataacgcgtgaagaagcgatacgtcatgtacgtgcgtggataggttttgatgtagaaggttgtcatgcgacgcgtgatgcggtaggtacgaatttaccgttacaattaggtttttcgacgggtgtaaatttagtagcggtaccgacgggttatgtagatacggaaaataatacggaatttacgcgtgtaaatgcgaaaccgccgccgggtgatcaatttaaacatttaataccgttaatgtataaaggtttaccgtggaatgtagtacgtataaaaatagtacaaatgttatcggatacgttaaaaggtttatcggatcgtgtagtatttgtattatgggcgcatggttttgaattaacgtcgatgaaatattttgtaaaaataggtccggaacgtacgtgttgtttatgtgataaacgtgcgacgtgtttttcgacgtcgtcggatacgtatgcgtgttggaatcattcggtaggttttgattatgtatataatccgtttatgatagatgtacaacaatggggttttacgggtaatttacaatcgaatcatgatcaacattgtcaagtacatggtaatgcgcatgtagcgtcgtgtgatgcgataatgacgcgttgtttagcggtacatgaatgttttgtaaaacgtgtagattggtcggtagaatatccgataataggtgatgaattacgtgtaaattcggcgtgtcgtaaagtacaacatatggtagtaaaatcggcgttattagcggataaatttccggtattacatgatataggtaatccgaaagcgataaaatgtgtaccgcaagcggaagtagaatggaaattttatgatgcgcaaccgtgttcggataaagcgtataaaatagaagaattattttattcgtatgcgacgcatcatgataaatttacggatggtgtatgtttattttggaattgtaatgtagatcgttatccggcgaatgcgatagtatgtcgttttgatacgcgtgtattatcgaatttaaatttaccgggttgtgatggtggttcgttatatgtaaataaacatgcgtttcatacgccggcgtttgataaatcggcgtttacgaatttaaaacaattaccgtttttttattattcggattcgccgtgtgaatcgcatggtaaacaagtagtatcggatatagattatgtaccgttaaaatcggcgacgtgtataacgcgttgtaatttaggtggtgcggtatgtcgtcatcatgcgaatgaatatcgtcaatatttagatgcgtataatatgatgatatcggcgggtttttcgttatggatatataaacaatttgatacgtataatttatggaatacgtttacgcgtttacaatcgttagaaaatgtagcgtataatgtagtaaataaaggtcattttgatggtcatgcgggtgaagcgccggtatcgataataaataatgcggtatatacgaaagtagatggtatagatgtagaaatatttgaaaataaaacgacgttaccggtaaatgtagcgtttgaattatgggcgaaacgtaatataaaaccggtaccggaaataaaaatattaaataatttaggtgtagatatagcggcgaatacggtaatatgggattataaacgtgaagcgccggcgcatgtatcgacgataggtgtatgtacgatgacggatatagcgaaaaaaccgacggaatcggcgtgttcgtcgttaacggtattatttgatggtcgtgtagaaggtcaagtagatttatttcgtaatgcgcgtaatggtgtattaataacggaaggttcggtaaaaggtttaacgccgtcgaaaggtccggcgcaagcgtcggtaaatggtgtaacgttaataggtgaatcggtaaaaacgcaatttaattattttaaaaaagtagatggtataatacaacaattaccggaaacgtattttacgcaatcgcgtgatttagaagattttaaaccgcgttcgcaaatggaaacggattttttagaattagcgatggatgaatttatacaacgttataaattagaaggttatgcgtttgaacatatagtatatggtgatttttcgcatggtcaattaggtggtttacatttaatgataggtttagcgaaacgttcgcaagattcgccgttaaaattagaagattttataccgatggattcgacggtaaaaaattattttataacggatgcgcaaacgggttcgtcgaaatgtgtatgttcggtaatagatttattattagatgattttgtagaaataataaaatcgcaagatttatcggtaatatcgaaagtagtaaaagtaacgatagattatgcggaaatatcgtttatgttatggtgtaaagatggtcatgtagaaacgttttatccgaaattacaagcgtcgcaagcgtggcaaccgggtgtagcgatgccgaatttatataaaatgcaacgtatgttattagaaaaatgtgatttacaaaattatggtgaaaatgcggtaataccgaaaggtataatgatgaatgtagcgaaatatacgcaattatgtcaatatttaaatacgttaacgttagcggtaccgtataatatgcgtgtaatacattttggtgcgggttcggataaaggtgtagcgccgggtacggcggtattacgtcaatggttaccgacgggtacgttattagtagattcggatttaaatgattttgtatcggatgcggattcgacgttaataggtgattgtgcgacggtacatacggcgaataaatgggatttaataatatcggatatgtatgatccgcgtacgaaacatgtaacgaaagaaaatgattcgaaagaaggtttttttacgtatttatgtggttttataaaacaaaaattagcgttaggtggttcgatagcggtaaaaataacggaacattcgtggaatgcggatttatataaattaatgggtcatttttcgtggtggacggcgtttgtaacgaatgtaaatgcgtcgtcgtcggaagcgtttttaataggtgcgaattatttaggtaaaccgaaagaacaaatagatggttatacgatgcatgcgaattatatattttggcgtaatacgaatccgatacaattatcgtcgtattcgttatttgatatgtcgaaatttccgttaaaattacgtggtacggcggtaatgtcgttaaaagaaaatcaaataaatgatatgatatattcgttattagaaaaaggtcgtttaataatacgtgaaaataatcgtgtagtagtatcgtcggatatattagtaaataattaaacgaacatgtttatatttttattatttttaacgttaacgtcgggttcggatttagatcgttgtacgacgtttgatgatgtacaagcgccgaattatacgcaacatacgtcgtcgatgcgtggtgtatattatccggatgaaatatttcgttcggatacgttatatttaacgcaagatttatttttaccgttttattcgaatgtaacgggttttcatacgataaatcatacgtttggtaatccggtaataccgtttaaagatggtatatattttgcggcgacggaaaaatcgaatgtagtacgtggttgggtatttggttcgacgatgaataataaatcgcaatcggtaataataataaataattcgacgaatgtagtaatacgtgcgtgtaattttgaattatgtgataatccgttttttgcggtatcgaaaccgatgggtacgcaaacgcatacgatgatatttgataatgcgtttaattgtacgtttgaatatatatcggatgcgttttcgttagatgtatcggaaaaatcgggtaattttaaacatttacgtgaatttgtatttaaaaataaagatggttttttatatgtatataaaggttatcaaccgatagatgtagtacgtgatttaccgtcgggttttaatacgttaaaaccgatatttaaattaccgttaggtataaatataacgaattttcgtgcgatattaacggcgttttcgccggcgcaagatatatggggtacgtcggcggcggcgtattttgtaggttatttaaaaccgacgacgtttatgttaaaatatgatgaaaatggtacgataacggatgcggtagattgttcgcaaaatccgttagcggaattaaaatgttcggtaaaatcgtttgaaatagataaaggtatatatcaaacgtcgaattttcgtgtagtaccgtcgggtgatgtagtacgttttccgaatataacgaatttatgtccgtttggtgaagtatttaatgcgacgaaatttccgtcggtatatgcgtgggaacgtaaaaaaatatcgaattgtgtagcggattattcggtattatataattcgacgtttttttcgacgtttaaatgttatggtgtatcggcgacgaaattaaatgatttatgtttttcgaatgtatatgcggattcgtttgtagtaaaaggtgatgatgtacgtcaaatagcgccgggtcaaacgggtgtaatagcggattataattataaattaccggatgattttatgggttgtgtattagcgtggaatacgcgtaatatagatgcgacgtcgacgggtaattataattataaatatcgttatttacgtcatggtaaattacgtccgtttgaacgtgatatatcgaatgtaccgttttcgccggatggtaaaccgtgtacgccgccggcgttaaattgttattggccgttaaatgattatggtttttatacgacgacgggtataggttatcaaccgtatcgtgtagtagtattatcgtttgaattattaaatgcgccggcgacggtatgtggtccgaaattatcgacggatttaataaaaaatcaatgtgtaaattttaattttaatggtttaacgggtacgggtgtattaacgccgtcgtcgaaacgttttcaaccgtttcaacaatttggtcgtgatgtatcggattttacggattcggtacgtgatccgaaaacgtcggaaatattagatatatcgccgtgtgcgtttggtggtgtatcggtaataacgccgggtacgaatgcgtcgtcggaagtagcggtattatatcaagatgtaaattgtacggatgtatcgacggcgatacatgcggatcaattaacgccggcgtggcgtatatattcgacgggtaataatgtatttcaaacgcaagcgggttgtttaataggtgcggaacatgtagatacgtcgtatgaatgtgatataccgataggtgcgggtatatgtgcgtcgtatcatacggtatcgttattacgttcgacgtcgcaaaaatcgatagtagcgtatacgatgtcgttaggtgcggattcgtcgatagcgtattcgaataatacgatagcgataccgacgaatttttcgatatcgataacgacggaagtaatgccggtatcgatggcgaaaacgtcggtagattgtaatatgtatatatgtggtgattcgacggaatgtgcgaatttattattacaatatggttcgttttgtacgcaattaaatcgtgcgttatcgggtatagcggcggaacaagatcgtaatacgcgtgaagtatttgcgcaagtaaaacaaatgtataaaacgccgacgttaaaatattttggtggttttaatttttcgcaaatattaccggatccgttaaaaccgacgaaacgttcgtttatagaagatttattatttaataaagtaacgttagcggatgcgggttttatgaaacaatatggtgaatgtttaggtgatataaatgcgcgtgatttaatatgtgcgcaaaaatttaatggtttaacggtattaccgccgttattaacggatgatatgatagcggcgtatacggcggcgttagtatcgggtacggcgacggcgggttggacgtttggtgcgggtgcggcgttacaaataccgtttgcgatgcaaatggcgtatcgttttaatggtataggtgtaacgcaaaatgtattatatgaaaatcaaaaacaaatagcgaatcaatttaataaagcgatatcgcaaatacaagaatcgttaacgacgacgtcgacggcgttaggtaaattacaagatgtagtaaatcaaaatgcgcaagcgttaaatacgttagtaaaacaattatcgtcgaattttggtgcgatatcgtcggtattaaatgatatattatcgcgtttagataaagtagaagcggaagtacaaatagatcgtttaataacgggtcgtttacaatcgttacaaacgtatgtaacgcaacaattaatacgtgcggcggaaatacgtgcgtcggcgaatttagcggcgacgaaaatgtcggaatgtgtattaggtcaatcgaaacgtgtagatttttgtggtaaaggttatcatttaatgtcgtttccgcaagcggcgccgcatggtgtagtatttttacatgtaacgtatgtaccgtcgcaagaacgtaattttacgacggcgccggcgatatgtcatgaaggtaaagcgtattttccgcgtgaaggtgtatttgtatttaatggtacgtcgtggtttataacgcaacgtaattttttttcgccgcaaataataacgacggataatacgtttgtatcgggtaattgtgatgtagtaataggtataataaataatacggtatatgatccgttacaaccggaattagattcgtttaaagaagaattagataaatattttaaaaatcatacgtcgccggatgtagatttaggtgatatatcgggtataaatgcgtcggtagtaaatatacaaaaagaaatagatcgtttaaatgaagtagcgaaaaatttaaatgaatcgttaatagatttacaagaattaggtaaatatgaacaatatataaaatggccgtggtatgtatggttaggttttatagcgggtttaatagcgatagtaatggtaacgatattattatgttgtatgacgtcgtgttgttcgtgtttaaaaggtgcgtgttcgtgtggttcgtgttgtaaatttgatgaagatgattcggaaccggtattaaaaggtgtaaaattacattatacgtaaacgaacttatggatttgtttatgagattttttactcttagatcaattactgcacagccagtaaaaattgacaatgcttctcctgcaagtactgttcatgctacagcaacgataccgctacaagcctcactccctttcggatggcttgttattggcgttgcatttcttgctgtttttcagagcgctaccaaaataattgcgctcaataaaagatggcagctagccctttataagggcttccagttcatttgcaatttactgctgctatttgttaccatctattcacatcttttgcttgtcgctgcaggtatggaggcgcaatttttgtacctctatgccttgatatattttctacaatgcatcaacgcatgtagaattattatgagatgttggctttgttggaagtgcaaatccaagaacccattactttatgatgccaactactttgtttgctggcacacacataactatgactactgtataccatataacagtgtcacagatacaattgtcgttactgaaggtgacggcatttcaacaccaaaactcaaagaagactaccaaattggtggttattctgaggataggcactcaggtgttaaagactatgtcgttgtacatggctatttcaccgaagtttactaccagcttgagtctacacaaattactacagacactggtattgaaaatgctacattcttcatctttaacaagcttgttaaagacccaccgaatgtgcaaatacacacaatcgacggctcttcaggagttgctaatccagcaatggatccaatttatgatgagccgacgacgactactagcgtgcctttgtaagcacaagaaagtgagtacgaacttatgtactcattcgtttcggaagaaacaggtacgttaatagttaatagcgtacttctttttcttgctttcgtggtattcttgctagtcacactagccatccttactgcgcttcgattgtgtgcgtactgctgcaatattgttaacgtgagtttagtaaaaccaacggtttacgtctactcgcgtgttaaaaatctgaactcttctgaaggagttcctgatcttctggtctaaacgaactaactattattattattctgtttggaactttaacattgcttatcatggcggataatggtacgataacggtagaagaattaaaacaattattagaacaatggaatttagtaataggttttttatttttagcgtggataatgttattacaatttgcgtattcgaatcgtaatcgttttttatatataataaaattagtatttttatggttattatggccggtaacgttagcgtgttttgtattagcggcggtatatcgtataaattgggtaacgggtggtatagcgatagcgatggcgtgtatagtaggtttaatgtggttatcgtattttgtagcgtcgtttcgtttatttgcgcgtacgcgttcgatgtggtcgtttaatccggaaacgaatatattattaaatgtaccgttacgtggtacgatagtaacgcgtccgttaatggaatcggaattagtaataggtgcggtaataatacgtggtcatttacgtatggcgggtcattcgttaggtcgttgtgatataaaagatttaccgaaagaaataacggtagcgacgtcgcgtacgttatcgtattataaattaggtgcgtcgcaacgtgtaggtacggattcgggttttgcggcgtataatcgttatcgtataggtaattataaattaaatacggatcatgcgggttcgaatgataatatagcgttattagtacaataagtgacaacagatgtttcatcttgttgacttccaggttacaatagcagagatattgattatcattatgaggactttcaggattgctatttggaatcttgacgttataataagttcaatagtgagacaattatttaagcctctaactaagaagaattattcggagttagatgatgaagaacctatggagttagattatccataaaacgaacatgaaaattattctcttcctgacattgattgtatttacatcttgcgagctatatcactatcaggagtgtgttagaggtacgactgtactactaaaagaaccttgcccatcaggaacatacgagggcaattcaccatttcaccctcttgctgacaataaatttgcactaacttgcactagcacacactttgcttttgcttgtgctgacggtactcgacatacctatcagctgcgtgcaagatcagtttcaccaaaacttttcatcagacaagaggaggttcaacaagagctctactcgccactttttctcattgttgctgctctagtatttttaatactttgcttcaccattaagagaaagacagaatgaatgagctcactttaattgacttctatttgtgctttttagcctttctgctattccttgttttaataatgcttattatattttggttttcactcgaaatccaggatctagaagaaccttgtaccaaagtctaaacgaacatgaaacttctcattgttttgacttgtatttctctatgcagttgcatatgcactgtagtacagcgctgtgcatctaataaacctcatgtgcttgaagatccttgtaaggtacaacactaggggtaatacttatagcactgcttggctttgtgctctaggaaaggttttaccttttcatagatggcacactatggttcaaacatgcacacctaatgttactatcaactgtcaagatccagctggtggtgcgcttatagctaggtgttggtaccttcatgaaggtcaccaaactgctgcatttagagacgtacttgttgttttaaataaacgaacaaattaaaatgtctgataatggaccccaatcaaaccaacgtagtgccccccgcattacatttggtggacccacagattcaactgacaataaccagaatggaggacgcaatggggcaaggccaaaacagcgccgaccccaaggtttacccaataatactgcgtcttggttcacagctctcactcagcatggcaaggaggaacttagattccctcgaggccagggcgttccaatcaacaccaatagtggtccagatgaccaaattggctactaccgaagagctacccgacgagttcgtggtggtgacggcaaaatgaaagagctcagccccagatggtacttctattacctaggaactggcccagaagcttcacttccctacggcgctaacaaagaaggcatcgtatgggttgcaactgagggagccttgaatacacccaaagaccacattggcacccgcaatcctaataacaatgctgccaccgtgctacaacttcctcaaggaacaacattgccaaaaggcttctacgcagagggaagcagaggcggcagtcaagcctcttctcgctcctcatcacgtagtcgcggtaattcaagaaattcaactcctggcagcagtaggggaaattctcctgctcgaatggctagcggaggtggtgaaactgccctcgcgctattgctgctagacagattgaaccagcttgagagcaaagtttctggtaaaggccaacaacaacaaggccaaactgtcactaagaaatctgctgctgaggcatctaaaaagcctcgccaaaaacgtactgccacaaaacagtacaacgtcactcaagcatttgggagacgtggtccagaacaaacccaaggaaatttcggggaccaagacctaatcagacaaggaactgattacaaacattggccgcaaattgcacaatttgctccaagtgcctctgcattctttggaatgtcacgcattggcatggaagtcacaccttcgggaacatggctgacttatcatggagccattaaattggatgacaaagatccacaattcaaagacaacgtcatactgctgaacaagcacattgacgcatacaaaacattcccaccaacagagcctaaaaaggacaaaaagaaaaagactgatgaagctcagcctttgccgcagagacaaaagaagcagcccactgtgactcttcttcctgcggctgacatggatgatttctccagacaacttcaaaattccatgagtggagcttctgctgattcaactcaggcataaacactcatgatgaccacacaaggcagatgggctatgtaaacgttttcgcaattccgtttacgatacatagtctactcttgtgcagaatgaattctcgtaactaaacagcacaagtaggtttagttaactttaatctcacatagcaatctttaatcaatgtgtaacattagggaggacttgaaagagccaccacattttcatcgaggccacgcggagtacgatcgagggtacagtgaataatgctagggagagctgcctatatggaagagccctaatgtgtaaaattaattttagtagtgctatccccatgtgattttaatagcttcttaggagaatgacaaaaaaaaaaaaaaaaaaaaaaaa

SEQ ID NO: 42 - DNA, 29751 bp, Unknown
  synthetic
atattaggtttttacctacccaggaaaagccaaccaacctcgatctcttgtagatctgttctctaaacgaactttaaaatctgtgtagctgtcgctcggctgcatgcctagtgcacctacgcagtataaacaataataaattttactgtcgttgacaagaaacgagtaactcgtccctcttctgcagactgcttacggtttcgtccgtgttgcagtcgatcatcagcatacctaggtttcgtccgggtgtgaccgaaaggtaagatggagtcattagtgttaggcgttaacgaaaaaactcacgttcaattgtcactaccagtgttacaggttagagacgtactcgttagggggttcggtgattcagtcgaagaggcactatccgaagctagagagcatcttaaaaacggtacatgcggattagtcgaactcgaaaaaggcgtactaccacaattggagcaaccatacgtttttattaaacggtctgacgcacttagtactaatcacggtcataaggtagtcgagttagtcgccgaaatggacggtattcaatacggtaggtcaggtattacactcggagtgttagtgccacacgtaggcgaaacacctatcgcttatcgtaacgttctattgcgtaaaaacggtaataagggcgcaggcggacattcatacggtatcgatcttaagtcatacgatttaggcgacgaactcggtacggatccaatcgaagattacgaacagaattggaatactaaacacggatctggcgcattacgcgaacttacacgcgaacttaacggaggcgcagtgactagatacgtcgataataatttttgcggtccagacggatatccactcgattgtattaaggattttctcgctagggcaggtaagtctatgtgtacacttagcgaacaactcgattatatcgaatctaaaagaggcgtatattgttgtcgcgatcacgaacacgaaatcgcttggtttactgagcgatctgataagtcatacgaacatcagactccattcgaaattaagtctgctaaaaaattcgatacttttaaaggcgaatgtcctaaattcgtttttccacttaactctaaggttaaggttattcaacctagagtcgaaaaaaaaaaaactgagggttttatgggtaggattaggtcagtgtatccagtcgctagtccacaagagtgtaataatatgcatctatctacacttatgaaatgtaatcattgtgacgaagtgtcatggcaaacatgcgatttccttaaggctacatgcgaacattgcggtaccgaaaatctcgtaatcgagggacctactacatgcggatacttacctactaacgcagtcgttaaaatgccatgtccagcttgtcaggatccagagataggtccagagcatagcgttgccgattatcataatcattctaatatcgaaactagattgcgtaaaggcggtaggacacgttgtttcggcggatgcgtattcgcatacgtaggttgttataataagagagcgtattgggtgcctagagctagtgccgatatcggtagcggacataccggtattacaggcgataacgttgagacacttaacgaggatctgttagagattctatcacgcgaacgcgttaatattaacatagtcggcgattttcatcttaacgaagaggtcgctattatactcgctagtttttccgctagtacatccgcttttatcgatactattaagtctcttgactataagtcttttaaaactatcgttgagtcatgcggtaattataaggttactaagggtaagccagtgaaaggcgcatggaatatcggtcagcaacgttcagtgcttacaccactatgcggttttcctagtcaagccgcaggcgtaattagatctattttcgcacgtacacttgacgctgctaatcattctattcccgatctgcaacgtgctgccgttacgatactcgacggtattagcgaacagtcacttagactcgttgacgctatggtgtatacatccgatctgttaacgaatagtgtgattattatggcttacgttacaggcggattagtgcaacagactagtcaatggttgtctaatctgttaggtactacagtcgaaaaattgcgacctattttcgaatggattgaggctaaattgtctgccggagtcgaattccttaaagacgcttgggagatacttaaatttctgattaccggcgtattcgatatcgttaagggtcagattcaggtcgctagcgataatattaaggattgcgttaagtgttttatcgacgtagtgaataaggcactcgaaatgtgtatcgatcaggttacaattgccggagctaagcttagatcacttaacttaggcgaagtgtttatcgctcaatctaagggattgtatcgtcaatgtatacgcggtaaggagcaattgcaattgcttatgccacttaaggctcctaaagaggttacattccttgagggcgattcacacgatacagtgcttactagcgaagaggttgtgcttaaaaacggcgaactcgaagcacttgagacaccagtcgattcttttactaacggcgcaatcgtaggtacacccgtatgcgttaacggtcttatgttgcttgagattaaggataaagagcaatattgcgcacttagtccaggtctgttagcgactaataacgtttttagacttaagggaggcgcacctattaaaggcgttacattcggtgaggatacagtttgggaagtgcaagggtataaaaacgttaggattacattcgaactcgacgaacgtgtcgataaggtacttaacgaaaagtgtagcgtatatacagtcgaatccggtactgaggttactgagttcgcatgcgtagtcgctgaggcagtcgttaagacattgcaaccggttagcgatctgttaactaatatgggtatcgatcttgacgaatggtcagtcgctactttttatctattcgatgacgctggcgaagagaatttttcgtcacgtatgtattgttctttttaccctcctgacgaagaggaagaggacgacgctgaatgcgaagaggaagagatagacgaaacatgcgaacacgaatacggtacggaagacgattatcagggattgccactcgaattcggcgctagcgctgagactgttagagtcgaagaggaagaggaagaggattggttagacgatactactgagcaatccgaaatcgaacccgaacccgaacctacacctgaggaacccgttaatcaatttacagggtatcttaagcttaccgataacgttgcgattaaatgcgttgatatcgttaaagaggctcaatccgctaatcctatggtaatcgttaacgctgctaatatacatcttaagcatggcggaggcgttgcaggcgcacttaataaggctactaacggcgctatgcaaaaagagtctgacgattatattaagcttaacggtccacttaccgtaggcggatcatgtctattgtcaggtcataatctcgctaaaaaatgtcttcacgtagtcggacctaatcttaacgctggcgaagacatacaattgcttaaagccgcatacgagaattttaattcgcaagacatattgctcgcaccactgttatccgcaggtattttcggagctaaaccattgcaatcattgcaggtatgcgttcagacagtgcgtacacaggtatatatcgcagttaacgataaggcactatacgaacaggtcgttatggattatctcgataatcttaagcctagagtcgaagctcctaaacaggaagagccacctaatactgaggattctaagactgaggaaaaatccgttgtgcaaaaaccagtcgacgttaagcctaaaattaaggcatgtattgacgaagtgactactacacttgaggagactaagtttcttactaataagttactgttattcgctgatattaacggtaagttgtatcacgattcacagaatatgcttagaggcgaagatatgtcttttctcgaaaaagacgctccatatatggtaggcgacgttattacatctggcgatattacatgcgtagtgatacctagtaaaaaagccggaggtactaccgaaatgctatcacgtgcacttaaaaaagtgccagtcgacgaatacattactacttatcccggtcagggatgcgcaggttatacactcgaagaggctaaaaccgcacttaaaaaatgtaaatccgctttttacgttctgccatctgaggcacctaacgctaaagaggagatactcggtacagtgtcatggaatttacgcgaaatgcttgcgcatgccgaagagacacgtaagcttatgcctatttgtatggacgttagggctattatggctactattcaacgtaagtataagggtattaagattcaagagggtatagtcgattacggagtgagattttttttttatacatctaaagagccagtcgctagtattattactaagcttaactcacttaacgaaccattagtgactatgcctatcggatacgttacacacggttttaatctcgaagaggccgctagatgtatgcgatcacttaaggcaccagccgtagtgtcagtgtcatcacctgacgccgttactacttataacggataccttacatctagttctaagactagtgaggaacatttcgttgagacagtgtcacttgccggttcatatcgcgattggtcttattcaggtcaacgtactgagttaggcgttgagtttcttaaacgcggagataagatagtgtatcatacacttgagtcaccagtcgagtttcacttagacggcgaagtgcttagtctcgataagcttaagtctctattgtcacttagagaggttaagactattaaagtgtttactacagtcgataatactaatctgcatacacagttagtcgatatgtctatgacatacggtcagcaattcggacctacttatcttgacggtgcagacgttactaagattaagcctcacgttaatcacgaaggtaagacttttttcgtattgccatctgacgatacacttagatccgaagcattcgaatactatcatacacttgacgaatcttttctcggtaggtatatgtcagcacttaaccatacaaaaaaatggaaattcccacaggtaggcggacttacatctattaaatgggccgataataattgttatctgtcatcagtgttactcgcattgcagcaactcgaagtgaaatttaacgctcctgcattgcaagaggcatactatagggctagagccggtgacgctgctaatttttgcgcacttatactcgcatactctaataaaaccgtaggcgaactcggtgacgttagagagactatgacacatctattgcaacacgctaatctcgaatccgctaaaagagtgcttaacgtagtgtgtaaacattgcggtcagaaaactactacacttaccggagtcgaagccgttatgtatatgggtacactatcatacgataatcttaaaaccggagtgtcaattccatgcgtatgcggtagggacgctacacaatacttagtgcaacaagagtctagtttcgttatgatgtcagctccacctgccgaatacaaattgcaacagggtacattcttatgcgctaacgagtataccggtaattatcaatgcggtcattatacacatattaccgctaaagagacattgtatcgtatagacggtgcacatcttactaaaatgtctgagtataagggtccagttactgacgttttttacaaagagactagttatactactactattaaaccggttagttataagttagacggagtgacttataccgaaatcgaacctaagttagacggatactataaaaaagataacgcttattataccgaacagccaatcgatttagtgcctacacaaccattgcctaacgctagtttcgataattttaagcttacatgttctaatactaaattcgcagacgatcttaatcagatgaccggttttactaagcctgctagtagagagttatccgttactttttttcccgatcttaacggtgacgtagtcgcaatcgattatcgtcattactctgctagttttaaaaaaggcgctaagctattgcataaacctatcgtttggcatattaatcaggctactactaagactacttttaaacctaatacttggtgtcttagatgtctttggtctactaagccagtcgatacatctaattcattcgaagtgcttgcagtcgaggatacacagggtatggataatctcgcatgcgaatcgcaacaacctacatccgaagaggtagtcgagaatcctacaattcagaaagaggtaatcgaatgcgacgttaagactaccgaagtggtaggtaacgttatacttaaaccgtctgacgaaggcgttaaggttacgcaagagttaggccatgaggatcttatggccgcatacgttgagaatacatctattactattaaaaaacctaacgaactatcactcgcattaggtcttaagactatcgctacacacggtatagccgctattaattcggttccatggtctaagatactcgcatacgttaagccttttctcggtcaagccgctattactacatctaattgcgctaaacgacttgcgcaacgcgtttttaataattatatgccatacgtttttacattgctttttcaattgtgtacttttactaagtctactaactcacgtatacgcgctagtctacctactactatcgctaaaaattccgttaaatccgttgcgaaattgtgtcttgacgcaggtattaattacgttaagtcacctaaattttctaaattgtttacaatcgctatgtggttactgttattgtctatttgtctcggttcattgatttgcgttaccgctgcattcggagtgttactatctaatttcggcgcacctagttattgtaacggagtgagagagttgtatctgaatagttctaacgttactactatggatttttgcgaaggatcttttccatgttcaatttgtctatctggtctcgattcactcgattcatatcccgctctcgaaactattcaggttacgattagttcttataaactcgatcttactatactcggtctagccgctgaatgggtgttagcgtatatgctttttactaagtttttttacttactcggtctatccgctattatgcaagtgtttttcggatatttcgctagtcattttatttctaatagttggcttatgtggtttattatttcgattgtgcaaatggcaccagttagcgctatggtacgtatgtatatttttttcgctagtttttactatatttggaaatcatacgttcatattatggacggatgtacatctagtacatgtatgatgtgttataaacgtaatcgcgctactagagtcgagtgtactactatcgttaacggtatgaaacgatctttttacgtttacgctaacggaggtagggggttttgtaagactcataattggaattgtcttaattgcgatactttttgtaccggtagtacttttatttctgacgaagtcgcacgcgatctatcattgcaatttaaacgtccaattaaccctaccgatcaatctagttatatagtcgatagcgttgcggttaaaaacggcgcattgcatctatatttcgataaagccggtcagaaaacatacgaacgtcatccactatcacatttcgttaacttagacaatcttagggctaataatactaagggtagtctgccaattaacgtaatcgtattcgacggtaagtctaaatgcgacgaatccgctagtaagtctgctagtgtgtattactctcagcttatgtgtcaacctatactgttactcgatcaggcattagtgtcagacgtaggcgatagtactgaggttagcgttaaaatgttcgacgcttacgtcgatacttttagcgctacattctcagtgcctatggagaaacttaaggcattagtcgctaccgctcattctgagttagcgaaaggcgttgcgttagacggagtgctatctacattcgtatctgccgctagacagggcgtagtcgatactgacgtcgatactaaagacgtaatcgaatgtcttaagctatcacatcattccgatcttgaggttacaggcgattcatgtaataattttatgcttacatataataaggtcgagaatatgacacctagagacttaggcgcatgtatcgattgtaacgctagacatattaacgctcaggttgcgaaatcacataacgtatcattgatttggaacgttaaagactatatgtcactatctgagcaattgcgtaaacagatacgatccgctgctaaaaaaaataatataccgtttagacttacatgcgctactactagacaggtcgttaacgttattactactaagattagtcttaagggaggtaagatcgttagtacatgttttaagcttatgcttaaggctacactgttatgcgtactcgctgcactcgtatgttatatcgttatgccagtgcatacactatctattcacgacggatatactaacgaaattatcggatataaggctattcaagacggagtgacacgcgatattattagtactgacgattgtttcgctaataaacacgctggattcgacgcttggttttcgcaacgcggagggtcatataaaaacgataagtcatgtccagtcgttgccgctattattacacgcgaaatcggattcatagtgccagggttacccggtacagtgttgcgtgctattaacggcgattttttgcattttctgccacgcgtttttagcgcagtcggtaatatttgttatacacctagtaagttaatcgaatactctgatttcgctactagcgcatgcgtacttgccgctgagtgtactatttttaaagacgctatgggtaagccagtgccatattgttacgatactaatctgttagagggatctatttcatactctgagttgcgacctgatactaggtacgtacttatggacggatctattattcaattccctaatacttatcttgagggatccgttagagtcgttactacattcgacgctgagtattgtagacacggtacatgcgaacgatctgaggtcggtatttgtctatctacatctggtagatgggtacttaataacgaacattatcgcgcactatctggcgttttttgcggcgtagacgctatgaatcttatcgctaatatttttacaccattagtgcaaccagtcggcgcacttgacgtatccgctagcgtagtcgcaggcggtattatcgctatactcgttacatgcgctgcatactattttatgaaatttcgtagggtattcggtgagtataatcacgtagtcgctgctaacgctctattattccttatgtcttttacgatactgtgtctcgtacctgcatactcttttctgccaggcgtatactctgtgttttatctgtatcttacattttactttactaacgacgtttcgtttctcgcacatctgcaatggttcgctatgttttcacctatagtgccattttggattaccgctatttacgttttttgtatttcgcttaagcattgtcattggttttttaataattatttgcgtaaacgcgttatgtttaacggagtgactttttcgacattcgaagaggccgcactttgtacttttctgcttaataaagagatgtatcttaagttacggtctgagacactgttaccacttacacaatacaataggtatctcgcactatataataagtataagtatttttcaggcgcactcgatactacatcttatcgcgaagccgcatgttgtcatctcgctaaagcgcttaacgatttttctaactctggcgcagacgtactgtatcaacctccacaaacatctattacgtctgccgtactgcaatccggttttcgtaaaatggcttttccatcaggtaaggtcgagggatgtatggtgcaagttacatgcggtactactacacttaacggtctatggttagacgatacggtttattgtcctagacacgttatttgtactgccgaagatatgcttaaccctaattacgaagacttactgatacgtaaatctaatcactcttttttagtgcaagccggtaacgttcaattgcgcgttatcggtcattctatgcaaaattgtctgttacgtcttaaagtcgatacatctaatcctaaaactcctaagtataaattcgttaggattcaacccggtcagacattctcagtactcgcatgttataacggttcacctagcggagtgtatcaatgcgctatgcgacctaatcatacaattaagggatcttttcttaacggttcatgcggatcagtcggttttaatatcgattacgattgcgttagtttttgttatatgcatcatatggagttacctacaggcgtacacgctggtactgatcttgagggtaagttttacggtccattcgttgatcgtcaaaccgctcaagccgcaggtaccgatactactattacacttaacgtactcgcatggttatacgctgccgttattaacggcgatagatggtttcttaatagatttactactacacttaacgattttaacttagtcgctatgaaatataattacgaaccacttacacaggatcacgtcgatatactcggtccacttagtgcgcaaaccggtatagccgtactcgatatgtgcgctgcacttaaagagttactgcaaaacggtatgaacggtaggactatactcggtagtactatactcgaagacgaatttacaccattcgacgtcgttagacagtgttcaggcgttacatttcagggtaagtttaaaaaaatcgttaagggtacacatcattggatgttgcttacattccttactagtctattgatactcgtacaatctacacaatggtcattgttttttttcgtatacgaaaacgcttttttgccttttacactcggtattatggctatagccgcatgcgctatgttgttagtgaaacataaacacgcattcttatgtctattcctattgcctagtctcgctacagtcgcatactttaatatggtgtatatgcctgctagttgggttatgcgtattatgacttggcttgagttagccgatacatctctatctggttatagacttaaggattgcgttatgtacgctagtgcattagtgttactgatacttatgactgcacgtacagtttacgacgacgctgctagacgcgtttggacacttatgaacgttattacacttgtgtataaagtgtattacggtaacgctctcgatcaggctattagtatgtgggcattagtgatatccgttacgtctaattactctggagtcgttacgactattatgtttctcgctagggctatcgtattcgtatgcgttgagtattatccactattgtttattaccggtaatacattgcaatgtattatgttagtgtattgttttttagggtattgttgttgttgttatttcggattgttttgtctacttaataggtattttagacttacattaggcgtatacgattatctcgttagtacgcaagagtttagatatatgaattcacagggactgttaccacctaaatcttcaatcgacgcttttaagcttaacattaagttactcggtataggcggtaagccttgtattaaggttgcgacagtgcaatctaaaatgtctgacgttaagtgtactagtgtcgtactgttatcagtgttacagcaattgcgagtcgaatctagttctaaattgtgggctcaatgcgttcaattgcataacgatatcttactcgctaaggatactactgaggcattcgaaaaaatggttagtctgttaagcgtactgttatctatgcaaggcgcagtcgatattaatcgattatgcgaagagatgttagacaatagggctacattgcaggctattgcgtcagagttttctagtctgccatcatacgctgcatacgctaccgctcaagaggcatacgaacaggcagtcgctaacggcgattctgaggtagtgcttaaaaaacttaaaaaatcacttaacgttgcgaaatctgagttcgatagagacgctgctatgcaacgtaaactcgaaaaaatggccgatcaggctatgacacaaatgtataaacaggctagatctgaggataagcgtgctaaggttacatccgctatgcaaactatgttgtttactatgttgcgtaaactcgataacgacgcacttaacaatattattaataacgctagagacggatgcgtaccacttaatattataccgcttactactgccgctaagcttatggtagtcgttcccgattacggtacttataagaatacatgcgacggtaatacttttacatacgctagtgcattgtgggagattcaacaggtcgttgacgctgattctaaaatcgttcaattgtctgagattaatatggataactcacctaatctcgcatggccattaatcgttacagcgttacgcgctaactctgccgttaagttacagaataacgaattgtcaccagtcgcattgcgtcaaatgtcatgcgctgccggtactacacaaaccgcttgtactgacgataacgctctcgcatactataataactctaaaggcggtagattcgtactcgcactattatccgatcatcaggatcttaaatgggctagattccctaagtctgacggtacaggtacaatttataccgaactcgaaccaccatgtagattcgttaccgatacacctaagggacctaaggttaagtatctatactttattaagggactgaataatctgaataggggtatggtgttagggtcactcgcagctaccgttagattgcaagccggtaacgctactgaggttcccgctaactcaaccgtacttagtttttgcgcattcgcagtcgatccagctaaggcttataaggattacttagctagcggaggtcaacctattactaattgcgttaaaatgctatgtacacataccggtacaggtcaggctattacggttacacctgaggctaatatggatcaggagtcattcggaggcgcatcatgttgtctatattgtagatgtcatatcgatcatcctaatcctaagggtttttgcgatcttaagggtaagtacgttcagattcctactacatgcgctaacgatccagtcggttttacattgcgtaataccgtttgtacagtatgcggtatgtggaaaggttacggatgttcatgcgatcagttacgcgaaccacttatgcaatccgctgacgctagtacattccttaatgggtttgcggtgtaagtgccgctagattgactccatgcggtacaggtactagtactgacgtagtgtatcgcgcattcgatatttataacgaaaaggttgccggattcgctaaattccttaagactaattgttgtagatttcaggaaaaagacgaagagggtaatctgttagactcatatttcgtagtgaaacgtcatactatgtctaattatcaacacgaagagactatttataatctcgttaaggattgtccagccgttgcggtacacgatttttttaaatttagagtcgacggtgatatggtgccacatatttctagacagagattgactaagtatactatggccgatctagtttacgctcttagacatttcgacgaaggtaattgcgatacacttaaagagatactcgttacatataattgttgcgacgacgattactttaataaaaaagattggtacgatttcgttgagaatcccgatatacttagggtttacgctaacttaggcgaacgcgttagacagtcattgcttaagacagtgcaattttgcgacgctatgcgtgacgcaggtatagtcggcgtacttacactcgataatcaggatcttaacggtaattggtacgatttcggcgatttcgttcaggtcgcaccaggttgcggagtgcctatagtcgattcatactattcattgcttatgcctatacttacacttacacgtgcacttgccgctgagtcacatatggacgctgatctcgctaaaccattgattaaatgggatctacttaaatacgattttactgaggaacgattgtgtctattcgataggtattttaagtattgggatcagacttatcatcctaattgtattaattgtcttgacgatagatgtatactgcattgcgctaattttaacgtattgttctcaaccgtattcccacctacatcattcggtccactcgtacgtaagattttcgttgacggcgtaccattcgtagtgtcaaccggttatcattttagagagttaggcgtagtgcataatcaggacgttaatctgcattctagtagactatcttttaaagagttgttagtgtacgctgccgatccagctatgcatgccgctagcggtaatctgttactcgataagcgtactacatgttttagcgttgccgcacttactaataacgttgcgtttcagactgttaaacccggtaattttaataaggatttttacgatttcgcagtgagtaagggtttttttaaagagggatctagcgttgagcttaagcatttttttttcgctcaagacggtaacgctgctattagcgattacgattactatagatataatctgccaactatgtgcgatatacgtcaattgttgttcgtcgttgaggtagtcgataagtatttcgattgttacgacggaggttgtattaacgctaatcaggtaatcgttaataatctcgataagtctgccggattcccattcaataaatggggtaaggctagattgtattacgattctatgtcatacgaggatcaggacgctctattcgcatatactaagcgtaacgttataccgacaattacgcaaatgaatcttaaatacgctattagcgctaaaaatcgtgcacgtacagtcgcaggcgtatcaatttgtagtactatgactaatcgtcaatttcaccaaaaattgcttaagtctattgccgctactagaggcgctacagtcgttatcggtacatctaaattttacggaggttggcataatatgcttaagacagtgtattctgacgttgagactccacatcttatgggttgggattaccctaaatgcgatagggctatgcctaatatgttgcgtattatggctagtctcgtactcgcacgtaaacataatacatgttgtaatctatcacatagattctatagactcgctaacgaatgcgctcaagtgcttagcgaaatggttatgtgtggcggatcactttacgttaagcctggcggtacatctagcggagacgctactaccgcttacgctaattccgtttttaatatttgtcaagccgttaccgctaacgttaacgctctattgtctactgacggtaataagattgccgataaatacgtacgtaatctgcaacatagattgtacgaatgtctgtatcgtaatcgcgatgtcgatcacgaattcgttgacgaattttacgcttacttacgtaaacatttttctatgatgattctatctgacgacgcagtcgtttgttataactctaattacgctgcacaggggttagtcgctagtattaagaattttaaagccgtactgtattatcagaataacgtttttatgtctgaggctaagtgttggaccgaaaccgatctgactaagggtccacacgaattttgttcacagcatactatgctcgttaaacagggtgacgattacgtttatctaccatatcccgatccgtcacgtatattaggcgcaggttgtttcgttgacgatatcgttaagactgacggtacacttatgattgagagattcgttagtctcgcaatcgacgcttatccattgactaagcatcctaatcaggaatacgctgacgtttttcacttatacttacagtatatacgtaaattgcacgacgaacttacagggcatatgcttgatatgtattcggttatgcttactaacgataatactagtaggtattgggaacctgagttttacgaagctatgtatacaccacataccgtactgcaagccgtaggcgcatgcgtactatgtaattcacagactagtcttagatgtggcgcatgtatacgtagaccattcttatgttgtaagtgttgttacgatcacgttattagtacatcacataagttagtgttatccgttaacccatacgtttgtaacgctccaggttgcgacgttactgacgttacgcaattgtacttaggcggtatgtcatactattgtaaatcacataaacctcctattagttttccgttatgcgctaacggtcaggtattcggtctatataagaatacatgcgtagggtctgataacgttaccgattttaacgctatcgctacatgcgattggactaacgctggcgattatatactcgctaatacatgtactgagcgacttaagttattcgcagccgaaacacttaaggctaccgaagagacttttaaattgtcatacggtatcgctaccgtacgcgaagtgcttagcgatagagagttgcatctatcatgggaggtcggtaagcctagaccaccacttaatcgtaattacgtttttacagggtatcgggttactaagaattcgaaagtgcaaattggcgaatatacattcgaaaaaggcgattacggtgacgccgtagtgtatagaggtactactacttataagcttaacgtaggcgattatttcgtacttacatcacataccgttatgccattatccgctcctacattagtgccacaagagcattacgttaggattaccggattgtatcctacacttaatatttctgacgaattttcatctaacgttgcgaattatcagaaagtgggtatgcaaaaatactctacattgcagggacctcccggtaccggtaagtctcatttcgcaatcggactcgcattgtattatcctagtgctaggattgtgtataccgcttgttcacacgctgcagtcgacgctctatgcgaaaaagctcttaagtatctaccaatcgataagtgttcacgtattatacccgctagggctagagtcgaatgtttcgataagtttaaagtgaattcgacactcgaacaatacgttttttgtacggttaacgctctaccagagactactgccgatatcgtagtgttcgacgaaatttctatggctactaattacgatctatcagtcgttaacgctagacttagggctaagcattacgtttatataggcgatccagcgcaattgcctgcaccacgtacattgttgactaagggtacactcgaacctgagtattttaattcagtgtgtagacttatgaaaactatcggacctgatatgtttctcggtacatgtcgtagatgtcctgccgaaatagtcgatacagttagcgcactcgtatacgataataagcttaaggcacataaggataagtctgcgcaatgttttaaaatgttttacaaaggcgtaattacacacgacgttagttccgctattaatagaccacagataggcgtagtgagagagtttcttacacgtaatcccgcttggcgtaaagccgtttttattagtccatataactctcaaaacgcagtcgctagtaagatactcggattgcctacacagacagtcgattctagtcagggtagcgaatacgattacgttatttttacgcaaactaccgaaaccgctcattcatgtaacgttaatagatttaacgttgcgattactagggctaaaatcggtattctatgtattatgtctgatcgcgatctatacgataagttgcaatttacatcacttgagatacctagacgtaacgttgcgacattgcaagccgaaaacgttaccggattgtttaaggattgttctaagattattaccggattgcatcctacacaggcacctacacatctatcagtcgatattaagtttaagactgagggtctatgcgttgacatacccggtatacctaaggatatgacttatcgtagattgattagtatgatgggttttaaaatgaattatcaggttaacggttatcctaatatgtttattacacgcgaagaggctattagacacgttagggcttggatagggttcgacgttgagggatgtcacgctacacgtgacgcagtcggtactaatctgccattgcaattagggttttcgacaggcgttaatctggttgccgtacctaccggatacgtcgatactgagaataatactgagtttactagggttaacgctaaacctccacctggcgatcaatttaaacatctgattccacttatgtataagggattgccttggaacgtagtgcgtattaagattgtgcaaatgcttagcgatacacttaagggattgtctgatagggttgtgttcgtactttgggctcacggattcgaattgacatctatgaaatatttcgttaaaatcggacctgagcgtacatgttgtctatgcgataagcgtgctacatgttttagtacatctagcgatacatacgcttgttggaatcattcagtcggattcgattacgtttataatccttttatgattgacgttcagcaatgggggtttaccggtaatctgcaatctaatcacgatcagcattgtcaggtacacggtaacgctcacgttgcgtcatgcgacgctattatgactagatgtcttgccgtacacgaatgtttcgttaagagagtcgattggtcagtcgaataccctattataggcgacgaacttagggttaattccgcttgtcgtaaagtgcaacatatggtcgttaagtctgctctattagccgataagtttcccgtattgcacgatatcggtaatcctaaagcgattaaatgcgtaccacaagccgaagtcgaatggaaattttacgacgctcaaccatgttctgataaggcatacaaaatcgaagagttgttttactcatacgctacacatcacgataagtttactgacggcgtatgtctgttttggaattgtaacgttgataggtatcccgctaacgctatcgtttgtagattcgatactagggttctatctaatctgaatctgccaggttgcgatggcggatcactatacgttaataaacacgcttttcatacacctgcattcgataaatccgcttttacgaatcttaagcaattgccttttttttattactctgatagtccatgcgaatctcacggtaagcaagtcgttagcgatatcgattacgttccacttaaatccgctacatgtattacacgttgtaatctcggaggcgcagtttgtagacatcacgctaacgaatatcgtcaatacttagacgcttataatatgatgattagtgccggtttttcattgtggatttataagcaattcgatacttataatctatggaatacttttactagattgcaatctctcgaaaacgttgcgtataacgtcgttaataagggtcatttcgacggtcacgctggcgaagctcccgtatcaattattaataacgcagtgtatactaaggtcgacggtattgacgtcgagattttcgaaaataagactacattacccgttaacgttgcattcgaattgtgggctaaacgtaatattaaaccagtgccagagattaagatacttaataacttaggcgttgatatcgctgctaataccgttatttgggattataaacgcgaagctcctgcacatgtgtcaactataggcgtatgtactatgactgatatcgctaaaaaacctaccgaatccgcttgttcatcacttacagtgttattcgacggtagggttgagggtcaggtcgatctgtttcgtaacgcacgtaacggcgtactgattactgagggatcggttaagggattgacacctagtaagggacctgctcaagctagcgttaacggagtgacacttataggcgaatcagttaagactcaatttaattactttaaaaaagtcgacggtattattcaacagttaccagagacttattttacacaatcacgcgatcttgaggattttaaacctagatctcaaatggagactgattttctcgaactcgctatggacgaatttattcaacgatataagcttgagggatacgcattcgaacatatcgtttacggcgatttttcacacggtcagttaggcggattgcatcttatgatcggtctagctaaacgatcacaggatagtccacttaagcttgaggattttatacctatggattcaaccgttaagaattactttattaccgatgcgcaaaccggttcatctaaatgcgtttgtagcgtaatcgatttactgttagacgatttcgttgagattattaagtctcaggatctatcagtgattagtaaggtagtgaaagtgacaatcgattacgctgagatttcttttatgctttggtgtaaagacggtcacgttgagactttttaccctaaattgcaggctagtcaggcatggcaacctggagtcgctatgcctaatttgtataaaatgcaacgtatgttactcgaaaaatgcgatctgcaaaattacggtgagaacgcagtgatacctaagggtattatgatgaacgtcgctaagtatacacaattgtgtcaataccttaatacacttacacttgccgtaccatataatatgcgagtgatacatttcggagccggatctgataagggcgttgcgccaggtactgccgtattgcgtcaatggttgcctaccggtacactgttagtcgattccgatcttaacgatttcgtatctgacgctgatagtacacttataggcgattgcgctacagtgcataccgctaataaatgggatctgattattagcgatatgtacgatccacgtactaaacacgttacgaaagagaacgattctaaagagggtttttttacatatctatgcggttttattaaacagaaactcgcattaggcggatctattgccgttaagattactgagcatagttggaacgctgatctgtataagcttatgggtcattttagttggtggaccgcattcgttactaacgttaacgctagttctagcgaagcattcttaatcggcgctaattatctcggtaagcctaaagagcaaatcgacggatatactatgcacgctaattatattttttggcgtaatactaatcctattcaattgtctagttattcattgttcgatatgtctaaatttccacttaagttacgcggtactgccgttatgtcacttaaagagaatcagattaacgatatgatttactctttactcgaaaagggtaggttgattatacgcgaaaataatagggtagtcgttagttctgacatactcgttaataattaaacgaacatgtttatttttctgttattccttacacttacatccggttcagatctcgatagatgtactacattcgacgacgttcaggcacctaattatacacagcatacatctagtatgagaggcgtatactatcctgacgaaatttttagatccgatacattgtatcttacacaggatctattcttacctttttactctaacgttacagggtttcatacaattaatcatacattcggtaatcccgttataccgtttaaagacggtatttatttcgcagctaccgaaaaatctaacgtagtgagaggttgggtattcggtagtactatgaataataagtctcaatcagtgattattattaataattcgactaacgtagtgatacgcgcatgtaatttcgaattgtgcgataatccttttttcgcagtgtctaaacctatgggtacacagactcatactatgattttcgataacgcttttaattgtacattcgaatatatttctgacgctttttcacttgacgtatccgaaaaatctggtaattttaaacacttacgcgaattcgtttttaaaaataaagacggttttttgtacgtttataagggataccaacctatcgacgtcgttagggatctgccatcaggttttaatacacttaagcctatttttaagttaccgttaggcattaatattactaattttagagctatacttaccgcttttagtccagctcaggatatttggggtactagcgctgccgcatatttcgtcggatatcttaaacctactacttttatgcttaaatacgacgaaaacggtacaattactgacgcagtcgattgttcacagaatccattagccgaacttaagtgttcagttaagtcattcgaaatcgataagggtatttatcagactagtaattttagagtcgtacctagcggtgacgtagtgagattccctaatattacgaatctatgtccattcggcgaagtgtttaacgctactaaattccctagcgtatacgcttgggagcgtaaaaaaattagtaattgcgttgccgattactctgtgttgtataattcgactttttttagtacttttaagtgttacggagtgtcagctactaagcttaacgatctatgtttttctaacgtatacgctgattcattcgtagtgaaaggcgatgacgttaggcaaatcgctcccggtcagactggcgtaatcgctgattataattataagttacctgacgattttatgggttgcgtactcgcatggaatacacgtaatatcgacgctactagtaccggtaattataattataagtatagatatcttagacacggtaagcttagaccattcgaacgcgatatttctaacgtaccattctcacctgacggtaagccttgtacacctcctgcacttaattgttattggccacttaacgattacggtttttacactactaccggtatagggtatcaaccttatagggtagtcgttctatcattcgaattgcttaacgctccagctaccgtatgcggacctaaattgtcaaccgatctgattaagaatcaatgcgttaattttaattttaacggtcttaccggtacaggcgtacttacacctagttctaaacggtttcaaccttttcagcaattcggtagggacgttagcgattttaccgatagcgttagggatcctaaaactagtgagatactcgatattagtccatgcgcattcggaggcgtaagtgtgattactcccggtactaacgctagttctgaggttgccgtactgtatcaggacgttaattgtactgacgtatcaaccgctatacacgctgatcaattgacacctgcatggcgtatatactctaccggtaataacgtttttcagacacaagccggttgtctgataggcgcagagcatgtcgatacatcatacgaatgcgatataccgataggcgcaggtatttgcgctagttatcatacagtgtcattgcttagatctactagtcagaaatcaatcgttgcgtatactatgtcattaggcgctgatagttcaatcgcatactctaataatactatcgctatacctactaatttttcaatttcgattactactgaggttatgccagtgtctatggctaagactagtgtcgattgtaatatgtatatttgtggcgattcaaccgaatgcgctaatctgttattgcaatacggatctttttgtacgcaattgaatcgtgcactatcaggtatagccgctgaacaggatcgtaatactagagaggtattcgcacaggttaaacagatgtataagactcctacacttaagtatttcggagggtttaatttttcacagattttacccgatccacttaaacctactaaacgatcttttattgaggatctgttattcaataaggttacactcgcagacgcaggttttatgaaacaatacggcgaatgtttaggcgatattaacgctagggatctgatttgcgctcaaaaatttaacggtcttacagtgttaccaccactattgactgacgatatgatagccgcatatactgccgcattagtgtcaggtaccgctaccgcaggttggacattcggtgccggtgccgcattgcagattccattcgctatgcaaatggcttatagatttaacggtataggcgttacgcaaaacgtactttacgagaatcagaaacaaatcgctaaccaatttaataaggctattagtcagattcaagagtcacttactactactagtaccgcactcggtaagttgcaagacgtcgttaatcagaacgctcaggcacttaatacactcgttaagcaattgtctagtaatttcggagctattagttcagtgcttaacgatattctatctagactcgataaggtcgaagccgaagtgcaaatcgatagattgattaccggtaggttgcaatctctgcaaacatacgttacgcaacaattgatacgcgctgctgagattagggctagcgctaatctcgcagctactaaaatgtctgagtgcgtactcggtcaatctaaaagagtcgatttttgcggtaaggggtatcatcttatgtcttttccacaagccgcaccacacggagtggtttttttacacgttacatacgtacctagtcaggaacgtaattttactaccgctccagctatttgtcacgaaggtaaggcatactttccacgcgaaggcgtattcgtttttaacggtacatcatggtttattacgcaacgtaatttttttagtccacaaattattactactgataatacattcgttagcggtaattgcgatgtcgttatcggtattattaataataccgtttacgatccattgcaacctgagttagactcttttaaagaggaactcgataagtattttaaaaatcatacatcacctgacgttgacttaggcgatatttcaggtattaacgcttcagtcgttaatattcagaaagagattgatagacttaacgaagtcgctaaaaatcttaacgaatcacttatcgatctgcaagagttaggtaagtacgaacagtatattaaatggccttggtacgtttggttagggtttatagccggtctaatcgctatcgttatggttacgatactgttatgttgtatgacatcatgttgttcatgtcttaaaggcgcatgttcatgcggatcatgttgtaaattcgacgaagacgattctgagccagtgcttaagggagtgaaattgcattatacataaacgaacttatggatttgtttatgagattttttactcttagatcaattactgcacagccagtaaaaattgacaatgcttctcctgcaagtactgttcatgctacagcaacgataccgctacaagcctcactccctttcggatggcttgttattggcgttgcatttcttgctgtttttcagagcgctaccaaaataattgcgctcaataaaagatggcagctagccctttataagggcttccagttcatttgcaatttactgctgctatttgttaccatctattcacatcttttgcttgtcgctgcaggtatggaggcgcaatttttgtacctctatgccttgatatattttctacaatgcatcaacgcatgtagaattattatgagatgttggctttgttggaagtgcaaatccaagaacccattactttatgatgccaactactttgtttgctggcacacacataactatgactactgtataccatataacagtgtcacagatacaattgtcgttactgaaggtgacggcatttcaacaccaaaactcaaagaagactaccaaattggtggttattctgaggataggcactcaggtgttaaagactatgtcgttgtacatggctatttcaccgaagtttactaccagcttgagtctacacaaattactacagacactggtattgaaaatgctacattcttcatctttaacaagcttgttaaagacccaccgaatgtgcaaatacacacaatcgacggctcttcaggagttgctaatccagcaatggatccaatttatgatgagccgacgacgactactagcgtgcctttgtaagcacaagaaagtgagtacgaacttatgtactcattcgtttcggaagaaacaggtacgttaatagttaatagcgtacttctttttcttgctttcgtggtattcttgctagtcacactagccatccttactgcgcttcgattgtgtgcgtactgctgcaatattgttaacgtgagtttagtaaaaccaacggtttacgtctactcgcgtgttaaaaatctgaactcttctgaaggagttcctgatcttctggtctaaacgaactaactattattattattctgtttggaactttaacattgcttatcatggccgataacggtacaattaccgttgaggaacttaaacagttactcgaacaatggaatctcgtaatcggttttctgtttctcgcatggattatgctattgcaattcgcatactctaatcgtaatcggtttttgtatattattaaactcgtattcttatggttattgtggccagttacactcgcatgtttcgtactcgcagccgtttatcgtattaattgggttacaggcggtatcgctatcgctatggcttgtatagtcggacttatgtggttgtcttatttcgttgcgtcatttagattgttcgcacgtactagatctatgtggtcttttaatcccgaaactaatatactgcttaacgtaccacttagaggtacaatcgttactagaccacttatggagtctgagttagtgataggcgcagtgattattagggggcatttgcgtatggccggtcatagtctaggtagatgcgatattaaggatctacctaaagagattaccgttgcgactagtcgtacactatcttattataagttaggcgctagtcaacgtgtcggtactgatagcggattcgcagcttataataggtatcgtatcggtaattataagcttaataccgatcacgctggatctaacgataatatcgcattactcgtacagtaagtgacaacagatgtttcatcttgttgacttccaggttacaatagcagagatattgattatcattatgaggactttcaggattgctatttggaatcttgacgttataataagttcaatagtgagacaattatttaagcctctaactaagaagaattattcggagttagatgatgaagaacctatggagttagattatccataaaacgaacatgaaaattattctcttcctgacattgattgtatttacatcttgcgagctatatcactatcaggagtgtgttagaggtacgactgtactactaaaagaaccttgcccatcaggaacatacgagggcaattcaccatttcaccctcttgctgacaataaatttgcactaacttgcactagcacacactttgcttttgcttgtgctgacggtactcgacatacctatcagctgcgtgcaagatcagtttcaccaaaacttttcatcagacaagaggaggttcaacaagagctctactcgccactttttctcattgttgctgctctagtatttttaatactttgcttcaccattaagagaaagacagaatgaatgagctcactttaattgacttctatttgtgctttttagcctttctgctattccttgttttaataatgcttattatattttggttttcactcgaaatccaggatctagaagaaccttgtaccaaagtctaaacgaacatgaaacttctcattgttttgacttgtatttctctatgcagttgcatatgcactgtagtacagcgctgtgcatctaataaacctcatgtgcttgaagatccttgtaaggtacaacactaggggtaatacttatagcactgcttggctttgtgctctaggaaaggttttaccttttcatagatggcacactatggttcaaacatgcacacctaatgttactatcaactgtcaagatccagctggtggtgcgcttatagctaggtgttggtaccttcatgaaggtcaccaaactgctgcatttagagacgtacttgttgttttaaataaacgaacaaattaaaatgtctgataatggaccccaatcaaaccaacgtagtgccccccgcattacatttggtggacccacagattcaactgacaataaccagaatggaggacgcaatggggcaaggccaaaacagcgccgaccccaaggtttacccaataatactgcgtcttggttcacagctctcactcagcatggcaaggaggaacttagattccctcgaggccagggcgttccaatcaacaccaatagtggtccagatgaccaaattggctactaccgaagagctacccgacgagttcgtggtggtgacggcaaaatgaaagagctcagccccagatggtacttctattacctaggaactggcccagaagcttcacttccctacggcgctaacaaagaaggcatcgtatgggttgcaactgagggagccttgaatacacccaaagaccacattggcacccgcaatcctaataacaatgctgccaccgtgctacaacttcctcaaggaacaacattgccaaaaggcttctacgcagagggaagcagaggcggcagtcaagcctcttctcgctcctcatcacgtagtcgcggtaattcaagaaattcaactcctggcagcagtaggggaaattctcctgctcgaatggctagcggaggtggtgaaactgccctcgcgctattgctgctagacagattgaaccagcttgagagcaaagtttctggtaaaggccaacaacaacaaggccaaactgtcactaagaaatctgctgctgaggcatctaaaaagcctcgccaaaaacgtactgccacaaaacagtacaacgtcactcaagcatttgggagacgtggtccagaacaaacccaaggaaatttcggggaccaagacctaatcagacaaggaactgattacaaacattggccgcaaattgcacaatttgctccaagtgcctctgcattctttggaatgtcacgcattggcatggaagtcacaccttcgggaacatggctgacttatcatggagccattaaattggatgacaaagatccacaattcaaagacaacgtcatactgctgaacaagcacattgacgcatacaaaacattcccaccaacagagcctaaaaaggacaaaaagaaaaagactgatgaagctcagcctttgccgcagagacaaaagaagcagcccactgtgactcttcttcctgcggctgacatggatgatttctccagacaacttcaaaattccatgagtggagcttctgctgattcaactcaggcataaacactcatgatgaccacacaaggcagatgggctatgtaaacgttttcgcaattccgtttacgatacatagtctactcttgtgcagaatgaattctcgtaactaaacagcacaagtaggtttagttaactttaatctcacatagcaatctttaatcaatgtgtaacattagggaggacttgaaagagccaccacattttcatcgaggccacgcggagtacgatcgagggtacagtgaataatgctagggagagctgcctatatggaagagccctaatgtgtaaaattaattttagtagtgctatccccatgtgattttaatagcttcttaggagaatgacaaaaaaaaaaaaaaaaaaaaaaaa